European Patent Specification EP 3 934 668 B1, published April 8, 2026. Title: COMPOSITIONS AND METHODS FOR TREATING CANCER WITH SELF-DRIVING CHIMERIC ANTIGEN RECEPTORS. Applicant: LENTIGEN TECHNOLOGY, INC. The sequence listing filed with the application follows.

SEQUENCE LISTING (189 sequences)

SEQ ID NO: 1 - DNA, 8 bp, Artificial Sequence
  source: /note="Description of Artificial Sequence: Synthetic oligonucleotide"
ttctgaga

SEQ ID NO: 2 - DNA, 7 bp, Artificial Sequence
  source: /note="Description of Artificial Sequence: Synthetic oligonucleotide"
tgagtca

SEQ ID NO: 3 - DNA, 7 bp, Artificial Sequence
  source: /note="Description of Artificial Sequence: Synthetic oligonucleotide"
tgactca

SEQ ID NO: 4 - DNA, 10 bp, Artificial Sequence
  source: /note="Description of Artificial Sequence: Synthetic oligonucleotide"
gggaatttcc

SEQ ID NO: 5 - DNA, 10 bp, Artificial Sequence
  source: /note="Description of Artificial Sequence: Synthetic oligonucleotide"
gggactttcc

SEQ ID NO: 6 - DNA, 9 bp, Artificial Sequence
  source: /note="Description of Artificial Sequence: Synthetic oligonucleotide"
ggaatttcc

SEQ ID NO: 7 - DNA, 1494 bp, Artificial Sequence
  source: /note="Description of Artificial Sequence: Synthetic polynucleotide"
atgctgctgctggtgaccagcctgctgctgtgcgaactgccgcatccggcgtttctgctgattccggaagtgcaattggtgcagagcggtggaggacttgtgaaacctggtggatccctgagactttcctgtgccgcttcgggcttcaccttctcggactactacatgtcctggattcgccaggcccctggaaagggactggaatgggtgtcatacatcagctcctccggttccaccatctactatgccgattccgtgaagggcagattcaccatctcgcgcgacaacgccaagaacactctctatctgcaaatgaactcactgcgggctgaggacaccgcggtctactactgcgcccgggacctcagcggaaagtccagcggatggtcccattacttcgattactggggacagggaaccctggtcaccgtgtccagcggcggggggggctcgggtggcggcggctccggcggcggcgggagcaacttcatgctgactcagccccactccgtgtccgagagcccgggaaagaccgtgactatttcgtgcacacggtcctccgggagcattgcgaacaactacgtgcagtggtaccagcagcggcccgatagggccccaaccactgtgatctacgaagatgaccagcggccgtctggagtcccggaccgcttctcggggtccatcgactcatcatccaattccgcatcgctgacgatcagcggactgaagatcgaggacgaagccgattactactgccagtcctacgacggcaccaactgggtctttgggggtggaaccaagctgactgtgctcggagcggccgcaactaccacccctgcccctcggccgccgactccggccccaaccatcgcaagccaacccctctccttgcgccccgaagcttgccgcccggccgcgggtggagccgtgcatacccgggggctggactttgcctgcgatatctacatttgggccccgctggccggcacttgcggcgtgctcctgctgtcgctggtcatcaccctttactgcaagaggggccggaagaagctgctttacatcttcaagcagccgttcatgcggcccgtgcagacgactcaggaagaggacggatgctcgtgcagattccctgaggaggaagaggggggatgcgaactgcgcgtcaagttctcacggtccgccgacgcccccgcatatcaacagggccagaatcagctctacaacgagctgaacctgggaaggagagaggagtacgacgtgctggacaagcgacgcggacgcgacccggagatgggggggaaaccacggcggaaaaaccctcaggaaggactgtacaacgaactccagaaagacaagatggcggaagcctactcagaaatcgggatgaagggagagcggaggaggggaaagggtcacgacgggctgtaccagggactgagcaccgccactaaggatacctacgatgccttgcatatgcaagcactcccaccccgg

SEQ ID NO: 8 - protein, 498 aa, Artificial Sequence
  source: /note="Description of Artificial Sequence: Synthetic polypeptide"
MLLLVTSLLLCELPHPAFLLIPEVQLVQSGGGLVKPGGSLRLSCAASGFTFSDYYMSWIRQAPGKGLEWVSYISSSGSTIYYADSVKGRFTISRDNAKNTLYLQMNSLRAEDTAVYYCARDLSGKSSGWSHYFDYWGQGTLVTVSSGGGGSGGGGSGGGGSNFMLTQPHSVSESPGKTVTISCTRSSGSIANNYVQWYQQRPDRAPTTVIYEDDQRPSGVPDRFSGSIDSSSNSASLTISGLKIEDEADYYCQSYDGTNWVFGGGTKLTVLGAAATTTPAPRPPTPAPTIASQPLSLRPEACRPAAGGAVHTRGLDFACDIYIWAPLAGTCGVLLLSLVITLYCKRGRKKLLYIFKQPFMRPVQTTQEEDGCSCRFPEEEEGGCELRVKFSRSADAPAYQQGQNQLYNELNLGRREEYDVLDKRRGRDPEMGGKPRRKNPQEGLYNELQKDKMAEAYSEIGMKGERRRGKGHDGLYQGLSTATKDTYDALHMQALPPR

SEQ ID NO: 9 - DNA, 1473 bp, Artificial Sequence
  source: /note="Description of Artificial Sequence: Synthetic polynucleotide"
atgctgctgctggtgaccagcctgctgctgtgcgaactgccgcatccggcgtttctgctgattccggaagtgcaacttgtcgaaagcggtggaggtcttgtccaacctggtcgctccctgaggctctcgtgtgccgcgagcggattcaccttctcatcgtacgctatgtcctgggtcagacaggctcctggaaagggcctggaatgggtggccgtgatctcctacgacggcagcaacaagtattacgccgactcagtgaagggccggttcaccatttcccgggacaacagcaagaacaccctgtacttgcaaatgaactccctgcgggccgaggataccgcggtgtactactgcgcccacctccgctttggatacggaatggatgtctggggacagggaactaccgtgaccgtgtcgtccgggggggggggaagcggcggcgggggatcgggtggcggcggatcccagactgtggtcacccaagagccttcactgaccgtgtccccgggtggcaccgtgacgctgacttgcgcgtcatctaccggggccgtgacctcggaccactacccctgctggttccagcagaaacccggacatccaccgagagccctggtgtactccactgacaccatccactcctggactccggcccggttctccggaagcctcctgggcgggaaggccgcactgacagtgtccggagtgcagcccgaggatgaagccgactactactgtctgctctactatgggggagcacgcgtgttcggtggcggcactcagctgaccgtgctgggagcggccgcaactaccacccctgcccctcggccgccgactccggccccaaccatcgcaagccaacccctctccttgcgccccgaagcttgccgcccggccgcgggtggagccgtgcatacccgggggctggactttgcctgcgatatctacatttgggccccgctggccggcacttgcggcgtgctcctgctgtcgctggtcatcaccctttactgcaagaggggccggaagaagctgctttacatcttcaagcagccgttcatgcggcccgtgcagacgactcaggaagaggacggatgctcgtgcagattccctgaggaggaagaggggggatgcgaactgcgcgtcaagttctcacggtccgccgacgcccccgcatatcaacagggccagaatcagctctacaacgagctgaacctgggaaggagagaggagtacgacgtgctggacaagcgacgcggacgcgacccggagatgggggggaaaccacggcggaaaaaccctcaggaaggactgtacaacgaactccagaaagacaagatggcggaagcctactcagaaatcgggatgaagggagagcggaggaggggaaagggtcacgacgggctgtaccagggactgagcaccgccactaaggatacctacgatgccttgcatatgcaagcactcccaccccgg

SEQ ID NO: 10 - protein, 491 aa, Artificial Sequence
  source: /note="Description of Artificial Sequence: Synthetic polypeptide"
MLLLVTSLLLCELPHPAFLLIPEVQLVESGGGLVQPGRSLRLSCAASGFTFSSYAMSWVRQAPGKGLEWVAVISYDGSNKYYADSVKGRFTISRDNSKNTLYLQMNSLRAEDTAVYYCAHLRFGYGMDVWGQGTTVTVSSGGGGSGGGGSGGGGSQTVVTQEPSLTVSPGGTVTLTCASSTGAVTSDHYPCWFQQKPGHPPRALVYSTDTIHSWTPARFSGSLLGGKAALTVSGVQPEDEADYYCLLYYGGARVFGGGTQLTVLGAAATTTPAPRPPTPAPTIASQPLSLRPEACRPAAGGAVHTRGLDFACDIYIWAPLAGTCGVLLLSLVITLYCKRGRKKLLYIFKQPFMRPVQTTQEEDGCSCRFPEEEEGGCELRVKFSRSADAPAYQQGQNQLYNELNLGRREEYDVLDKRRGRDPEMGGKPRRKNPQEGLYNELQKDKMAEAYSEIGMKGERRRGKGHDGLYQGLSTATKDTYDALHMQALPPR

SEQ ID NO: 11 - DNA, 1467 bp, Artificial Sequence
  source: /note="Description of Artificial Sequence: Synthetic polynucleotide"
atgctgctgctggtgaccagcctgctgctgtgcgaactgccgcatccggcgtttctgctgattccgcaagtccaactcgtccagtccggtgccgaagtcaagaagcctggctcatccgtgaaagtgtcctgcaaagcatcgggcggaaccttctcctcctatgccatttcctgggtccgccaggcaccgggccagggtctggagtggatgggcgggattatccctatcttcggaactgccaaccacgcccaaaagttccagggacgcgtgaccattaccgccgatgaatcaacctcaaccgcctacatggaactgtccagcttgaggtccgaggacaccgccgtgtactactgcgcgttcatgatggtgccggagtactactttgactactggggccagggaacccttgtgaccgtgtcgtccggtggtggcggatccgggggggggggatctgggggcggcggaagcgatatccagatgacccagtcgccatcgagcctgtccgcttccgtgggcgacagagtgacgatcacttgccgggcttcacaaggcatcagaaatgacctgggctggtatcagcagaagcccggagaagcgcccaagcggctgatctacgcggccagcaccctgcaaaacggagtgccttcgcggttctccgggagcggctccggaactgacttcactctgactattaacagcctccagcccgaggatttcgccacatactactgtcagcagtacaacagctacccgtacaccttcggacagggaactaagctcgaaatcaaggcggccgcaactaccacccctgcccctcggccgccgactccggccccaaccatcgcaagccaacccctctccttgcgccccgaagcttgccgcccggccgcgggtggagccgtgcatacccgggggctggactttgcctgcgatatctacatttgggccccgctggccggcacttgcggcgtgctcctgctgtcgctggtcatcaccctttactgcaagaggggccggaagaagctgctttacatcttcaagcagccgttcatgcggcccgtgcagacgactcaggaagaggacggatgctcgtgcagattccctgaggaggaagaggggggatgcgaactgcgcgtcaagttctcacggtccgccgacgcccccgcatatcaacagggccagaatcagctctacaacgagctgaacctgggaaggagagaggagtacgacgtgctggacaagcgacgcggacgcgacccggagatgggggggaaaccacggcggaaaaaccctcaggaaggactgtacaacgaactccagaaagacaagatggcggaagcctactcagaaatcgggatgaagggagagcggaggaggggaaagggtcacgacgggctgtaccagggactgagcaccgccactaaggatacctacgatgccttgcatatgcaagcactcccaccccgg

SEQ ID NO: 12 - protein, 489 aa, Artificial Sequence
  source: /note="Description of Artificial Sequence: Synthetic polypeptide"
MLLLVTSLLLCELPHPAFLLIPQVQLVQSGAEVKKPGSSVKVSCKASGGTFSSYAISWVRQAPGQGLEWMGGIIPIFGTANHAQKFQGRVTITADESTSTAYMELSSLRSEDTAVYYCAFMMVPEYYFDYWGQGTLVTVSSGGGGSGGGGSGGGGSDIQMTQSPSSLSASVGDRVTITCRASQGIRNDLGWYQQKPGEAPKRLIYAASTLQNGVPSRFSGSGSGTDFTLTINSLQPEDFATYYCQQYNSYPYTFGQGTKLEIKAAATTTPAPRPPTPAPTIASQPLSLRPEACRPAAGGAVHTRGLDFACDIYIWAPLAGTCGVLLLSLVITLYCKRGRKKLLYIFKQPFMRPVQTTQEEDGCSCRFPEEEEGGCELRVKFSRSADAPAYQQGQNQLYNELNLGRREEYDVLDKRRGRDPEMGGKPRRKNPQEGLYNELQKDKMAEAYSEIGMKGERRRGKGHDGLYQGLSTATKDTYDALHMQALPPR

SEQ ID NO: 13 - DNA, 66 bp, Artificial Sequence
  source: /note="Description of Artificial Sequence: Synthetic oligonucleotide"
atgctgctgctggtgaccagcctgctgctgtgcgaactgccgcatccggcgtttctgctgattccg

SEQ ID NO: 14 - protein, 22 aa, Artificial Sequence
  source: /note="Description of Artificial Sequence: Synthetic peptide"
MLLLVTSLLLCELPHPAFLLIP

SEQ ID NO: 15 - DNA, 1500 bp, Artificial Sequence
  source: /note="Description of Artificial Sequence: Synthetic polynucleotide"
atgctgctgctggtgaccagcctgctgctgtgcgaactgccgcatccggcgtttctgctgattccgcaactccaactccaagaatctggaccaggcctcgtgaagccctcccaaactctgtccctgacctgtaccgtgtcgggtggaagcatttcgagcggtggatactactggtcctggatcaggcagcatcctggaaagggactggagtggattgggtacatctactactccggctcaacctactacaacccgtccttgaaatcgcgcgtgacgatctccgtggacacttcaaagaaccagttcagcctgaagctttcctccgtgaccgcggccgatacagcggtgtactactgcgctcgggatcagagcgtggccgaccctggtggcggctactactactacggaatggatgtctggggacagggaaccaccgtgactgtgtccagcgggggcggcggatccgggggggggggatcgggcggcggcggttcgcagtccgtgctgacccagccacctagcgtgtcagtggcaccgggacagaccgcctccatttcctgcgggggaaatgacttcggtagccgctccgtgtcatggtatcaccagaagccgggacaggccccggtgctggtcatctatgacgacaacgacagaccctcgggcatccccgaacggttttcgggaagcacctccggagacactgccaccctgaccatctcccgggtcgaggtcggcgatgaagccgattactactgccaagtctgggacgacgactccgaccactgggtgttcggcggcggaactaagctgactgtgctgggggcggccgcaactaccacccctgcccctcggccgccgactccggccccaaccatcgcaagccaacccctctccttgcgccccgaagcttgccgcccggccgcgggtggagccgtgcatacccgggggctggactttgcctgcgatatctacatttgggccccgctggccggcacttgcggcgtgctcctgctgtcgctggtcatcaccctttactgcaagaggggccggaagaagctgctttacatcttcaagcagccgttcatgcggcccgtgcagacgactcaggaagaggacggatgctcgtgcagattccctgaggaggaagaggggggatgcgaactgcgcgtcaagttctcacggtccgccgacgcccccgcatatcaacagggccagaatcagctctacaacgagctgaacctgggaaggagagaggagtacgacgtgctggacaagcgacgcggacgcgacccggagatgggggggaaaccacggcggaaaaaccctcaggaaggactgtacaacgaactccagaaagacaagatggcggaagcctactcagaaatcgggatgaagggagagcggaggaggggaaagggtcacgacgggctgtaccagggactgagcaccgccactaaggatacctacgatgccttgcatatgcaagcactcccaccccgg

SEQ ID NO: 16 - protein, 500 aa, Artificial Sequence
  source: /note="Description of Artificial Sequence: Synthetic polypeptide"
MLLLVTSLLLCELPHPAFLLIPQLQLQESGPGLVKPSQTLSLTCTVSGGSISSGGYYWSWIRQHPGKGLEWIGYIYYSGSTYYNPSLKSRVTISVDTSKNQFSLKLSSVTAADTAVYYCARDQSVADPGGGYYYYGMDVWGQGTTVTVSSGGGGSGGGGSGGGGSQSVLTQPPSVSVAPGQTASISCGGNDFGSRSVSWYHQKPGQAPVLVIYDDNDRPSGIPERFSGSTSGDTATLTISRVEVGDEADYYCQVWDDDSDHWVFGGGTKLTVLGAAATTTPAPRPPTPAPTIASQPLSLRPEACRPAAGGAVHTRGLDFACDIYIWAPLAGTCGVLLLSLVITLYCKRGRKKLLYIFKQPFMRPVQTTQEEDGCSCRFPEEEEGGCELRVKFSRSADAPAYQQGQNQLYNELNLGRREEYDVLDKRRGRDPEMGGKPRRKNPQEGLYNELQKDKMAEAYSEIGMKGERRRGKGHDGLYQGLSTATKDTYDALHMQALPPR

SEQ ID NO: 17 - DNA, 1467 bp, Artificial Sequence
  source: /note="Description of Artificial Sequence: Synthetic polynucleotide"
atgctgctgctggtgaccagcctgctgctgtgcgaactgccgcatccggcgtttctgctgattccgcaagttcagctgcaagaatcaggacctgggcttgtcaaaccatctgaaaccctcagcttgacttgtaccgtatcaggagggtcaatttcaagctcatcctactattggggatggatcagacaaccacccgggaaagggctcgagtggatagggtccatatattacagcggatctacatactacaacccgtcattgaagtccagggtaacgattccggtggacactagcaagaatcagtttagcctcaagttgagcagtgtaactgctgcggacacggcggtatattattgtgctcgacacctcggtggagatgcttttgacatatggggtcaagggacaacagtcaccgttagctcaggtggagggggtagcggggggggcggatctgggggaggcggttcattgcccgtacttacacagccaccctctgtcagcgtcgcacctggacaaaccgctcgcatcacctgtggcggaaataatataggttccaagtctgttcattggtatcagcagaaaccgggacaggcccccgtccttgtggtgtatgatgattctgataggccatctggtatcccagaacggttttcaggtagcaattcagggaatactgccactctcactattagcggtactcaagctatggatgaggccgactatttttgccagagctacgactctagtaacccagtcgtgttcgggggagggacccagttgaccgtgctggcggccgcaactaccacccctgcccctcggccgccgactccggccccaaccatcgcaagccaacccctctccttgcgccccgaagcttgccgcccggccgcgggtggagccgtgcatacccgggggctggactttgcctgcgatatctacatttgggccccgctggccggcacttgcggcgtgctcctgctgtcgctggtcatcaccctttactgcaagaggggccggaagaagctgctttacatcttcaagcagccgttcatgcggcccgtgcagacgactcaggaagaggacggatgctcgtgcagattccctgaggaggaagaggggggatgcgaactgcgcgtcaagttctcacggtccgccgacgcccccgcatatcaacagggccagaatcagctctacaacgagctgaacctgggaaggagagaggagtacgacgtgctggacaagcgacgcggacgcgacccggagatgggggggaaaccacggcggaaaaaccctcaggaaggactgtacaacgaactccagaaagacaagatggcggaagcctactcagaaatcgggatgaagggagagcggaggaggggaaagggtcacgacgggctgtaccagggactgagcaccgccactaaggatacctacgatgccttgcatatgcaagcactcccaccccgg

SEQ ID NO: 18 - protein, 489 aa, Artificial Sequence
  source: /note="Description of Artificial Sequence: Synthetic polypeptide"
MLLLVTSLLLCELPHPAFLLIPQVQLQESGPGLVKPSETLSLTCTVSGGSISSSSYYWGWIRQPPGKGLEWIGSIYYSGSTYYNPSLKSRVTIPVDTSKNQFSLKLSSVTAADTAVYYCARHLGGDAFDIWGQGTTVTVSSGGGGSGGGGSGGGGSLPVLTQPPSVSVAPGQTARITCGGNNIGSKSVHWYQQKPGQAPVLVVYDDSDRPSGIPERFSGSNSGNTATLTISGTQAMDEADYFCQSYDSSNPVVFGGGTQLTVLAAATTTPAPRPPTPAPTIASQPLSLRPEACRPAAGGAVHTRGLDFACDIYIWAPLAGTCGVLLLSLVITLYCKRGRKKLLYIFKQPFMRPVQTTQEEDGCSCRFPEEEEGGCELRVKFSRSADAPAYQQGQNQLYNELNLGRREEYDVLDKRRGRDPEMGGKPRRKNPQEGLYNELQKDKMAEAYSEIGMKGERRRGKGHDGLYQGLSTATKDTYDALHMQALPPR

SEQ ID NO: 19 - DNA, 1476 bp, Artificial Sequence
  source: /note="Description of Artificial Sequence: Synthetic polynucleotide"
atgctgctgctggtgaccagcctgctgctgtgcgaactgccgcatccggcgtttctgctgattccgcaggcggcccaggtacagctgcagcagtcaggggctgaggtgaagaagcctgggtcctcggtgaaggtctcctgcaaggcttctggaggcaccttcagcagctatgctatcagctgggtgcgacaggcccctggacaagggcttgagtggatgggatggatcaaccctaacagtggtggcacaaactatgcacagaggtttcagggcagggtcaccatgaccagggacacgtccatcagcacagcctacatggagctgagcaggctgagatctgacgacacggccgtgtattactgtgcgagttataatgatgcttttgatatctggggccaaggcaccctggtcaccgtctcctcaggaggtggcgggtctggtggtggcggtagcggtggtggcggatccaattttatgctgactcagccccactctgtgtcggagtctccggggaagacggtaaccatctcctgcacccgcagcagtggcagcattgccagcaactatgtgcagtggtaccagcagcgcccgggcagtgcccccaccattgtgatctatgaggatgatcaaagaccctctggggtccctgatcggttctctggctccatcgacacctcctccaactctgcctccctcaccatctctggactgcagagtgaggacgaggctgactactactgtcagtcttatgagcccggcaatggggtattcggcggagggaccaaggtcaccgtcctagcggccgcaactaccacccctgcccctcggccgccgactccggccccaaccatcgcaagccaacccctctccttgcgccccgaagcttgccgcccggccgcgggtggagccgtgcatacccgggggctggactttgcctgcgatatctacatttgggccccgctggccggcacttgcggcgtgctcctgctgtcgctggtcatcaccctttactgcaagaggggccggaagaagctgctttacatcttcaagcagccgttcatgcggcccgtgcagacgactcaggaagaggacggatgctcgtgcagattccctgaggaggaagaggggggatgcgaactgcgcgtcaagttctcacggtccgccgacgcccccgcatatcaacagggccagaatcagctctacaacgagctgaacctgggaaggagagaggagtacgacgtgctggacaagcgacgcggacgcgacccggagatgggggggaaaccacggcggaaaaaccctcaggaaggactgtacaacgaactccagaaagacaagatggcggaagcctactcagaaatcgggatgaagggagagcggaggaggggaaagggtcacgacgggctgtaccagggactgagcaccgccactaaggatacctacgatgccttgcatatgcaagcactcccaccccgg

SEQ ID NO: 20 - protein, 492 aa, Artificial Sequence
  source: /note="Description of Artificial Sequence: Synthetic polypeptide"
MLLLVTSLLLCELPHPAFLLIPQAAQVQLQQSGAEVKKPGSSVKVSCKASGGTFSSYAISWVRQAPGQGLEWMGWINPNSGGTNYAQRFQGRVTMTRDTSISTAYMELSRLRSDDTAVYYCASYNDAFDIWGQGTLVTVSSGGGGSGGGGSGGGGSNFMLTQPHSVSESPGKTVTISCTRSSGSIASNYVQWYQQRPGSAPTIVIYEDDQRPSGVPDRFSGSIDTSSNSASLTISGLQSEDEADYYCQSYEPGNGVFGGGTKVTVLAAATTTPAPRPPTPAPTIASQPLSLRPEACRPAAGGAVHTRGLDFACDIYIWAPLAGTCGVLLLSLVITLYCKRGRKKLLYIFKQPFMRPVQTTQEEDGCSCRFPEEEEGGCELRVKFSRSADAPAYQQGQNQLYNELNLGRREEYDVLDKRRGRDPEMGGKPRRKNPQEGLYNELQKDKMAEAYSEIGMKGERRRGKGHDGLYQGLSTATKDTYDALHMQALPPR

SEQ ID NO: 21 - DNA, 1488 bp, Artificial Sequence
  source: /note="Description of Artificial Sequence: Synthetic polynucleotide"
atgctgctgctggtgaccagcctgctgctgtgcgaactgccgcatccggcgtttctgctgattccgcaagaacagcttgtagagtccggcggtagattggtgacaccgggggggagccttaccctgtcttgtaaggcatctgggttcgatttcagtgcgtattatatgagctgggttcggcaggcgcccgggaaggggctggaatggatagccactatatacccgtcatccggcaagacttactacgcgacttgggtaaacgggaggtttacgataagctcagataacgcccaaaacacggttgatctccaaatgaatagcttgaccgccgctgatagggcgacctatttctgtgcgcgggactcttacgctgatgacggggccctcttcaatatatggggaccgggaacgctcgtaaccatatcatctggaggaggtgggagcggaggcggagggtcaggtgggggcgggagcgaactcgtacttacacaatctccaagcgtaagcgcagcgttggggagtccagcaaagatcacctgcactttgtcaagcgcccacaaaacggatacgatagattggtatcagcaactccaaggtgaagcgccacgatatctcatgcaggtacagagcgacgggagttatactaagaggcccggggtcccagacagattcagtggcagcagttcaggtgccgacagatacctgataataccctcagttcaagccgatgatgaagccgattactactgtggggctgactacataggtgggtatgttttcgggggcggcactcaattgacagttacaggggcggccgcaactaccacccctgcccctcggccgccgactccggccccaaccatcgcaagccaacccctctccttgcgccccgaagcttgccgcccggccgcgggtggagccgtgcatacccgggggctggactttgcctgcgatatctacatttgggccccgctggccggcacttgcggcgtgctcctgctgtcgctggtcatcaccctttactgcaagaggggccggaagaagctgctttacatcttcaagcagccgttcatgcggcccgtgcagacgactcaggaagaggacggatgctcgtgcagattccctgaggaggaagaggggggatgcgaactgcgcgtcaagttctcacggtccgccgacgcccccgcatatcaacagggccagaatcagctctacaacgagctgaacctgggaaggagagaggagtacgacgtgctggacaagcgacgcggacgcgacccggagatgggggggaaaccacggcggaaaaaccctcaggaaggactgtacaacgaactccagaaagacaagatggcggaagcctactcagaaatcgggatgaagggagagcggaggaggggaaagggtcacgacgggctgtaccagggactgagcaccgccactaaggatacctacgatgccttgcatatgcaagcactcccaccccgg

SEQ ID NO: 22 - protein, 496 aa, Artificial Sequence
  source: /note="Description of Artificial Sequence: Synthetic polypeptide"
MLLLVTSLLLCELPHPAFLLIPQEQLVESGGRLVTPGGSLTLSCKASGFDFSAYYMSWVRQAPGKGLEWIATIYPSSGKTYYATWVNGRFTISSDNAQNTVDLQMNSLTAADRATYFCARDSYADDGALFNIWGPGTLVTISSGGGGSGGGGSGGGGSELVLTQSPSVSAALGSPAKITCTLSSAHKTDTIDWYQQLQGEAPRYLMQVQSDGSYTKRPGVPDRFSGSSSGADRYLIIPSVQADDEADYYCGADYIGGYVFGGGTQLTVTGAAATTTPAPRPPTPAPTIASQPLSLRPEACRPAAGGAVHTRGLDFACDIYIWAPLAGTCGVLLLSLVITLYCKRGRKKLLYIFKQPFMRPVQTTQEEDGCSCRFPEEEEGGCELRVKFSRSADAPAYQQGQNQLYNELNLGRREEYDVLDKRRGRDPEMGGKPRRKNPQEGLYNELQKDKMAEAYSEIGMKGERRRGKGHDGLYQGLSTATKDTYDALHMQALPPR

SEQ ID NO: 23 - DNA, 1464 bp, Artificial Sequence
  source: /note="Description of Artificial Sequence: Synthetic polynucleotide"
atgctgctgctggtgaccagcctgctgctgtgcgaactgccgcatccggcgtttctgctgattccggaagtgcaactcgtcgaaactggagccgaagtgaaaaagcctggagcgtccgtcaaagtgtcgtgcaaggcctccggctacaccttcacgacctactacgtgcactgggtcagacaggctccgggtcaagggctggagtggatgggcatcattaacccctccggtggaagcacctcctatgcgcaaaagttccagggtcgcgtcaccatgactcgcgatacctccacttccactgtgtacatggaactgagctccctgaggtccgaggacaccgccgtgtactactgcgcacgggatggaggcttgggcggctacgaggcttggggacagggcaccctcgtgactgtgtcaagcggagggggtggatccggagggggaggatcaggcggtggtggaagcgatatccagcttacccagtcgccttccgcgctgtctgcatcggccggcgacagagtgacaattacctgtcaagccagccaggacatctccaactatctgaactggtaccagcagaagcccggaaaggctccgaagctgctgatctacgacgccagcaacctggaacggggcgtgccatcacggttctcgggatcagggtcgggcactgagttcaccttcaccatctcctccctccaacccgaggacattgccacctactactgccagcagtacgacaacctcccgatcacctttggacaggggactcgcctggaaatcaaggcggccgcaactaccacccctgcccctcggccgccgactccggccccaaccatcgcaagccaacccctctccttgcgccccgaagcttgccgcccggccgcgggtggagccgtgcatacccgggggctggactttgcctgcgatatctacatttgggccccgctggccggcacttgcggcgtgctcctgctgtcgctggtcatcaccctttactgcaagaggggccggaagaagctgctttacatcttcaagcagccgttcatgcggcccgtgcagacgactcaggaagaggacggatgctcgtgcagattccctgaggaggaagaggggggatgcgaactgcgcgtcaagttctcacggtccgccgacgcccccgcatatcaacagggccagaatcagctctacaacgagctgaacctgggaaggagagaggagtacgacgtgctggacaagcgacgcggacgcgacccggagatgggggggaaaccacggcggaaaaaccctcaggaaggactgtacaacgaactccagaaagacaagatggcggaagcctactcagaaatcgggatgaagggagagcggaggaggggaaagggtcacgacgggctgtaccagggactgagcaccgccactaaggatacctacgatgccttgcatatgcaagcactcccaccccgg

SEQ ID NO: 24 - protein, 488 aa, Artificial Sequence
  source: /note="Description of Artificial Sequence: Synthetic polypeptide"
MLLLVTSLLLCELPHPAFLLIPEVQLVETGAEVKKPGASVKVSCKASGYTFTTYYVHWVRQAPGQGLEWMGIINPSGGSTSYAQKFQGRVTMTRDTSTSTVYMELSSLRSEDTAVYYCARDGGLGGYEAWGQGTLVTVSSGGGGSGGGGSGGGGSDIQLTQSPSALSASAGDRVTITCQASQDISNYLNWYQQKPGKAPKLLIYDASNLERGVPSRFSGSGSGTEFTFTISSLQPEDIATYYCQQYDNLPITFGQGTRLEIKAAATTTPAPRPPTPAPTIASQPLSLRPEACRPAAGGAVHTRGLDFACDIYIWAPLAGTCGVLLLSLVITLYCKRGRKKLLYIFKQPFMRPVQTTQEEDGCSCRFPEEEEGGCELRVKFSRSADAPAYQQGQNQLYNELNLGRREEYDVLDKRRGRDPEMGGKPRRKNPQEGLYNELQKDKMAEAYSEIGMKGERRRGKGHDGLYQGLSTATKDTYDALHMQALPPR

SEQ ID NO: 25 - DNA, 1503 bp, Artificial Sequence
  source: /note="Description of Artificial Sequence: Synthetic polynucleotide"
atgctgctgctggtgaccagcctgctgctgtgcgaactgccgcatccggcgtttctgctgattccggaagtgcaattggtccagagcggaggaggacttgtgaagccaggcggatccctgagattgtcatgcgccgcatcggggttcaccttttcctcctactccatgaactgggtcagacaggcgcccggaaagggacttgaatgggtgtcgtccatttcctcctcctcgtcctacatctactacgccgactccgtgaagggccgcttcaccatctcccgggacaacgccaagaacagcctgtatctccaaatgaactccctgcgggccgaagatactgctgtgtattactgcgctcgggacttcccgtacgactcatcgggctattactcggacgcgttcgatatctggggccagggaactatggtcaccgtcagctctggtggcggtggttccggagggggtggatccggtggcggaggatcagagattgtgctgacccagtccccgctgtcactgcccgtgactccgggagagcctgcctcgatctcgtgtcggtccagccagtccctgctgcactcgaatgggtacaactacctcgattggtacctccaaaagcctgggcagtcaccccaactgctgatctacctcgggagcaacagagccagcggagtgcctgaccgctttagcggttccggatccggcaccgacttcaccctgaaaatcagccgggtggaagccgaggatgtcggcgtgtactactgcatgcaggcactgcagactctggggtacaccttcggccagggcacgaagctcgagatcaaggcggccgcaactaccacccctgcccctcggccgccgactccggccccaaccatcgcaagccaacccctctccttgcgccccgaagcttgccgcccggccgcgggtggagccgtgcatacccgggggctggactttgcctgcgatatctacatttgggccccgctggccggcacttgcggcgtgctcctgctgtcgctggtcatcaccctttactgcaagaggggccggaagaagctgctttacatcttcaagcagccgttcatgcggcccgtgcagacgactcaggaagaggacggatgctcgtgcagattccctgaggaggaagaggggggatgcgaactgcgcgtcaagttctcacggtccgccgacgcccccgcatatcaacagggccagaatcagctctacaacgagctgaacctgggaaggagagaggagtacgacgtgctggacaagcgacgcggacgcgacccggagatgggggggaaaccacggcggaaaaaccctcaggaaggactgtacaacgaactccagaaagacaagatggcggaagcctactcagaaatcgggatgaagggagagcggaggaggggaaagggtcacgacgggctgtaccagggactgagcaccgccactaaggatacctacgatgccttgcatatgcaagcactcccaccccgg

SEQ ID NO: 26 - protein, 501 aa, Artificial Sequence
  source: /note="Description of Artificial Sequence: Synthetic polypeptide"
MLLLVTSLLLCELPHPAFLLIPEVQLVQSGGGLVKPGGSLRLSCAASGFTFSSYSMNWVRQAPGKGLEWVSSISSSSSYIYYADSVKGRFTISRDNAKNSLYLQMNSLRAEDTAVYYCARDFPYDSSGYYSDAFDIWGQGTMVTVSSGGGGSGGGGSGGGGSEIVLTQSPLSLPVTPGEPASISCRSSQSLLHSNGYNYLDWYLQKPGQSPQLLIYLGSNRASGVPDRFSGSGSGTDFTLKISRVEAEDVGVYYCMQALQTLGYTFGQGTKLEIKAAATTTPAPRPPTPAPTIASQPLSLRPEACRPAAGGAVHTRGLDFACDIYIWAPLAGTCGVLLLSLVITLYCKRGRKKLLYIFKQPFMRPVQTTQEEDGCSCRFPEEEEGGCELRVKFSRSADAPAYQQGQNQLYNELNLGRREEYDVLDKRRGRDPEMGGKPRRKNPQEGLYNELQKDKMAEAYSEIGMKGERRRGKGHDGLYQGLSTATKDTYDALHMQALPPR

SEQ ID NO: 27 - DNA, 72 bp, Artificial Sequence
  source: /note="Description of Artificial Sequence: Synthetic oligonucleotide"
atctacatctgggcgcccttggccgggacttgtggggtccttctcctgtcactggttatcaccctttactgc

SEQ ID NO: 28 - protein, 22 aa, Artificial Sequence
  source: /note="Description of Artificial Sequence: Synthetic peptide"
IWAPLAGTCGVLLLSLVITLYC

SEQ ID NO: 29 - DNA, 135 bp, Artificial Sequence
  source: /note="Description of Artificial Sequence: Synthetic polynucleotide"
accacgacgccagcgccgcgaccaccaacaccggcgcccaccatcgcgtcgcagcccctgtccctgcgcccagaggcgtgccggccagcggcggggggcgcagtgcacacgagggggctggacttcgcctgtgat

SEQ ID NO: 30 - protein, 47 aa, Artificial Sequence
  source: /note="Description of Artificial Sequence: Synthetic polypeptide"
TTTPAPRPPTPAPTIASQPLSLRPEACRPAAGGAVHTRGLDFACDIY

SEQ ID NO: 31 - protein, 42 aa, Homo sapiens
KRGRKKLLYIFKQPFMRPVQTTQEEDGCSCRFPEEEEGGCEL

SEQ ID NO: 32 - protein, 106 aa, Homo sapiens
GQPKAAPSVTLFPPSSEELQANKATLVCLISDFYPGAVTVAWKADSSPVKAGVETTTPSKQSNNKYAASSYLSLTPEQWKSHRSYSCQVTHEGSTVEKTVAPTECS

SEQ ID NO: 33 - DNA, 126 bp, Artificial Sequence
  source: /note="Description of Artificial Sequence: Synthetic polynucleotide"
aaacggggcagaaagaaactcctgtatatattcaaacaaccatttatgagaccagtacaaactactcaagaggaagatggctgtagctgccgatttccagaagaagaagaaggaggatgtgaactg

SEQ ID NO: 34 - protein, 42 aa, Artificial Sequence; identical to SEQ ID NO: 31
  source: /note="Description of Artificial Sequence: Synthetic polypeptide"

SEQ ID NO: 35 - DNA, 336 bp, Artificial Sequence
  source: /note="Description of Artificial Sequence: Synthetic polynucleotide"
agagtgaagttcagcaggagcgcagacgcccccgcgtacaagcagggccagaaccagctctataacgagctcaatctaggacgaagagaggagtacgatgttttggacaagagacgtggccgggaccctgagatggggggaaagccgagaaggaagaaccctcaggaaggcctgtacaatgaactgcagaaagataagatggcggaggcctacagtgagattgggatgaaaggcgagcgccggaggggcaaggggcacgatggcctttaccagggtctcagtacagccaccaaggacacctacgacgcccttcacatgcaggccctgccccctcgc

SEQ ID NO: 36 - protein, 112 aa, Artificial Sequence
  source: /note="Description of Artificial Sequence: Synthetic polypeptide"
RVKFSRSADAPAYKQGQNQLYNELNLGRREEYDVLDKRRGRDPEMGGKPRRKNPQEGLYNELQKDKMAEAYSEIGMKGERRRGKGHDGLYQGLSTATKDTYDALHMQALPPR

SEQ ID NO: 37 - DNA, 726 bp, Artificial Sequence
  source: /note="Description of Artificial Sequence: Synthetic polynucleotide"
gacatccagatgacacagactacatcctccctgtctgcctctctgggagacagagtcaccatcagttgcagggcaagtcaggacattagtaaatatttaaattggtatcagcagaaaccagatggaactgttaaactcctgatctaccatacatcaagattacactcaggagtcccatcaaggttcagtggcagtgggtctggaacagattattctctcaccattagcaacctggagcaagaagatattgccacttacttttgccaacagggtaatacgcttccgtacacgttcggaggggggaccaagctggagatcacaggtggcggtggctcgggcggtggtgggtcgggtggcggcggatctgaggtgaaactgcaggagtcaggacctggcctggtggcgccctcacagagcctgtccgtcacatgcactgtctcaggggtctcattacccgactatggtgtaagctggattcgccagcctccacgaaagggtctggagtggctgggagtaatatggggtagtgaaaccacatactataattcagctctcaaatccagactgaccatcatcaaggacaactccaagagccaagttttcttaaaaatgaacagtctgcaaactgatgacacagccatttactactgtgccaaacattattactacggtggtagctatgctatggactactggggccaaggaacctcagtcaccgtctcctca

SEQ ID NO: 38 - protein, 242 aa, Artificial Sequence
  source: /note="Description of Artificial Sequence: Synthetic polypeptide"
DIQMTQTTSSLSASLGDRVTISCRASQDISKYLNWYQQKPDGTVKLLIYHTSRLHSGVPSRFSGSGSGTDYSLTISNLEQEDIATYFCQQGNTLPYTFGGGTKLEITGGGGSGGGGSGGGGSEVKLQESGPGLVAPSQSLSVTCTVSGVSLPDYGVSWIRQPPRKGLEWLGVIWGSETTYYNSALKSRLTIIKDNSKSQVFLKMNSLQTDDTAIYYCAKHYYYGGSYAMDYWGQGTSVTVSS

SEQ ID NO: 39 - DNA, 66 bp, Artificial Sequence; identical to SEQ ID NO: 13
  source: /note="Description of Artificial Sequence: Synthetic oligonucleotide"

SEQ ID NO: 40 - protein, 22 aa, Artificial Sequence
  source: /note="Description of Artificial Sequence: Synthetic peptide"
MLLLVTSLLLCELPHPAFLLIP

SEQ ID NO: 41 - DNA, 85 bp, Artificial Sequence
  source: /note="Description of Artificial Sequence: Synthetic oligonucleotide"
ggctctgaaagtgctgttggaacaagaaaagaccttcttcaccttgctcgtgttgctggggtacctgtcctgcaaagtcacctgt

SEQ ID NO: 42 - protein, 29 aa, Artificial Sequence
  source: /note="Description of Artificial Sequence: Synthetic peptide"
MALKVLLEQEKTFFTLLVLLGYLSCKVTC

SEQ ID NO: 43 - DNA, 63 bp, Artificial Sequence
  source: /note="Description of Artificial Sequence: Synthetic oligonucleotide"
atggcgctgccggtgaccgcgctgctgctgccgctggcgctgctgctgcatgcggcgcgcccg

SEQ ID NO: 44 - protein, 21 aa, Artificial Sequence
  source: /note="Description of Artificial Sequence: Synthetic peptide"
MALPVTALLLPLALLLHAARP

SEQ ID NO: 45 - DNA, 123 bp, Artificial Sequence
  source: /note="Description of Artificial Sequence: Synthetic polynucleotide"
cggtcgaagaggtccagactcttgcactccgactacatgaacatgactcctagaaggcccggacccactagaaagcactaccagccgtacgcccctcctcgggatttcgccgcataccggtcc

SEQ ID NO: 46 - protein, 41 aa, Artificial Sequence
  source: /note="Description of Artificial Sequence: Synthetic polypeptide"
RSKRSRLLHSDYMNMTPRRPGPTRKHYQPYAPPRDFAAYRS

SEQ ID NO: 47 - DNA, 336 bp, Artificial Sequence
  source: /note="Description of Artificial Sequence: Synthetic polynucleotide"
agagtgaagttcagccgctcagccgatgcaccggcctaccagcagggacagaaccagctctacaacgagctcaacctgggtcggcgggaagaatatgacgtgctggacaaacggcgcggcagagatccggagatggggggaaagccgaggaggaagaaccctcaagagggcctgtacaacgaactgcagaaggacaagatggcggaagcctactccgagatcggcatgaagggagaacgccggagagggaagggtcatgacggactgtaccagggcctgtcaactgccactaaggacacttacgatgcgctccatatgcaagctttgcccccgcgg

SEQ ID NO: 48 - protein, 112 aa, Artificial Sequence
  source: /note="Description of Artificial Sequence: Synthetic polypeptide"
RVKFSRSADAPAYQQGQNQLYNELNLGRREEYDVLDKRRGRDPEMGGKPRRKNPQEGLYNELQKDKMAEAYSEIGMKGERRRGKGHDGLYQGLSTATKDTYDALHMQALPPR

SEQ ID NO: 49 - DNA, 201 bp, Artificial Sequence
  source: /note="Description of Artificial Sequence: Synthetic polynucleotide"
gcggccgcggtcggattccaagacatggaatgcgtgccctgcggcgacccgccacctccttacgagccgcactgcgcatcgaaggtcaacctcgtgaagatcgcgagcaccgcgtcctcaccccgggatactgctctggccgccgtgatttgttccgccttggccaccgtgcttctggccctgctgatcctctgtgtgatc

SEQ ID NO: 50 - protein, 67 aa, Artificial Sequence
  source: /note="Description of Artificial Sequence: Synthetic polypeptide"
AAAVGFQDMECVPCGDPPPPYEPHCASKVNLVKIASTASSPRDTALAAVICSALATVLLALLILCVI

SEQ ID NO: 51 - DNA, 63 bp, Artificial Sequence
  source: /note="Description of Artificial Sequence: Synthetic oligonucleotide"
gccgccgtgatttgttccgccttggccaccgtgcttctggccctgctgatcctctgtgtgatc

SEQ ID NO: 52 - protein, 21 aa, Artificial Sequence
  source: /note="Description of Artificial Sequence: Synthetic peptide"
AAVICSALATVLLALLILCVI

SEQ ID NO: 53 - DNA, 138 bp, Artificial Sequence
  source: /note="Description of Artificial Sequence: Synthetic polynucleotide"
gcggccgcggtcggattccaagacatggaatgcgtgccctgcggcgacccgccacctccttacgagccgcactgcgcatcgaaggtcaacctcgtgaagatcgcgagcaccgcgtcctcaccccgggatactgctctg

SEQ ID NO: 54 - protein, 46 aa, Artificial Sequence
  source: /note="Description of Artificial Sequence: Synthetic polypeptide"
AAAVGFQDMECVPCGDPPPPYEPHCASKVNLVKIASTASSPRDTAL

SEQ ID NO: 55 - DNA, 80 bp, Artificial Sequence
  source: /note="Description of Artificial Sequence: Synthetic oligonucleotide"
tacgagcctcactgcgccagcaaagtcaacttggtgaagatcgcgagcactgcctcgtcccctcgggacactgctctggc

SEQ ID NO: 56 - protein, 26 aa, Artificial Sequence
  source: /note="Description of Artificial Sequence: Synthetic peptide"
YEPHCASKVNLVKIASTASSPRDTAL

SEQ ID NO: 57 - DNA, 222 bp, Artificial Sequence
  source: /note="Description of Artificial Sequence: Synthetic polynucleotide"
gcggccgcgcccgcccctcggcccccgactcctgccccgacgatcgcttcccaacctctctcgctgcgcccggaagcatgccggcccgccgccggtggcgctgtccacactcgcggactggactttgataccgcactggcggccgtgatctgtagcgccctggccaccgtgctgctggcgctgctcatcctttgcgtgatctactgcaagcggcagcctagg

SEQ ID NO: 58 - protein, 74 aa, Artificial Sequence
  source: /note="Description of Artificial Sequence: Synthetic polypeptide"
AAAPAPRPPTPAPTIASQPLSLRPEACRPAAGGAVHTRGLDFDTALAAVICSALATVLLALLILCVIYCKRQPR

SEQ ID NO: 59 - DNA, 123 bp, Artificial Sequence; identical to SEQ ID NO: 45
  source: /note="Description of Artificial Sequence: Synthetic polynucleotide"

SEQ ID NO: 60 - protein, 41 aa, Artificial Sequence; identical to SEQ ID NO: 46
  source: /note="Description of Artificial Sequence: Synthetic polypeptide"

SEQ ID NO: 61 - DNA, 336 bp, Artificial Sequence
  source: /note="Description of Artificial Sequence: Synthetic polynucleotide"
cgcgtgaaatttagccgcagcgcggatgcgccggcgtatcagcagggccagaaccagctgtataacgaactgaacctgggccgccgcgaagaatatgatgtgctggataaacgccgcggccgcgatccggaaatgggcggcaaaccgcgccgcaaaaacccgcaggaaggcctgtataacgaactgcagaaagataaaatggcggaagcgtatagcgaaattggcatgaaaggcgaacgccgccgcggcaaaggccatgatggcctgtatcagggcctgagcaccgcgaccaaagatacctatgatgcgctgcatatgcaggcgctgccgccgcgc

SEQ ID NO: 62 - protein, 112 aa, Artificial Sequence; identical to SEQ ID NO: 48
  source: /note="Description of Artificial Sequence: Synthetic polypeptide"

SEQ ID NO: 63 - DNA, 93 bp, Artificial Sequence
  source: /note="Description of Artificial Sequence: Synthetic oligonucleotide"
cgcgcgaaacgcagcggcagcggcgcgaccaactttagcctgctgaaacaggcgggcgatgtggaagaaaacccgggcccgcgagcaaagagg

SEQ ID NO: 64 - protein, 31 aa, Artificial Sequence
  source: /note="Description of Artificial Sequence: Synthetic polypeptide"
RAKRSGSGATNFSLLKQAGDVEENPGPRAKR

SEQ ID NO: 65 - DNA, 78 bp, Artificial Sequence
  source: /note="Description of Artificial Sequence: Synthetic oligonucleotide"
agagctaaacgctctgggtctggtgaaggacgaggtagccttcttacgtgcggagacgtggaggaaaacccaggaccc

SEQ ID NO: 66 - protein, 26 aa, Artificial Sequence
  source: /note="Description of Artificial Sequence: Synthetic peptide"
RAKRSGSGEGRGSLLTCGDVEENPGP

SEQ ID NO: 67 - DNA, 1005 bp, Artificial Sequence
  source: /note="Description of Artificial Sequence: Synthetic polynucleotide"
aggaaggtttgcaatggaatcggtataggggagtttaaggattcacttagcataaacgctactaatattaaacacttcaaaaactgtacgagtataagtggagatcttcacattttgccggttgcattccgaggcgattcattcacccacacgccaccgcttgacccacaagaattggatattcttaaaaccgttaaagaaataacggggtttttgctcattcaagcgtggccagaaaatcgcactgacctccatgctttcgagaacctggagattataagaggacgaactaagcagcatggtcaattctcccttgctgtggtcagcctgaacatcaccagtcttggtttgcggtccctcaaggaaatttcagatggagatgtcatcataagcggcaacaagaatttgtgctatgcaaataccataaactggaaaaaactgtttggcacttccggccagaaaaccaagattatttcaaatcggggtgagaacagctgcaaagccaccggccaggtttgtcatgccttgtgctctccggaaggctgttgggggccagaacccagggactgcgtcagttgcagaaacgtctcaagaggccgcgaatgcgttgacaagtgtaacctccttgagggtgagccacgagagtttgttgagaacagcgagtgtatacaatgtcaccctgaatgtttgccccaggctatgaatataacctgcacaggccgcgggcctgataactgcatccagtgtgctcattacatagatggacctcactgtgtgaaaacctgcccggccggagttatgggagaaaacaacactctggtgtggaaatacgctgatgcaggccacgtgtgccacctttgtcacccgaattgtacatatgggtgtaccggtcctggacttgaaggttgccctaccaatggccctaaaatacccagtatcgcaactggcatggtaggcgctcttctcttgctcttggtagttgctctcggcataggtctttttatg

SEQ ID NO: 68 - protein, 335 aa, Artificial Sequence
  source: /note="Description of Artificial Sequence: Synthetic polypeptide"
RKVCNGIGIGEFKDSLSINATNIKHFKNCTSISGDLHILPVAFRGDSFTHTPPLDPQELDILKTVKEITGFLLIQAWPENRTDLHAFENLEIIRGRTKQHGQFSLAVVSLNITSLGLRSLKEISDGDVIISGNKNLCYANTINWKKLFGTSGQKTKIISNRGENSCKATGQVCHALCSPEGCWGPEPRDCVSCRNVSRGRECVDKCNLLEGEPREFVENSECIQCHPECLPQAMNITCTGRGPDNCIQCAHYIDGPHCVKTCPAGVMGENNTLVWKYADAGHVCHLCHPNCTYGCTGPGLEGCPTNGPKIPSIATGMVGALLLLLVVALGIGLFM

SEQ ID NO: 69 - DNA, 1482 bp, Artificial Sequence
  source: /note="Description of Artificial Sequence: Synthetic polynucleotide"
atgcttcttttggtgacttcccttttgctgtgcgagttgccacaccccgccttcctgcttattccccaggtacagctccagcagagtggcccagggctcgtgaagccaagccagacgctgtccctgacttgtgcaatttcaggggattcagtttcatcaaatagcgcggcgtggaattggattcgacaatctccttcccgagggttggaatggcttggacgaacatattacagatccaaatggtataacgactatgcggtatcagtaaagtcaagaataaccattaaccccgacacaagcaagaaccaattctctttgcagcttaactctgtcacgccagaagacacggcagtctattattgcgctcgcgaggtaacgggtgacctggaagacgcttttgacatttgggggcagggtacgatggtgacagtcagttcagggggcggtgggagtgggggagggggtagcggggggggagggtcagacattcagatgacccagtccccttcatccttgtctgcctccgtcggtgacagggtgacaataacatgcagagcaagccaaacaatctggagctatctcaactggtaccagcagcgaccaggaaaagcgccaaacctgctgatttacgctgcttcctccctccaatcaggcgtgcctagtagatttagcggtaggggctccggcaccgattttacgctcactataagctctcttcaagcagaagattttgcgacttattactgccagcagtcctatagtatacctcagactttcggacagggtaccaagttggagattaaggcggccgcaactaccacccctgcccctcggccgccgactccggccccaaccatcgcaagccaacccctctccttgcgccccgaagcttgccgcccggccgcgggtggagccgtgcatacccgggggctggactttgcctgcgatatctacatttgggccccgctggccggcacttgcggcgtgctcctgctgtcgctggtcatcaccctttactgcaagaggggccggaagaagctgctttacatcttcaagcagccgttcatgcggcccgtgcagacgactcaggaagaggacggatgctcgtgcagattccctgaggaggaagaggggggatgcgaactgcgcgtcaagttctcacggtccgccgacgcccccgcatatcaacagggccagaatcagctctacaacgagctgaacctgggaaggagagaggagtacgacgtgctggacaagcgacgcggacgcgacccggagatgggggggaaaccacggcggaaaaaccctcaggaaggactgtacaacgaactccagaaagacaagatggcggaagcctactcagaaatcgggatgaagggagagcggaggaggggaaagggtcacgacgggctgtaccagggactgagcaccgccactaaggatacctacgatgccttgcatatgcaagcactcccaccccgg

SEQ ID NO: 70 - protein, 494 aa, Artificial Sequence
  source: /note="Description of Artificial Sequence: Synthetic polypeptide"
MLLLVTSLLLCELPHPAFLLIPQVQLQQSGPGLVKPSQTLSLTCAISGDSVSSNSAAWNWIRQSPSRGLEWLGRTYYRSKWYNDYAVSVKSRITINPDTSKNQFSLQLNSVTPEDTAVYYCAREVTGDLEDAFDIWGQGTMVTVSSGGGGSGGGGSGGGGSDIQMTQSPSSLSASVGDRVTITCRASQTIWSYLNWYQQRPGKAPNLLIYAASSLQSGVPSRFSGRGSGTDFTLTISSLQAEDFATYYCQQSYSIPQTFGQGTKLEIKAAATTTPAPRPPTPAPTIASQPLSLRPEACRPAAGGAVHTRGLDFACDIYIWAPLAGTCGVLLLSLVITLYCKRGRKKLLYIFKQPFMRPVQTTQEEDGCSCRFPEEEEGGCELRVKFSRSADAPAYQQGQNQLYNELNLGRREEYDVLDKRRGRDPEMGGKPRRKNPQEGLYNELQKDKMAEAYSEIGMKGERRRGKGHDGLYQGLSTATKDTYDALHMQALPPR

SEQ ID NO: 71 - DNA, 1485 bp, Artificial Sequence
  source: /note="Description of Artificial Sequence: Synthetic polynucleotide"
atgcttctcctggtcacctccctgctcctctgcgaactgcctcaccctgccttccttctgattcctgacactgacattcagatgactcagaccacctcttccttgtccgcgtcactgggagacagagtgaccatctcgtgtcgcgcaagccaggatatctccaagtacctgaactggtaccaacagaagcccgacgggactgtgaagctgctgatctaccacacctcacgcctgcacagcggagtgccaagcagattctccggctccggctcgggaaccgattactcgcttaccattagcaacctcgagcaggaggacatcgctacctacttctgccagcaaggaaataccctgccctacaccttcggcggaggaaccaaattggaaatcaccggctccacgagcggctccgggaagcctggttccggggaaggctccactaagggtgaagtgaagctccaggagtccggccccggcctggtggcgccgtcgcaatcactctctgtgacctgtaccgtgtcgggagtgtccctgcctgattacggcgtgagctggattcggcagccgccgcggaagggcctggaatggctgggtgtcatctggggatccgagactacctactacaactcggccctgaagtcccgcctgactatcatcaaagacaactcgaagtcccaggtctttctgaagatgaactccctgcaaactgacgacaccgccatctattactgtgctaagcactactactacggtggaagctatgctatggactactggggccaggggacatccgtgacagtcagctccgcggccgcaactaccacccctgcccctcggccgccgactccggccccaaccatcgcaagccaacccctctccttgcgccccgaagcttgccgcccggccgcgggtggagccgtgcatacccgggggctggactttgcctgcgatatctacatttgggccccgctggccggcacttgcggcgtgctcctgctgtcgctggtcatcaccctttactgcaagaggggccggaagaagctgctttacatcttcaagcagccgttcatgcggcccgtgcagacgactcaggaagaggacggatgctcgtgcagattccctgaggaggaagaggggggatgcgaactgcgcgtcaagttctcacggtccgccgacgcccccgcatatcaacagggccagaatcagctctacaacgagctgaacctgggaaggagagaggagtacgacgtgctggacaagcgacgcggacgcgacccggagatgggggggaaaccacggcggaaaaaccctcaggaaggactgtacaacgaactccagaaagacaagatggcggaagcctactcagaaatcgggatgaagggagagcggaggaggggaaagggtcacgacgggctgtaccagggactgagcaccgccactaaggatacctacgatgccttgcatatgcaagcactcccaccccgg

SEQ ID NO: 72 - protein, 495 aa, Artificial Sequence
  source: /note="Description of Artificial Sequence: Synthetic polypeptide"
MLLLVTSLLLCELPHPAFLLIPDTDIQMTQTTSSLSASLGDRVTISCRASQDISKYLNWYQQKPDGTVKLLIYHTSRLHSGVPSRFSGSGSGTDYSLTISNLEQEDIATYFCQQGNTLPYTFGGGTKLEITGSTSGSGKPGSGEGSTKGEVKLQESGPGLVAPSQSLSVTCTVSGVSLPDYGVSWIRQPPRKGLEWLGVIWGSETTYYNSALKSRLTIIKDNSKSQVFLKMNSLQTDDTAIYYCAKHYYYGGSYAMDYWGQGTSVTVSSAAATTTPAPRPPTPAPTIASQPLSLRPEACRPAAGGAVHTRGLDFACDIYIWAPLAGTCGVLLLSLVITLYCKRGRKKLLYIFKQPFMRPVQTTQEEDGCSCRFPEEEEGGCELRVKFSRSADAPAYQQGQNQLYNELNLGRREEYDVLDKRRGRDPEMGGKPRRKNPQEGLYNELQKDKMAEAYSEIGMKGERRRGKGHDGLYQGLSTATKDTYDALHMQALPPR

SEQ ID NO: 73 - DNA, 1470 bp, Artificial Sequence
  source: /note="Description of Artificial Sequence: Synthetic polynucleotide"
atgcttctcctggtcacctccctgctcctctgcgaactgcctcaccctgccttccttctgattcctgacattcagatgactcagaccacctcttccttgtccgcgtcactgggagacagagtgaccatctcgtgtcgcgcaagccaggatatctccaagtacctgaactggtaccaacagaagcccgacgggactgtgaagctgctgatctaccacacctcacgcctgcacagcggagtgccaagcagattctccggctccggctcgggaaccgattactcgcttaccattagcaacctcgagcaggaggacatcgctacctacttctgccagcaaggaaataccctgccctacaccttcggcggaggaaccaaattggaaatcaccggcggaggaggctccgggggaggaggttccgggggcgggggttccgaagtgaagctccaggagtccggccccggcctggtggcgccgtcgcaatcactctctgtgacctgtaccgtgtcgggagtgtccctgcctgattacggcgtgagctggattcggcagccgccgcggaagggcctggaatggctgggtgtcatctggggatccgagactacctactacaactcggccctgaagtcccgcctgactatcatcaaagacaactcgaagtcccaggtctttctgaagatgaactccctgcaaactgacgacaccgccatctattactgtgctaagcactactactacggtggaagctatgctatggactactgggggcaaggcacttcggtgactgtgtcaagcgcggccgcaactaccacccctgcccctcggccgccgactccggccccaaccatcgcaagccaacccctctccttgcgccccgaagcttgccgcccggccgcgggtggagccgtgcatacccgggggctggactttgcctgcgatatctacatttgggccccgctggccggcacttgcggcgtgctcctgctgtcgctggtcatcaccctttactgcaagaggggccggaagaagctgctttacatcttcaagcagccgttcatgcggcccgtgcagacgactcaggaagaggacggatgctcgtgcagattccctgaggaggaagaggggggatgcgaactgcgcgtcaagttctcacggtccgccgacgcccccgcatatcaacagggccagaatcagctctacaacgagctgaacctgggaaggagagaggagtacgacgtgctggacaagcgacgcggacgcgacccggagatgggggggaaaccacggcggaaaaaccctcaggaaggactgtacaacgaactccagaaagacaagatggcggaagcctactcagaaatcgggatgaagggagagcggaggaggggaaagggtcacgacgggctgtaccagggactgagcaccgccactaaggatacctacgatgccttgcatatgcaagcactcccaccccgg

SEQ ID NO: 74 - protein, 490 aa, Artificial Sequence
  source: /note="Description of Artificial Sequence: Synthetic polypeptide"
MLLLVTSLLLCELPHPAFLLIPDIQMTQTTSSLSASLGDRVTISCRASQDISKYLNWYQQKPDGTVKLLIYHTSRLHSGVPSRFSGSGSGTDYSLTISNLEQEDIATYFCQQGNTLPYTFGGGTKLEITGGGGSGGGGSGGGGSEVKLQESGPGLVAPSQSLSVTCTVSGVSLPDYGVSWIRQPPRKGLEWLGVIWGSETTYYNSALKSRLTIIKDNSKSQVFLKMNSLQTDDTAIYYCAKHYYYGGSYAMDYWGQGTSVTVSSAAATTTPAPRPPTPAPTIASQPLSLRPEACRPAAGGAVHTRGLDFACDIYIWAPLAGTCGVLLLSLVITLYCKRGRKKLLYIFKQPFMRPVQTTQEEDGCSCRFPEEEEGGCELRVKFSRSADAPAYQQGQNQLYNELNLGRREEYDVLDKRRGRDPEMGGKPRRKNPQEGLYNELQKDKMAEAYSEIGMKGERRRGKGHDGLYQGLSTATKDTYDALHMQALPPR

SEQ ID NO: 75 - DNA, 1467 bp, Artificial Sequence
  source: /note="Description of Artificial Sequence: Synthetic polynucleotide"
atgctgctgctggtgaccagcctgctgctgtgcgaactgccgcatccggcgtttctgctgattccggatattcagatgacccagaccaccagcagcctgagcgcgagcctgggcgatcgcgtgaccattagctgccgcgcgagccaggatattagcaaatatctgaactggtatcagcagaaaccggatggcaccgtgaaactgctgatttatcataccagccgcctgcatagcggcgtgccgagccgctttagcggcagcggcagcggcaccgattatagcctgaccattagcaacctggaacaggaagatattgcgacctatttttgccagcagggcaacaccctgccgtatacctttggcggcggcaccaaactggaaattaccggcggcggcggcagcggcggcggcggcagcggcggcggcggcagcgaagtgaaactgcaggaaagcggcccgggcctggtggcgccgagccagagcctgagcgtgacctgcaccgtgagcggcgtgagcctgccggattatggcgtgagctggattcgccagccgccgcgcaaaggcctggaatggctgggcgtgatttggggcagcgaaaccacctattataacagcgcgctgaaaagccgcctgaccattattaaagataacagcaaaagccaggtgtttctgaaaatgaacagcctgcagaccgatgataccgcgatttattattgcgcgaaacattattattatggcggcagctatgcgatggattattggggccagggcaccagcgtgaccgtgagcagcgcggcggcgccggcgccgcgcccgccgaccccggcgccgaccattgcgagccagccgctgagcctgcgcccggaagcgtgccgcccggcggcgggcggcgcggtgcatacccgcggcctggattttgtgcagccgatggcgctgattgtgctgggcggcgtggcgggcctgctgctgtttattggcctgggcatttttttttgcgtgcgctgccgcccgcgccgcaaaaaactgctgtatatttttaaacagccgtttatgcgcccggtgcagaccacccaggaagaagatggctgcagctgccgctttccggaagaagaagaaggcggctgcgaactgcgcgtgaaatttagccgcagcgcggatgcgccggcgtatcagcagggccagaaccagctgtataacgaactgaacctgggccgccgcgaagaatatgatgtgctggataaacgccgcggccgcgatccggaaatgggcggcaaaccgcgccgcaaaaacccgcaggaaggcctgtataacgaactgcagaaagataaaatggcggaagcgtatagcgaaattggcatgaaaggcgaacgccgccgcggcaaaggccatgatggcctgtatcagggcctgagcaccgcgaccaaagatacctatgatgcgctgcatatgcaggcgctgccgccgcgc

SEQ ID NO: 76 - protein, 489 aa, Artificial Sequence
  source: /note="Description of Artificial Sequence: Synthetic polypeptide"
MLLLVTSLLLCELPHPAFLLIPDIQMTQTTSSLSASLGDRVTISCRASQDISKYLNWYQQKPDGTVKLLIYHTSRLHSGVPSRFSGSGSGTDYSLTISNLEQEDIATYFCQQGNTLPYTFGGGTKLEITGGGGSGGGGSGGGGSEVKLQESGPGLVAPSQSLSVTCTVSGVSLPDYGVSWIRQPPRKGLEWLGVIWGSETTYYNSALKSRLTIIKDNSKSQVFLKMNSLQTDDTAIYYCAKHYYYGGSYAMDYWGQGTSVTVSSAAAPAPRPPTPAPTIASQPLSLRPEACRPAAGGAVHTRGLDFVQPMALIVLGGVAGLLLFIGLGIFFCVRCRPRRKKLLYIFKQPFMRPVQTTQEEDGCSCRFPEEEEGGCELRVKFSRSADAPAYQQGQNQLYNELNLGRREEYDVLDKRRGRDPEMGGKPRRKNPQEGLYNELQKDKMAEAYSEIGMKGERRRGKGHDGLYQGLSTATKDTYDALHMQALPPR

SEQ ID NO: 77 - DNA, 1467 bp, Artificial Sequence
  source: /note="Description of Artificial Sequence: Synthetic polynucleotide"
atgctgctgctggtcaccagcctgctgctgtgcgagctccctcaccccgcctttctgcttatcccggacattcagatgacacagaccacctcgagcttgtccgcgtcgctgggcgatcgcgtgaccatctcctgccgggcctcccaagacatttcaaagtatctcaactggtaccagcagaagccggacggaaccgtgaaactgctgatctaccataccagccgcctgcactccggcgtgccgtcccgcttctccggatcgggttccggaactgactactcactgactatctccaacttggaacaagaggacatcgccacttacttctgtcaacaaggaaatacccttccctacaccttcggggggggtaccaagctggagatcactgggggcggaggctccggtggaggcggatccggcggtggagggagcgaagtcaagctgcaggaatcaggaccaggactcgtggcgccatcccagtccctgtcggtgacctgtactgtctccggagtcagcctccccgattacggagtgtcatggattaggcaacccccaagaaaagggctggaatggctcggagtgatctggggctccgaaaccacctactacaactcggcgctgaagtcccggctgaccatcatcaaggacaactccaagagccaagtgttcttgaagatgaacagcttgcagaccgacgataccgcaatctactactgtgccaagcactattactacggggggtcttacgccatggactactggggacagggcacctccgtgactgtgtcgtccgcggccgcgcccgcccctcggcccccgactcctgccccgacgatcgcttcccaacctctctcgctgcgcccggaagcatgccggcccgccgccggtggcgctgtccacactcgcggactggactttgataccgcactggcggccgtgatctgtagcgccctggccaccgtgctgctggcgctgctcatcctttgcgtgatctactgcaagcggcagcctaggcgaaagaagctcctctacattttcaagcaacccttcatgcgccccgtgcaaaccacccaggaggaggatggatgctcatgccggttccctgaggaagaagagggcggttgcgagctcagagtgaaattcagccggtcggctgacgccccggcgtaccagcagggccagaaccagctgtacaatgagctcaacctggggcgccgcgaagagtacgacgtgctggacaagaggagaggcagagatccggaaatgggcggaaagccaaggcggaagaacccgcaggaaggtctttacaacgaactgcagaaggacaagatggccgaggcctactccgagattgggatgaagggagaaagacggaggggaaagggacatgacggactttaccagggcctgagcactgccacgaaggacacctatgatgccctgcacatgcaggcgctgccgcctcgg

SEQ ID NO: 78 - protein, 489 aa, Artificial Sequence
  source: /note="Description of Artificial Sequence: Synthetic polypeptide"
MLLLVTSLLLCELPHPAFLLIPDIQMTQTTSSLSASLGDRVTISCRASQDISKYLNWYQQKPDGTVKLLIYHTSRLHSGVPSRFSGSGSGTDYSLTISNLEQEDIATYFCQQGNTLPYTFGGGTKLEITGGGGSGGGGSGGGGSEVKLQESGPGLVAPSQSLSVTCTVSGVSLPDYGVSWIRQPPRKGLEWLGVIWGSETTYYNSALKSRLTIIKDNSKSQVFLKMNSLQTDDTAIYYCAKHYYYGGSYAMDYWGQGTSVTVSSAAAPAPRPPTPAPTIASQPLSLRPEACRPAAGGAVHTRGLDFDTALAAVICSALATVLLALLILCVIYCKRQPRRKKLLYIFKQPFMRPVQTTQEEDGCSCRFPEEEEGGCELRVKFSRSADAPAYQQGQNQLYNELNLGRREEYDVLDKRRGRDPEMGGKPRRKNPQEGLYNELQKDKMAEAYSEIGMKGERRRGKGHDGLYQGLSTATKDTYDALHMQALPPR

SEQ ID NO: 79 - DNA, 36 bp, Homo sapiens
gagagcaaatacgggccgccatgtcccccgtgtccg

SEQ ID NO: 80 - protein, 12 aa, Homo sapiens
ESKYGPPCPPCP

SEQ ID NO: 81 - DNA, 327 bp, Homo sapiens
gcaccaccagttgctggccctagtgtcttcttgttccctcccaagcccaaagacaccttgatgatttccagaactcctgaggttacctgcgttgtcgtagatgtttctcaggaggacccagaggtccaatttaactggtacgttgatggggtggaagttcacaatgcgaagacaaagccgcgggaagaacaatttcagtccacttaccgggttgtcagcgttctgacggtattgcatcaagactggcttaatggaaaggaatataagtgtaaggtgtccaacaaaggtttgccgagcagtattgagaagaccatatcaaaggcgaag

SEQ ID NO: 82 - protein, 109 aa, Homo sapiens
APPVAGPSVFLFPPKPKDTLMISRTPEVTCVVVDVSQEDPEVQFNWYVDGVEVHNAKTKPREEQFQSTYRVVSVLTVLHQDWLNGKEYKCKVSNKGLPSSIEKTISKAK

SEQ ID NO: 83 - DNA, 321 bp, Homo sapiens
gggcagccgcgcgagccacaagtttacactttgccgccatctcaagaggaaatgactaaaaaccaggtatccttgacatgcctcgtaaaaggattttatccatctgatattgctgtggaatgggagtctaacgggcagccggaaaataattacaaaactacaccacctgtgctcgattcagatggaagtttcttcctttacagtagacttacggtggacaaatctaggtggcaggaagggaatgtgtttagttgtagtgtaatgcacgaggcacttcataaccactatacacagaagtcactgagtttgagtcttggcaaa

SEQ ID NO: 84 - protein, 107 aa, Homo sapiens
GQPREPQVYTLPPSQEEMTKNQVSLTCLVKGFYPSDIAVEWESNGQPENNYKTTPPVLDSDGSFFLYSRLTVDKSRWQEGNVFSCSVMHEALHNHYTQKSLSLSLGK

SEQ ID NO: 85 - DNA, 684 bp, Homo sapiens
gagagcaaatacgggccgccatgtcccccgtgtccggcaccaccagttgctggccctagtgtcttcttgttccctcccaagcccaaagacaccttgatgatttccagaactcctgaggttacctgcgttgtcgtagatgtttctcaggaggacccagaggtccaatttaactggtacgttgatggggtggaagttcacaatgcgaagacaaagccgcgggaagaacaatttcagtccacttaccgggttgtcagcgttctgacggtattgcatcaagactggcttaatggaaaggaatataagtgtaaggtgtccaacaaaggtttgccgagcagtattgagaagaccatatcaaaggcgaaggggcagccgcgcgagccacaagtttacactttgccgccatctcaagaggaaatgactaaaaaccaggtatccttgacatgcctcgtaaaaggattttatccatctgatattgctgtggaatgggagtctaacgggcagccggaaaataattacaaaactacaccacctgtgctcgattcagatggaagtttcttcctttacagtagacttacggtggacaaatctaggtggcaggaagggaatgtgtttagttgtagtgtaatgcacgaggcacttcataaccactatacacagaagtcactgagtttgagtcttggcaaa

SEQ ID NO: 86 - protein, 228 aa, Homo sapiens
ESKYGPPCPPCPAPPVAGPSVFLFPPKPKDTLMISRTPEVTCVVVDVSQEDPEVQFNWYVDGVEVHNAKTKPREEQFQSTYRVVSVLTVLHQDWLNGKEYKCKVSNKGLPSSIEKTISKAKGQPREPQVYTLPPSQEEMTKNQVSLTCLVKGFYPSDIAVEWESNGQPENNYKTTPPVLDSDGSFFLYSRLTVDKSRWQEGNVFSCSVMHEALHNHYTQKSLSLSLGK

SEQ ID NO: 87 - DNA, 732 bp, Artificial Sequence
  source: /note="Description of Artificial Sequence: Synthetic polynucleotide"
gaggtccagctggtacagtctgggggaggcttggtacagcctggggggtccctgagactctcctgtgcagcctctggattcacctttgatgattatgccatgcactgggtccggcaagctccagggaagggcctggagtgggtctcaggtattagttggaatagtggtagcataggctatgcggactctgtgaagggccgattcaccatctccagagacaacgccaagaactccctgtatctgcaaatgaacagtctgagagctgaggacacggccttgtattactgtgcaaaagatttatcgtcagtggctggaccctttaactactggggccagggcaccctggtcaccgtctcctcaggaggtggcgggtctggtggaggcggtagcggcggtggcggatcctcttctgagctgactcaggaccctgctgtgtctgtggccttgggacagacagtcaggatcacatgccaaggagacagcctcagaagctattatgcaagctggtaccagcagaagccaggacaggcccctgtacttgtcatctatggtaaaaacaaccggccctcagggatcccagaccgattctctggctccagctcaggaaacacagcttccttgaccatcactggggctcaggcggaggatgaggctgactattactgtaactcccgggacagcagtggtaaccatctggtattcggcggaggcacccagctgaccgtcctcggt

SEQ ID NO: 88 - protein, 244 aa, Artificial Sequence
  source: /note="Description of Artificial Sequence: Synthetic polypeptide"
EVQLVQSGGGLVQPGGSLRLSCAASGFTFDDYAMHWVRQAPGKGLEWVSGISWNSGSIGYADSVKGRFTISRDNAKNSLYLQMNSLRAEDTALYYCAKDLSSVAGPFNYWGQGTLVTVSSGGGGSGGGGSGGGGSSSELTQDPAVSVALGQTVRITCQGDSLRSYYASWYQQKPGQAPVLVIYGKNNRPSGIPDRFSGSSSGNTASLTITGAQAEDEADYYCNSRDSSGNHLVFGGGTQLTVLG

SEQ ID NO: 89 - DNA, 1476 bp, Artificial Sequence
  source: /note="Description of Artificial Sequence: Synthetic polynucleotide"
atgctgctgctggtgaccagcctgctgctgtgcgaactgccgcatccggcgtttctgctgattccggaggtccagctggtacagtctgggggaggcttggtacagcctggggggtccctgagactctcctgtgcagcctctggattcacctttgatgattatgccatgcactgggtccggcaagctccagggaagggcctggagtgggtctcaggtattagttggaatagtggtagcataggctatgcggactctgtgaagggccgattcaccatctccagagacaacgccaagaactccctgtatctgcaaatgaacagtctgagagctgaggacacggccttgtattactgtgcaaaagatttatcgtcagtggctggaccctttaactactggggccagggcaccctggtcaccgtctcctcaggaggtggcgggtctggtggaggcggtagcggcggtggcggatcctcttctgagctgactcaggaccctgctgtgtctgtggccttgggacagacagtcaggatcacatgccaaggagacagcctcagaagctattatgcaagctggtaccagcagaagccaggacaggcccctgtacttgtcatctatggtaaaaacaaccggccctcagggatcccagaccgattctctggctccagctcaggaaacacagcttccttgaccatcactggggctcaggcggaggatgaggctgactattactgtaactcccgggacagcagtggtaaccatctggtattcggcggaggcacccagctgaccgtcctcggtgcggccgcaactaccacccctgcccctcggccgccgactccggccccaaccatcgcaagccaacccctctccttgcgccccgaagcttgccgcccggccgcgggtggagccgtgcatacccgggggctggactttgcctgcgatatctacatttgggccccgctggccggcacttgcggcgtgctcctgctgtcgctggtcatcaccctttactgcaagaggggccggaagaagctgctttacatcttcaagcagccgttcatgcggcccgtgcagacgactcaggaagaggacggatgctcgtgcagattccctgaggaggaagaggggggatgcgaactgcgcgtcaagttctcacggtccgccgacgcccccgcatatcaacagggccagaatcagctctacaacgagctgaacctgggaaggagagaggagtacgacgtgctggacaagcgacgcggacgcgacccggagatgggggggaaaccacggcggaaaaaccctcaggaaggactgtacaacgaactccagaaagacaagatggcggaagcctactcagaaatcgggatgaagggagagcggaggaggggaaagggtcacgacgggctgtaccagggactgagcaccgccactaaggatacctacgatgccttgcatatgcaagcactcccaccccgg

SEQ ID NO: 90 - protein, 492 aa, Artificial Sequence
  source: /note="Description of Artificial Sequence: Synthetic polypeptide"
MLLLVTSLLLCELPHPAFLLIPEVQLVQSGGGLVQPGGSLRLSCAASGFTFDDYAMHWVRQAPGKGLEWVSGISWNSGSIGYADSVKGRFTISRDNAKNSLYLQMNSLRAEDTALYYCAKDLSSVAGPFNYWGQGTLVTVSSGGGGSGGGGSGGGGSSSELTQDPAVSVALGQTVRITCQGDSLRSYYASWYQQKPGQAPVLVIYGKNNRPSGIPDRFSGSSSGNTASLTITGAQAEDEADYYCNSRDSSGNHLVFGGGTQLTVLGAAATTTPAPRPPTPAPTIASQPLSLRPEACRPAAGGAVHTRGLDFACDIYIWAPLAGTCGVLLLSLVITLYCKRGRKKLLYIFKQPFMRPVQTTQEEDGCSCRFPEEEEGGCELRVKFSRSADAPAYQQGQNQLYNELNLGRREEYDVLDKRRGRDPEMGGKPRRKNPQEGLYNELQKDKMAEAYSEIGMKGERRRGKGHDGLYQGLSTATKDTYDALHMQALPPR

SEQ ID NO: 91 - DNA, 339 bp, Artificial Sequence
  source: /note="Description of Artificial Sequence: Synthetic polynucleotide"
gaggtgcagctggtggagtctgggggaggcttggtacagcctggagggtccctgagactctcctgtgcagcctctggattcaccttcagtagctatggcatgagctgggtccgccaggctccaagacaagggcttgagtgggtggccaacataaagcaagatggaagtgagaaatactatgcggactcagtgaagggccgattcaccatctccagagacaattccaagaacacgctgtatctgcaaatgaacagcctgagagccgaggacacagccacgtattactgtgcgaaagaaaatgtggactggggccagggcaccctggtcaccgtctcctca

SEQ ID NO: 92 - protein, 113 aa, Artificial Sequence
  source: /note="Description of Artificial Sequence: Synthetic polypeptide"
EVQLVESGGGLVQPGGSLRLSCAASGFTFSSYGMSWVRQAPRQGLEWVANIKQDGSEKYYADSVKGRFTISRDNSKNTLYLQMNSLRAEDTATYYCAKENVDWGQGTLVTVSS

SEQ ID NO: 93 - DNA, 1083 bp, Artificial Sequence
  source: /note="Description of Artificial Sequence: Synthetic polynucleotide"
atgctgctgctggtgaccagcctgctgctgtgcgaactgccgcatccggcgtttctgctgattccggaggtgcagctggtggagtctgggggaggcttggtacagcctggagggtccctgagactctcctgtgcagcctctggattcaccttcagtagctatggcatgagctgggtccgccaggctccaagacaagggcttgagtgggtggccaacataaagcaagatggaagtgagaaatactatgcggactcagtgaagggccgattcaccatctccagagacaattccaagaacacgctgtatctgcaaatgaacagcctgagagccgaggacacagccacgtattactgtgcgaaagaaaatgtggactggggccagggcaccctggtcaccgtctcctcagcggccgcaactaccacccctgcccctcggccgccgactccggccccaaccatcgcaagccaacccctctccttgcgccccgaagcttgccgcccggccgcgggtggagccgtgcatacccgggggctggactttgcctgcgatatctacatttgggccccgctggccggcacttgcggcgtgctcctgctgtcgctggtcatcaccctttactgcaagaggggccggaagaagctgctttacatcttcaagcagccgttcatgcggcccgtgcagacgactcaggaagaggacggatgctcgtgcagattccctgaggaggaagaggggggatgcgaactgcgcgtcaagttctcacggtccgccgacgcccccgcatatcaacagggccagaatcagctctacaacgagctgaacctgggaaggagagaggagtacgacgtgctggacaagcgacgcggacgcgacccggagatgggggggaaaccacggcggaaaaaccctcaggaaggactgtacaacgaactccagaaagacaagatggcggaagcctactcagaaatcgggatgaagggagagcggaggaggggaaagggtcacgacgggctgtaccagggactgagcaccgccactaaggatacctacgatgccttgcatatgcaagcactcccaccccgg

SEQ ID NO: 94 - protein, 361 aa, Artificial Sequence
  source: /note="Description of Artificial Sequence: Synthetic polypeptide"
MLLLVTSLLLCELPHPAFLLIPEVQLVESGGGLVQPGGSLRLSCAASGFTFSSYGMSWVRQAPRQGLEWVANIKQDGSEKYYADSVKGRFTISRDNSKNTLYLQMNSLRAEDTATYYCAKENVDWGQGTLVTVSSAAATTTPAPRPPTPAPTIASQPLSLRPEACRPAAGGAVHTRGLDFACDIYIWAPLAGTCGVLLLSLVITLYCKRGRKKLLYIFKQPFMRPVQTTQEEDGCSCRFPEEEEGGCELRVKFSRSADAPAYQQGQNQLYNELNLGRREEYDVLDKRRGRDPEMGGKPRRKNPQEGLYNELQKDKMAEAYSEIGMKGERRRGKGHDGLYQGLSTATKDTYDALHMQALPPR

SEQ ID NO: 95 - DNA, 2283 bp, Artificial Sequence
  source: /note="Description of Artificial Sequence: Synthetic polynucleotide"
atgctccttctcgtgacctccctgcttctctgcgaactgccccatcctgccttcctgctgattcccgacattcagatgactcagaccacctcctccctgtccgcctccctgggcgaccgcgtgaccatctcatgccgcgccagccaggacatctcgaagtacctcaactggtaccagcagaagcccgacggaaccgtgaagctcctgatctaccacacctcccggctgcacagcggagtgccgtctagattctcgggttcggggtcgggaactgactactcccttactatttccaacctggagcaggaggatattgccacctacttctgccaacaaggaaacaccctgccgtacacttttggcgggggaaccaagctggaaatcactggcagcacatccggttccgggaagcccggctccggagagggcagcaccaagggggaagtcaagctgcaggaatcaggacctggcctggtggccccgagccagtcactgtccgtgacttgtactgtgtccggagtgtcgctcccggattacggagtgtcctggatcaggcagccacctcggaaaggattggaatggctcggagtcatctggggttccgaaaccacctattacaactcggcactgaaatccaggctcaccattatcaaggataactccaagtcacaagtgttcctgaagatgaatagcctgcagactgacgacacggcgatctactattgcgccaagcactactactacggcggatcctacgctatggactactggggccaggggaccagcgtgaccgtgtcatccggaggcggcggcagcggcgggggagggtccggagggggtggttctggtggaggaggatcgggaggcggtggcagcgaggtgcagttgcaacagtcaggagctgaactggtcaagccaggagccagcgtgaagatgagctgcaaggcctccggttacaccttcacctcctacaacatgcactgggtgaaacagaccccgggacaagggctcgaatggattggcgccatctaccccgggaatggcgatacttcgtacaaccagaagttcaagggaaaggccaccctgaccgccgacaagagctcctccaccgcgtatatgcagttgagctccctgacctccgaggactccgccgactactactgcgcacggtccaactactatggaagctcgtactggttcttcgatgtctggggggccggcaccactgtgaccgtcagctccgggggcggaggatccggtggaggcggaagcgggggtggaggatccgacattgtgctgactcagtccccggcaatcctgtcggcctcaccgggcgaaaaggtcacgatgacttgtagagcgtcgtccagcgtgaactacatggattggtaccaaaagaagcctggatcgtcacccaagccttggatctacgctacatctaacctggcctccggcgtgccagcgcggttcagcgggtccggctcgggcacctcatactcgctgaccatctcccgcgtggaggctgaggacgccgcgacctactactgccagcagtggtccttcaacccgccgacttttggaggcggtactaagctggagatcaaagcggccgcaactaccacccctgcccctcggccgccgactccggccccaaccatcgcaagccaacccctctccttgcgccccgaagcttgccgcccggccgcgggtggagccgtgcatacccgggggctggactttgcctgcgatatctacatttgggccccgctggccggcacttgcggcgtgctcctgctgtcgctggtcatcaccctttactgcaagaggggccggaagaagctgctttacatcttcaagcagccgttcatgcggcccgtgcagacgactcaggaagaggacggatgctcgtgcagattccctgaggaggaagaggggggatgcgaactgcgcgtcaagttctcacggtccgccgacgcccccgcatatcaacagggccagaatcagctctacaacgagctgaacctgggaaggagagaggagtacgacgtgctggacaagcgacgcggacgcgacccggagatgggggggaaaccacggcggaaaaaccctcaggaaggactgtacaacgaactccagaaagacaagatggcggaagcctactcagaaatcgggatgaagggagagcggaggaggggaaagggtcacgacgggctgtaccagggactgagcaccgccactaaggatacctacgatgccttgcatatgcaagcactcccaccccgg

SEQ ID NO: 96 - protein, 761 aa, Artificial Sequence
  source: /note="Description of Artificial Sequence: Synthetic polypeptide"
MLLLVTSLLLCELPHPAFLLIPDIQMTQTTSSLSASLGDRVTISCRASQDISKYLNWYQQKPDGTVKLLIYHTSRLHSGVPSRFSGSGSGTDYSLTISNLEQEDIATYFCQQGNTLPYTFGGGTKLEITGSTSGSGKPGSGEGSTKGEVKLQESGPGLVAPSQSLSVTCTVSGVSLPDYGVSWIRQPPRKGLEWLGVIWGSETTYYNSALKSRLTIIKDNSKSQVFLKMNSLQTDDTAIYYCAKHYYYGGSYAMDYWGQGTSVTVSSGGGGSGGGGSGGGGSGGGGSGGGGSEVQLQQSGAELVKPGASVKMSCKASGYTFTSYNMHWVKQTPGQGLEWIGAIYPGNGDTSYNQKFKGKATLTADKSSSTAYMQLSSLTSEDSADYYCARSNYYGSSYWFFDVWGAGTTVTVSSGGGGSGGGGSGGGGSDIVLTQSPAILSASPGEKVTMTCRASSSVNYMDWYQKKPGSSPKPWIYATSNLASGVPARFSGSGSGTSYSLTISRVEAEDAATYYCQQWSFNPPTFGGGTKLEIKAAATTTPAPRPPTPAPTIASQPLSLRPEACRPAAGGAVHTRGLDFACDIYIWAPLAGTCGVLLLSLVITLYCKRGRKKLLYIFKQPFMRPVQTTQEEDGCSCRFPEEEEGGCELRVKFSRSADAPAYQQGQNQLYNELNLGRREEYDVLDKRRGRDPEMGGKPRRKNPQEGLYNELQKDKMAEAYSEIGMKGERRRGKGHDGLYQGLSTATKDTYDALHMQALPPR

SEQ ID NO: 97 - DNA, 2283 bp, Artificial Sequence
  source: /note="Description of Artificial Sequence: Synthetic polynucleotide"
atgctccttctcgtgacctccctgcttctctgcgaactgccccatcctgccttcctgctgattcccgaggtgcagttgcaacagtcaggagctgaactggtcaagccaggagccagcgtgaagatgagctgcaaggcctccggttacaccttcacctcctacaacatgcactgggtgaaacagaccccgggacaagggctcgaatggattggcgccatctaccccgggaatggcgatacttcgtacaaccagaagttcaagggaaaggccaccctgaccgccgacaagagctcctccaccgcgtatatgcagttgagctccctgacctccgaggactccgccgactactactgcgcacggtccaactactatggaagctcgtactggttcttcgatgtctggggggccggcaccactgtgaccgtcagctccgggggcggaggatccggtggaggcggaagcgggggtggaggatccgacattgtgctgactcagtccccggcaatcctgtcggcctcaccgggcgaaaaggtcacgatgacttgtagagcgtcgtccagcgtgaactacatggattggtaccaaaagaagcctggatcgtcacccaagccttggatctacgctacatctaacctggcctccggcgtgccagcgcggttcagcgggtccggctcgggcacctcatactcgctgaccatctcccgcgtggaggctgaggacgccgcgacctactactgccagcagtggtccttcaacccgccgacttttggaggcggtactaagctggagatcaaaggaggcggcggcagcggcgggggagggtccggagggggtggttctggtggaggaggatcgggaggcggtggcagcgacattcagatgactcagaccacctcctccctgtccgcctccctgggcgaccgcgtgaccatctcatgccgcgccagccaggacatctcgaagtacctcaactggtaccagcagaagcccgacggaaccgtgaagctcctgatctaccacacctcccggctgcacagcggagtgccgtctagattctcgggttcggggtcgggaactgactactcccttactatttccaacctggagcaggaggatattgccacctacttctgccaacaaggaaacaccctgccgtacacttttggcgggggaaccaagctggaaatcactggcagcacatccggttccgggaagcccggctccggagagggcagcaccaagggggaagtcaagctgcaggaatcaggacctggcctggtggccccgagccagtcactgtccgtgacttgtactgtgtccggagtgtcgctcccggattacggagtgtcctggatcaggcagccacctcggaaaggattggaatggctcggagtcatctggggttccgaaaccacctattacaactcggcactgaaatccaggctcaccattatcaaggataactccaagtcacaagtgttcctgaagatgaatagcctgcagactgacgacacggcgatctactattgcgccaagcactactactacggcggatcctacgctatggactactggggccaggggaccagcgtgaccgtgtcatccgcggccgcaactaccacccctgcccctcggccgccgactccggccccaaccatcgcaagccaacccctctccttgcgccccgaagcttgccgcccggccgcgggtggagccgtgcatacccgggggctggactttgcctgcgatatctacatttgggccccgctggccggcacttgcggcgtgctcctgctgtcgctggtcatcaccctttactgcaagaggggccggaagaagctgctttacatcttcaagcagccgttcatgcggcccgtgcagacgactcaggaagaggacggatgctcgtgcagattccctgaggaggaagaggggggatgcgaactgcgcgtcaagttctcacggtccgccgacgcccccgcatatcaacagggccagaatcagctctacaacgagctgaacctgggaaggagagaggagtacgacgtgctggacaagcgacgcggacgcgacccggagatgggggggaaaccacggcggaaaaaccctcaggaaggactgtacaacgaactccagaaagacaagatggcggaagcctactcagaaatcgggatgaagggagagcggaggaggggaaagggtcacgacgggctgtaccagggactgagcaccgccactaaggatacctacgatgccttgcatatgcaagcactcccaccccgg

SEQ ID NO: 98 - protein, 761 aa, Artificial Sequence
  source: /note="Description of Artificial Sequence: Synthetic polypeptide"
MLLLVTSLLLCELPHPAFLLIPEVQLQQSGAELVKPGASVKMSCKASGYTFTSYNMHWVKQTPGQGLEWIGAIYPGNGDTSYNQKFKGKATLTADKSSSTAYMQLSSLTSEDSADYYCARSNYYGSSYWFFDVWGAGTTVTVSSGGGGSGGGGSGGGGSDIVLTQSPAILSASPGEKVTMTCRASSSVNYMDWYQKKPGSSPKPWIYATSNLASGVPARFSGSGSGTSYSLTISRVEAEDAATYYCQQWSFNPPTFGGGTKLEIKGGGGSGGGGSGGGGSGGGGSGGGGSDIQMTQTTSSLSASLGDRVTISCRASQDISKYLNWYQQKPDGTVKLLIYHTSRLHSGVPSRFSGSGSGTDYSLTISNLEQEDIATYFCQQGNTLPYTFGGGTKLEITGSTSGSGKPGSGEGSTKGEVKLQESGPGLVAPSQSLSVTCTVSGVSLPDYGVSWIRQPPRKGLEWLGVIWGSETTYYNSALKSRLTIIKDNSKSQVFLKMNSLQTDDTAIYYCAKHYYYGGSYAMDYWGQGTSVTVSSAAATTTPAPRPPTPAPTIASQPLSLRPEACRPAAGGAVHTRGLDFACDIYIWAPLAGTCGVLLLSLVITLYCKRGRKKLLYIFKQPFMRPVQTTQEEDGCSCRFPEEEEGGCELRVKFSRSADAPAYQQGQNQLYNELNLGRREEYDVLDKRRGRDPEMGGKPRRKNPQEGLYNELQKDKMAEAYSEIGMKGERRRGKGHDGLYQGLSTATKDTYDALHMQALPPR

SEQ ID NO: 99 - DNA, 797 bp, Artificial Sequence
  source: /note="Description of Artificial Sequence: Synthetic polynucleotide"
atggcactgcccgtgaccgccctgcttctgccgcttgcacttctgctgcacgccgctaggccccaagtcaccctcaaagagtcagggccaggaatcctcaagccctcacagactctgtctcttacttgctcattcagcggattcagcctttccacctctggtatgggcgtggggtggattaggcaacctagcggaaaggggcttgaatggctggcccacatctggtgggacgacgacaagtactacaacccctcactgaagtcccagctcactatttccaaagatacttcccggaatcaggtgttcctcaagattacctctgtcgacaccgctgataccgccacttactattgttcacgcagaccgagaggtaccatggacgcaatggactactggggacagggcaccagcgtgaccgtgtcatctggcggtggagggtcaggaggtggaggtagcggaggcggtgggtccgacattgtcatgacccaggccgccagcagcctgagcgcttcactgggcgacagggtgaccatcagctgtcgcgcatcacaagatatctctaagtatcttaattggtaccagcaaaagccggatggaaccgtgaagctgctgatctactacacctcacggctgcattctggagtgcctagccgctttagcggatctgggtccggtactgactacagcctcaccattagaaaccttgaacaggaggacatcgcaacttatttctgccaacaggtctatactctgccgtggaccttcggcggaggtaccaaactggagattaagtccgg

SEQ ID NO: 100 - protein, 265 aa, Artificial Sequence
  source: /note="Description of Artificial Sequence: Synthetic polypeptide"
MALPVTALLLPLALLLHAARPQVTLKESGPGILKPSQTLSLTCSFSGFSLSTSGMGVGWIRQPSGKGLEWLAHIWWDDDKYYNPSLKSQLTISKDTSRNQVFLKITSVDTADTATYYCSRRPRGTMDAMDYWGQGTSVTVSSGGGGSGGGGSGGGGSDIVMTQAASSLSASLGDRVTISCRASQDISKYLNWYQQKPDGTVKLLIYYTSRLHSGVPSRFSGSGSGTDYSLTIRNLEQEDIATYFCQQVYTLPWTFGGGTKLEIKS

SEQ ID NO: 101 - DNA, 1170 bp, Artificial Sequence
  source: /note="Description of Artificial Sequence: Synthetic polynucleotide"
atggcactgcccgtgaccgccctgcttctgccgcttgcacttctgctgcacgccgctaggccccaagtcaccctcaaagagtcagggccaggaatcctcaagccctcacagactctgtctcttacttgctcattcagcggattcagcctttccacctctggtatgggcgtggggtggattaggcaacctagcggaaaggggcttgaatggctggcccacatctggtgggacgacgacaagtactacaacccctcactgaagtcccagctcactatttccaaagatacttcccggaatcaggtgttcctcaagattacctctgtcgacaccgctgataccgccacttactattgttcacgcagaccgagaggtaccatggacgcaatggactactggggacagggcaccagcgtgaccgtgtcatctggcggtggagggtcaggaggtggaggtagcggaggcggtgggtccgacattgtcatgacccaggccgccagcagcctgagcgcttcactgggcgacagggtgaccatcagctgtcgcgcatcacaagatatctctaagtatcttaattggtaccagcaaaagccggatggaaccgtgaagctgctgatctactacacctcacggctgcattctggagtgcctagccgctttagcggcacttgcggcgtgctcctgctgtcgctggtcatcaccctttactgcaagaggggccggaagaagctgctttacatcttcaagcagccgttcatgcggcccgtgcagacgactcaggaagaggacggatgctcgtgcagattccctgaggaggaagaggggggatgcgaactgcgcgtcaagttctcacggtccgccgacgcccccgcatatcaacagggccagaatcagctctacaacgagctgaacctgggaaggagagaggagtacgacgtgctggacaagcgacgcggacgcgacccggagatgggggggaaaccacggcggaaaaaccctcaggaaggactgtacaacgaactccagaaagacaagatggcggaagcctactcagaaatcgggatgaagggagagcggaggaggggaaagggtcacgacgggctgtaccagggactgagcaccgccactaaggatacctacgatgccttgcatatgcaagcactcccaccccgg

SEQ ID NO: 102 - protein, 490 aa, Artificial Sequence
  source: /note="Description of Artificial Sequence: Synthetic polypeptide"
MALPVTALLLPLALLLHAARPQVTLKESGPGILKPSQTLSLTCSFSGFSLSTSGMGVGWIRQPSGKGLEWLAHIWWDDDKYYNPSLKSQLTISKDTSRNQVFLKITSVDTADTATYYCSRRPRGTMDAMDYWGQGTSVTVSSGGGGSGGGGSGGGGSDIVMTQAASSLSASLGDRVTISCRASQDISKYLNWYQQKPDGTVKLLIYYTSRLHSGVPSRFSGSGSGTDYSLTIRNLEQEDIATYFCQQVYTLPWTFGGGTKLEIKAAATTTPAPRPPTPAPTIASQPLSLRPEACRPAAGGAVHTRGLDFACDIYIWAPLAGTCGVLLLSLVITLYCKRGRKKLLYIFKQPFMRPVQTTQEEDGCSCRFPEEEEGGCELRVKFSRSADAPAYQQGQNQLYNELNLGRREEYDVLDKRRGRDPEMGGKPRRKNPQEGLYNELQKDKMAEAYSEIGMKGERRRGKGHDGLYQGLSTATKDTYDALHMQALPPR

SEQ ID NO: 103 - DNA, 2366 bp, Artificial Sequence
  source: /note="Description of Artificial Sequence: Synthetic polynucleotide"
tgagctctgagtcagtgactcagtgagtcagtgactcagtgagtcagtgactcagctcgaggatctcgctagcgggaatttccggggactttccgggaatttccggggactttccgggaatttccagatctggcctcggcggccaagcttagacactagagggtatataatggaagctcgacttccagcttggcaatccggtactgttggtaaaggcgcgccccaccatgctgctgctggtcaccagcctgctgctgtgcgagctccctcaccccgcctttctgcttatcccggacattcagatgacacagaccacctcgagcttgtccgcgtcgctgggcgatcgcgtgaccatctcctgccgggcctcccaagacatttcaaagtatctcaactggtaccagcagaagccggacggaaccgtgaaactgctgatctaccataccagccgcctgcactccggcgtgccgtcccgcttctccggatcgggttccggaactgactactcactgactatctccaacttggaacaagaggacatcgccacttacttctgtcaacaaggaaatacccttccctacaccttcggggggggtaccaagctggagatcactgggggcggaggctccggtggaggcggatccggcggtggagggagcgaagtcaagctgcaggaatcaggaccaggactcgtggcgccatcccagtccctgtcggtgacctgtactgtctccggagtcagcctccccgattacggagtgtcatggattaggcaacccccaagaaaagggctggaatggctcggagtgatctggggctccgaaaccacctactacaactcggcgctgaagtcccggctgaccatcatcaaggacaactccaagagccaagtgttcttgaagatgaacagcttgcagaccgacgataccgcaatctactactgtgccaagcactattactacggggggtcttacgccatggactactggggacagggcacctccgtgactgtgtcgtccgcggccgctaccacaacccctgcgccccggcctcctacccccgcacccacgattgcttctcaacctctttcactccgacctgaggcttgtagacctgcagccgggggtgccgtccacacacggggactcgacttcgcttgtgatatatatatttgggcgcccctggccggcacttgtggagttcttttgctctctcttgttatcacattgtactgcaagcgaggtaggaagaaattgctttacatttttaagcagccgttcatgcgaccagtacagactactcaagaagaagatgggtgctcttgtcggttcccggaagaagaagagggtggttgcgagttgagggtgaagttctcccgctctgccgacgcaccggcatatcagcagggacaaaaccagctctacaacgaattgaacctgggtcggcgggaagaatatgacgtgctcgataagcggcggggtcgcgacccagaaatgggaggcaaaccgcgcaggaaaaatccacaggagggactttataacgaacttcaaaaggataagatggcagaggcatacagcgaaatcgggatgaaaggcgagagaagaagggggaaagggcacgatggtctttaccaggggctttctaccgcgacgaaggatacctacgatgctctccatatgcaagcacttcctcctagacgggcaaagcggggctcaggggcgactaacttttcactgttgaagcaggccggggatgtggaggagaatcctggtcctagagctaagcgagtagacatgggaagagggctgctccgaggcttgtggccgttgcatattgtattgtggacgcggatagcgagtacaatcccgcctcacgtgcaaaaatcagttaataacgacatgatcgttactgacaacaatggcgcagttaaatttccgcagctttgtaaattctgtgatgtaagattttcaacgtgcgataaccagaaaagctgtatgtccaactgcagcatcacatcaatctgtgaaaaaccccaagaggtatgtgtggccgtctggcgaaagaatgacgaaaatatcacactggagaccgtttgtcacgatcctaaactcccttatcatgactttattctggaagacgcagcgtcaccgaagtgtataatgaaagagaagaagaagcctggagagacgtttttcatgtgcagttgctcctcagatgagtgtaatgacaacatcattttttccgaggagtacaatacgagtaacccagacctcctgctggttattttccaggtaaccggcatcagtttgttgcccccactgggtgttgcaatcagtgtaataatcatattttattgttaccgggtg

SEQ ID NO: 104 - protein, 713 aa, Artificial Sequence
  source: /note="Description of Artificial Sequence: Synthetic polypeptide"
MLLLVTSLLLCELPHPAFLLIPDIQMTQTTSSLSASLGDRVTISCRASQDISKYLNWYQQKPDGTVKLLIYHTSRLHSGVPSRFSGSGSGTDYSLTISNLEQEDIATYFCQQGNTLPYTFGGGTKLEITGGGGSGGGGSGGGGSEVKLQESGPGLVAPSQSLSVTCTVSGVSLPDYGVSWIRQPPRKGLEWLGVIWGSETTYYNSALKSRLTIIKDNSKSQVFLKMNSLQTDDTAIYYCAKHYYYGGSYAMDYWGQGTSVTVSSAAATTTPAPRPPTPAPTIASQPLSLRPEACRPAAGGAVHTRGLDFACDIYIWAPLAGTCGVLLLSLVITLYCKRGRKKLLYIFKQPFMRPVQTTQEEDGCSCRFPEEEEGGCELRVKFSRSADAPAYQQGQNQLYNELNLGRREEYDVLDKRRGRDPEMGGKPRRKNPQEGLYNELQKDKMAEAYSEIGMKGERRRGKGHDGLYQGLSTATKDTYDALHMQALPPRRAKRGSGATNFSLLKQAGDVEENPGPRAKRVDMGRGLLRGLWPLHIVLWTRIASTIPPHVQKSVNNDMIVTDNNGAVKFPQLCKFCDVRFSTCDNQKSCMSNCSITSICEKPQEVCVAVWRKNDENITLETVCHDPKLPYHDFILEDAASPKCIMKEKKKPGETFFMCSCSSDECNDNIIFSEEYNTSNPDLLLVIFQVTGISLLPPLGVAISVIIIFYCYRV

SEQ ID NO: 105 - DNA, 2390 bp, Artificial Sequence
  source: /note="Description of Artificial Sequence: Synthetic polynucleotide"
tgagctctgagtcagtgactcagtgagtcagtgactcagtgagtcagtgactcagctcgaggatctcgctagcgggaatttccggggactttccgggaatttccggggactttccgggaatttccagatctggcctcggcggccaagcttagacactagagggtatataatggaagctcgacttccagcttggcaatccggtactgttggtaaaggcgcgccccaccatgctgctgctggtcaccagcctgctgctgtgcgagctccctcaccccgcctttctgcttatcccggacattcagatgacacagaccacctcgagcttgtccgcgtcgctgggcgatcgcgtgaccatctcctgccgggcctcccaagacatttcaaagtatctcaactggtaccagcagaagccggacggaaccgtgaaactgctgatctaccataccagccgcctgcactccggcgtgccgtcccgcttctccggatcgggttccggaactgactactcactgactatctccaacttggaacaagaggacatcgccacttacttctgtcaacaaggaaatacccttccctacaccttcggggggggtaccaagctggagatcactgggggcggaggctccggtggaggcggatccggcggtggagggagcgaagtcaagctgcaggaatcaggaccaggactcgtggcgccatcccagtccctgtcggtgacctgtactgtctccggagtcagcctccccgattacggagtgtcatggattaggcaacccccaagaaaagggctggaatggctcggagtgatctggggctccgaaaccacctactacaactcggcgctgaagtcccggctgaccatcatcaaggacaactccaagagccaagtgttcttgaagatgaacagcttgcagaccgacgataccgcaatctactactgtgccaagcactattactacggggggtcttacgccatggactactggggacagggcacctccgtgactgtgtcgtccgcggccgctaccacaacccctgcgccccggcctcctacccccgcacccacgattgcttctcaacctctttcactccgacctgaggcttgtagacctgcagccgggggtgccgtccacacacggggactcgacttcgcttgtgatatatatatttgggcgcccctggccggcacttgtggagttcttttgctctctcttgttatcacattgtactgcaagcgaggtaggaagaaattgctttacatttttaagcagccgttcatgcgaccagtacagactactcaagaagaagatgggtgctcttgtcggttcccggaagaagaagagggtggttgcgagttgagggtgaagttctcccgctctgccgacgcaccggcatatcagcagggacaaaaccagctctacaacgaattgaacctgggtcggcgggaagaatatgacgtgctcgataagcggcggggtcgcgacccagaaatgggaggcaaaccgcgcaggaaaaatccacaggagggactttataacgaacttcaaaaggataagatggcagaggcatacagcgaaatcgggatgaaaggcgagagaagaagggggaaagggcacgatggtctttaccaggggctttctaccgcgacgaaggatacctacgatgctctccatatgcaagcacttcctcctagacgggcaaagcggggctcaggggcgactaacttttcactgttgaagcaggccggggatgtggaggagaatcctggtcctagagctaagcgagtagacatgcaaataccacaagcgccgtggcccgtcgtctgggctgttcttcagcttggctggagacctggctggtttctcgattctccagataggccctggaacccaccgacgttcagtccggcacttctcgtggtcacagagggggacaacgccacttttacgtgctcctttagcaacacctccgagtccttcgtactgaattggtatcgcatgagtccgtccaatcagacggacaagttggccgcgtttcctgaagataggtcacaacctggccaagactgtcggttccgggtcacccagttgccgaatgggagggactttcatatgagcgtcgttcgggcaagaaggaacgattctggaacgtatttgtgcggggccattagccttgcgccaaaagcgcagataaaggagtcccttcgggcagaacttcgcgtgacagagcgacgcgctgaagttccgactgcccatccctctccgagcccacgaccagccggacaatttcagactcttgtggtgggtgtggtaggcggcctgctcggaagcttggtcttgctggtgtgggtcctggctgtgatttgcagtcgagcagcccgcggcacc

SEQ ID NO: 106 - protein, 721 aa, Artificial Sequence
  source: /note="Description of Artificial Sequence: Synthetic polypeptide"
MLLLVTSLLLCELPHPAFLLIPDIQMTQTTSSLSASLGDRVTISCRASQDISKYLNWYQQKPDGTVKLLIYHTSRLHSGVPSRFSGSGSGTDYSLTISNLEQEDIATYFCQQGNTLPYTFGGGTKLEITGGGGSGGGGSGGGGSEVKLQESGPGLVAPSQSLSVTCTVSGVSLPDYGVSWIRQPPRKGLEWLGVIWGSETTYYNSALKSRLTIIKDNSKSQVFLKMNSLQTDDTAIYYCAKHYYYGGSYAMDYWGQGTSVTVSSAAATTTPAPRPPTPAPTIASQPLSLRPEACRPAAGGAVHTRGLDFACDIYIWAPLAGTCGVLLLSLVITLYCKRGRKKLLYIFKQPFMRPVQTTQEEDGCSCRFPEEEEGGCELRVKFSRSADAPAYQQGQNQLYNELNLGRREEYDVLDKRRGRDPEMGGKPRRKNPQEGLYNELQKDKMAEAYSEIGMKGERRRGKGHDGLYQGLSTATKDTYDALHMQALPPRRAKRGSGATNFSLLKQAGDVEENPGPRAKRVDMQIPQAPWPVVWAVLQLGWRPGWFLDSPDRPWNPPTFSPALLVVTEGDNATFTCSFSNTSESFVLNWYRMSPSNQTDKLAAFPEDRSQPGQDCRFRVTQLPNGRDFHMSVVRARRNDSGTYLCGAISLAPKAQIKESLRAELRVTERRAEVPTAHPSPSPRPAGQFQTLVVGVVGGLLGSLVLLVWVLAVICSRAARGT

SEQ ID NO: 107 - DNA, 3050 bp, Artificial Sequence
  source: /note="Description of Artificial Sequence: Synthetic polynucleotide"
tgagctctgagtcagtgactcagtgagtcagtgactcagtgagtcagtgactcagctcgaggatctcgctagcgggaatttccggggactttccgggaatttccggggactttccgggaatttccagatctggcctcggcggccaagcttagacactagagggtatataatggaagctcgacttccagcttggcaatccggtactgttggtaaaggcgcgccccaccatgctgctgctggtcaccagcctgctgctgtgcgagctccctcaccccgcctttctgcttatcccggacattcagatgacacagaccacctcgagcttgtccgcgtcgctgggcgatcgcgtgaccatctcctgccgggcctcccaagacatttcaaagtatctcaactggtaccagcagaagccggacggaaccgtgaaactgctgatctaccataccagccgcctgcactccggcgtgccgtcccgcttctccggatcgggttccggaactgactactcactgactatctccaacttggaacaagaggacatcgccacttacttctgtcaacaaggaaatacccttccctacaccttcggggggggtaccaagctggagatcactgggggcggaggctccggtggaggcggatccggcggtggagggagcgaagtcaagctgcaggaatcaggaccaggactcgtggcgccatcccagtccctgtcggtgacctgtactgtctccggagtcagcctccccgattacggagtgtcatggattaggcaacccccaagaaaagggctggaatggctcggagtgatctggggctccgaaaccacctactacaactcggcgctgaagtcccggctgaccatcatcaaggacaactccaagagccaagtgttcttgaagatgaacagcttgcagaccgacgataccgcaatctactactgtgccaagcactattactacggggggtcttacgccatggactactggggacagggcacctccgtgactgtgtcgtccgcggccgctaccacaacccctgcgccccggcctcctacccccgcacccacgattgcttctcaacctctttcactccgacctgaggcttgtagacctgcagccgggggtgccgtccacacacggggactcgacttcgcttgtgatatatatatttgggcgcccctggccggcacttgtggagttcttttgctctctcttgttatcacattgtactgcaagcgaggtaggaagaaattgctttacatttttaagcagccgttcatgcgaccagtacagactactcaagaagaagatgggtgctcttgtcggttcccggaagaagaagagggtggttgcgagttgagggtgaagttctcccgctctgccgacgcaccggcatatcagcagggacaaaaccagctctacaacgaattgaacctgggtcggcgggaagaatatgacgtgctcgataagcggcggggtcgcgacccagaaatgggaggcaaaccgcgcaggaaaaatccacaggagggactttataacgaacttcaaaaggataagatggcagaggcatacagcgaaatcgggatgaaaggcgagagaagaagggggaaagggcacgatggtctttaccaggggctttctaccgcgacgaaggatacctacgatgctctccatatgcaagcacttcctcctagacgggcaaagcggggctcaggggcgactaacttttcactgttgaagcaggccggggatgtggaggagaatcctggtcctagagctaagcgagtagacatgcaaataccacaagcgccgtggcccgtcgtctgggctgttcttcagcttggctggagacctggctggtttctcgattctccagataggccctggaacccaccgacgttcagtccggcacttctcgtggtcacagagggggacaacgccacttttacgtgctcctttagcaacacctccgagtccttcgtactgaattggtatcgcatgagtccgtccaatcagacggacaagttggccgcgtttcctgaagataggtcacaacctggccaagactgtcggttccgggtcacccagttgccgaatgggagggactttcatatgagcgtcgttcgggcaagaaggaacgattctggaacgtatttgtgcggggccattagccttgcgccaaaagcgcagataaaggagtcccttcgggcagaacttcgcgtgacagagcgacgcgctgaagttccgactgcccatccctctccgagcccacgaccagccggacaatttcagactcttgtggtgggtgtggtaggcggcctgctcggaagcttggtcttgctggtgtgggtcctggctgtgatttgcagtcgagcagcccgcggcacccgggctaaacggagcggctccggggcaaccaactttagtctgctgaaacaggcaggagatgtggaggaaaacccaggaccagctagcatgggaagagggctgctccgaggcttgtggccgttgcatattgtattgtggacgcggatagcgagtacaatcccgcctcacgtgcaaaaatcagttaataacgacatgatcgttactgacaacaatggcgcagttaaatttccgcagctttgtaaattctgtgatgtaagattttcaacgtgcgataaccagaaaagctgtatgtccaactgcagcatcacatcaatctgtgaaaaaccccaagaggtatgtgtggccgtctggcgaaagaatgacgaaaatatcacactggagaccgtttgtcacgatcctaaactcccttatcatgactttattctggaagacgcagcgtcaccgaagtgtataatgaaagagaagaagaagcctggagagacgtttttcatgtgcagttgctcctcagatgagtgtaatgacaacatcattttttccgaggagtacaatacgagtaacccagacctcctgctggttattttccaggtaaccggcatcagtttgttgcccccactgggtgttgcaatcagtgtaataatcatattttattgttaccgggtg

SEQ ID NO: 108 - protein, 941 aa, Artificial Sequence
  source: /note="Description of Artificial Sequence: Synthetic polypeptide"
MLLLVTSLLLCELPHPAFLLIPDIQMTQTTSSLSASLGDRVTISCRASQDISKYLNWYQQKPDGTVKLLIYHTSRLHSGVPSRFSGSGSGTDYSLTISNLEQEDIATYFCQQGNTLPYTFGGGTKLEITGGGGSGGGGSGGGGSEVKLQESGPGLVAPSQSLSVTCTVSGVSLPDYGVSWIRQPPRKGLEWLGVIWGSETTYYNSALKSRLTIIKDNSKSQVFLKMNSLQTDDTAIYYCAKHYYYGGSYAMDYWGQGTSVTVSSAAATTTPAPRPPTPAPTIASQPLSLRPEACRPAAGGAVHTRGLDFACDIYIWAPLAGTCGVLLLSLVITLYCKRGRKKLLYIFKQPFMRPVQTTQEEDGCSCRFPEEEEGGCELRVKFSRSADAPAYQQGQNQLYNELNLGRREEYDVLDKRRGRDPEMGGKPRRKNPQEGLYNELQKDKMAEAYSEIGMKGERRRGKGHDGLYQGLSTATKDTYDALHMQALPPRRAKRGSGATNFSLLKQAGDVEENPGPRAKRVDMQIPQAPWPVVWAVLQLGWRPGWFLDSPDRPWNPPTFSPALLVVTEGDNATFTCSFSNTSESFVLNWYRMSPSNQTDKLAAFPEDRSQPGQDCRFRVTQLPNGRDFHMSVVRARRNDSGTYLCGAISLAPKAQIKESLRAELRVTERRAEVPTAHPSPSPRPAGQFQTLVVGVVGGLLGSLVLLVWVLAVICSRAARGTRAKRSGSGATNFSLLKQAGDVEENPGPASMGRGLLRGLWPLHIVLWTRIASTIPPHVQKSVNNDMIVTDNNGAVKFPQLCKFCDVRFSTCDNQKSCMSNCSITSICEKPQEVCVAVWRKNDENITLETVCHDPKLPYHDFILEDAASPKCIMKEKKKPGETFFMCSCSSDECNDNIIFSEEYNTSNPDLLLVIFQVTGISLLPPLGVAISVIIIFYCYRV

SEQ ID NO: 109 - DNA, 2342 bp, Artificial Sequence
  source: /note="Description of Artificial Sequence: Synthetic polynucleotide"
ggtacctgagctcagttctgagaaaagtagttctgagaaaagtagttctgagaaaagtagttctgagaaaagtagttctgagaaaagtctcgaggatatcaagatctggcctcggcggccaagcttagacactagagggtatataatggaagctcgacttccagcttggcaatccggtactgttggtaaaggcgcgccccaccatgctgctgctggtcaccagcctgctgctgtgcgagctccctcaccccgcctttctgcttatcccggacattcagatgacacagaccacctcgagcttgtccgcgtcgctgggcgatcgcgtgaccatctcctgccgggcctcccaagacatttcaaagtatctcaactggtaccagcagaagccggacggaaccgtgaaactgctgatctaccataccagccgcctgcactccggcgtgccgtcccgcttctccggatcgggttccggaactgactactcactgactatctccaacttggaacaagaggacatcgccacttacttctgtcaacaaggaaatacccttccctacaccttcggggggggtaccaagctggagatcactgggggcggaggctccggtggaggcggatccggcggtggagggagcgaagtcaagctgcaggaatcaggaccaggactcgtggcgccatcccagtccctgtcggtgacctgtactgtctccggagtcagcctccccgattacggagtgtcatggattaggcaacccccaagaaaagggctggaatggctcggagtgatctggggctccgaaaccacctactacaactcggcgctgaagtcccggctgaccatcatcaaggacaactccaagagccaagtgttcttgaagatgaacagcttgcagaccgacgataccgcaatctactactgtgccaagcactattactacggggggtcttacgccatggactactggggacagggcacctccgtgactgtgtcgtccgcggccgctaccacaacccctgcgccccggcctcctacccccgcacccacgattgcttctcaacctctttcactccgacctgaggcttgtagacctgcagccgggggtgccgtccacacacggggactcgacttcgcttgtgatatatatatttgggcgcccctggccggcacttgtggagttcttttgctctctcttgttatcacattgtactgcaagcgaggtaggaagaaattgctttacatttttaagcagccgttcatgcgaccagtacagactactcaagaagaagatgggtgctcttgtcggttcccggaagaagaagagggtggttgcgagttgagggtgaagttctcccgctctgccgacgcaccggcatatcagcagggacaaaaccagctctacaacgaattgaacctgggtcggcgggaagaatatgacgtgctcgataagcggcggggtcgcgacccagaaatgggaggcaaaccgcgcaggaaaaatccacaggagggactttataacgaacttcaaaaggataagatggcagaggcatacagcgaaatcgggatgaaaggcgagagaagaagggggaaagggcacgatggtctttaccaggggctttctaccgcgacgaaggatacctacgatgctctccatatgcaagcacttcctcctagacgggcaaagcggggctcaggggcgactaacttttcactgttgaagcaggccggggatgtggaggagaatcctggtcctagagctaagcgagtagacatgggaagagggctgctccgaggcttgtggccgttgcatattgtattgtggacgcggatagcgagtacaatcccgcctcacgtgcaaaaatcagttaataacgacatgatcgttactgacaacaatggcgcagttaaatttccgcagctttgtaaattctgtgatgtaagattttcaacgtgcgataaccagaaaagctgtatgtccaactgcagcatcacatcaatctgtgaaaaaccccaagaggtatgtgtggccgtctggcgaaagaatgacgaaaatatcacactggagaccgtttgtcacgatcctaaactcccttatcatgactttattctggaagacgcagcgtcaccgaagtgtataatgaaagagaagaagaagcctggagagacgtttttcatgtgcagttgctcctcagatgagtgtaatgacaacatcattttttccgaggagtacaatacgagtaacccagacctcctgctggttattttccaggtaaccggcatcagtttgttgcccccactgggtgttgcaatcagtgtaataatcatattttattgttaccgggtg

SEQ ID NO: 110 - DNA, 2366 bp, Artificial Sequence
  source: /note="Description of Artificial Sequence: Synthetic polynucleotide"
ggtacctgagctcagttctgagaaaagtagttctgagaaaagtagttctgagaaaagtagttctgagaaaagtagttctgagaaaagtctcgaggatatcaagatctggcctcggcggccaagcttagacactagagggtatataatggaagctcgacttccagcttggcaatccggtactgttggtaaaggcgcgccccaccatgctgctgctggtcaccagcctgctgctgtgcgagctccctcaccccgcctttctgcttatcccggacattcagatgacacagaccacctcgagcttgtccgcgtcgctgggcgatcgcgtgaccatctcctgccgggcctcccaagacatttcaaagtatctcaactggtaccagcagaagccggacggaaccgtgaaactgctgatctaccataccagccgcctgcactccggcgtgccgtcccgcttctccggatcgggttccggaactgactactcactgactatctccaacttggaacaagaggacatcgccacttacttctgtcaacaaggaaatacccttccctacaccttcggggggggtaccaagctggagatcactgggggcggaggctccggtggaggcggatccggcggtggagggagcgaagtcaagctgcaggaatcaggaccaggactcgtggcgccatcccagtccctgtcggtgacctgtactgtctccggagtcagcctccccgattacggagtgtcatggattaggcaacccccaagaaaagggctggaatggctcggagtgatctggggctccgaaaccacctactacaactcggcgctgaagtcccggctgaccatcatcaaggacaactccaagagccaagtgttcttgaagatgaacagcttgcagaccgacgataccgcaatctactactgtgccaagcactattactacggggggtcttacgccatggactactggggacagggcacctccgtgactgtgtcgtccgcggccgctaccacaacccctgcgccccggcctcctacccccgcacccacgattgcttctcaacctctttcactccgacctgaggcttgtagacctgcagccgggggtgccgtccacacacggggactcgacttcgcttgtgatatatatatttgggcgcccctggccggcacttgtggagttcttttgctctctcttgttatcacattgtactgcaagcgaggtaggaagaaattgctttacatttttaagcagccgttcatgcgaccagtacagactactcaagaagaagatgggtgctcttgtcggttcccggaagaagaagagggtggttgcgagttgagggtgaagttctcccgctctgccgacgcaccggcatatcagcagggacaaaaccagctctacaacgaattgaacctgggtcggcgggaagaatatgacgtgctcgataagcggcggggtcgcgacccagaaatgggaggcaaaccgcgcaggaaaaatccacaggagggactttataacgaacttcaaaaggataagatggcagaggcatacagcgaaatcgggatgaaaggcgagagaagaagggggaaagggcacgatggtctttaccaggggctttctaccgcgacgaaggatacctacgatgctctccatatgcaagcacttcctcctagacgggcaaagcggggctcaggggcgactaacttttcactgttgaagcaggccggggatgtggaggagaatcctggtcctagagctaagcgagtagacatgcaaataccacaagcgccgtggcccgtcgtctgggctgttcttcagcttggctggagacctggctggtttctcgattctccagataggccctggaacccaccgacgttcagtccggcacttctcgtggtcacagagggggacaacgccacttttacgtgctcctttagcaacacctccgagtccttcgtactgaattggtatcgcatgagtccgtccaatcagacggacaagttggccgcgtttcctgaagataggtcacaacctggccaagactgtcggttccgggtcacccagttgccgaatgggagggactttcatatgagcgtcgttcgggcaagaaggaacgattctggaacgtatttgtgcggggccattagccttgcgccaaaagcgcagataaaggagtcccttcgggcagaacttcgcgtgacagagcgacgcgctgaagttccgactgcccatccctctccgagcccacgaccagccggacaatttcagactcttgtggtgggtgtggtaggcggcctgctcggaagcttggtcttgctggtgtgggtcctggctgtgatttgcagtcgagcagcccgcggcacc

SEQ ID NO: 111 - DNA, 3026 bp, Artificial Sequence
  source: /note="Description of Artificial Sequence: Synthetic polynucleotide"
ggtacctgagctcagttctgagaaaagtagttctgagaaaagtagttctgagaaaagtagttctgagaaaagtagttctgagaaaagtctcgaggatatcaagatctggcctcggcggccaagcttagacactagagggtatataatggaagctcgacttccagcttggcaatccggtactgttggtaaaggcgcgccccaccatgctgctgctggtcaccagcctgctgctgtgcgagctccctcaccccgcctttctgcttatcccggacattcagatgacacagaccacctcgagcttgtccgcgtcgctgggcgatcgcgtgaccatctcctgccgggcctcccaagacatttcaaagtatctcaactggtaccagcagaagccggacggaaccgtgaaactgctgatctaccataccagccgcctgcactccggcgtgccgtcccgcttctccggatcgggttccggaactgactactcactgactatctccaacttggaacaagaggacatcgccacttacttctgtcaacaaggaaatacccttccctacaccttcggggggggtaccaagctggagatcactgggggcggaggctccggtggaggcggatccggcggtggagggagcgaagtcaagctgcaggaatcaggaccaggactcgtggcgccatcccagtccctgtcggtgacctgtactgtctccggagtcagcctccccgattacggagtgtcatggattaggcaacccccaagaaaagggctggaatggctcggagtgatctggggctccgaaaccacctactacaactcggcgctgaagtcccggctgaccatcatcaaggacaactccaagagccaagtgttcttgaagatgaacagcttgcagaccgacgataccgcaatctactactgtgccaagcactattactacggggggtcttacgccatggactactggggacagggcacctccgtgactgtgtcgtccgcggccgctaccacaacccctgcgccccggcctcctacccccgcacccacgattgcttctcaacctctttcactccgacctgaggcttgtagacctgcagccgggggtgccgtccacacacggggactcgacttcgcttgtgatatatatatttgggcgcccctggccggcacttgtggagttcttttgctctctcttgttatcacattgtactgcaagcgaggtaggaagaaattgctttacatttttaagcagccgttcatgcgaccagtacagactactcaagaagaagatgggtgctcttgtcggttcccggaagaagaagagggtggttgcgagttgagggtgaagttctcccgctctgccgacgcaccggcatatcagcagggacaaaaccagctctacaacgaattgaacctgggtcggcgggaagaatatgacgtgctcgataagcggcggggtcgcgacccagaaatgggaggcaaaccgcgcaggaaaaatccacaggagggactttataacgaacttcaaaaggataagatggcagaggcatacagcgaaatcgggatgaaaggcgagagaagaagggggaaagggcacgatggtctttaccaggggctttctaccgcgacgaaggatacctacgatgctctccatatgcaagcacttcctcctagacgggcaaagcggggctcaggggcgactaacttttcactgttgaagcaggccggggatgtggaggagaatcctggtcctagagctaagcgagtagacatgcaaataccacaagcgccgtggcccgtcgtctgggctgttcttcagcttggctggagacctggctggtttctcgattctccagataggccctggaacccaccgacgttcagtccggcacttctcgtggtcacagagggggacaacgccacttttacgtgctcctttagcaacacctccgagtccttcgtactgaattggtatcgcatgagtccgtccaatcagacggacaagttggccgcgtttcctgaagataggtcacaacctggccaagactgtcggttccgggtcacccagttgccgaatgggagggactttcatatgagcgtcgttcgggcaagaaggaacgattctggaacgtatttgtgcggggccattagccttgcgccaaaagcgcagataaaggagtcccttcgggcagaacttcgcgtgacagagcgacgcgctgaagttccgactgcccatccctctccgagcccacgaccagccggacaatttcagactcttgtggtgggtgtggtaggcggcctgctcggaagcttggtcttgctggtgtgggtcctggctgtgatttgcagtcgagcagcccgcggcacccgggctaaacggagcggctccggggcaaccaactttagtctgctgaaacaggcaggagatgtggaggaaaacccaggaccagctagcatgggaagagggctgctccgaggcttgtggccgttgcatattgtattgtggacgcggatagcgagtacaatcccgcctcacgtgcaaaaatcagttaataacgacatgatcgttactgacaacaatggcgcagttaaatttccgcagctttgtaaattctgtgatgtaagattttcaacgtgcgataaccagaaaagctgtatgtccaactgcagcatcacatcaatctgtgaaaaaccccaagaggtatgtgtggccgtctggcgaaagaatgacgaaaatatcacactggagaccgtttgtcacgatcctaaactcccttatcatgactttattctggaagacgcagcgtcaccgaagtgtataatgaaagagaagaagaagcctggagagacgtttttcatgtgcagttgctcctcagatgagtgtaatgacaacatcattttttccgaggagtacaatacgagtaacccagacctcctgctggttattttccaggtaaccggcatcagtttgttgcccccactgggtgttgcaatcagtgtaataatcatattttattgttaccgggtg

SEQ ID NO: 112 - protein, 245 aa, Artificial Sequence
  source: /note="Description of Artificial Sequence: Synthetic polypeptide"
DIQMTQTTSSLSASLGDRVTISCRASQDISKYLNWYQQKPDGTVKLLIYHTSRLHSGVPSRFSGSGSGTDYSLTISNLEQEDIATYFCQQGNTLPYTFGGGTKLEITGSTSGSGKPGSGEGSTKGEVKLQESGPGLVAPSQSLSVTCTVSGVSLPDYGVSWIRQPPRKGLEWLGVIWGSETTYYNSALKSRLTIIKDNSKSQVFLKMNSLQTDDTAIYYCAKHYYYGGSYAMDYWGQGTSVTVSS

SEQ ID NO: 113 - DNA, 729 bp, Artificial Sequence
  source: /note="Description of Artificial Sequence: Synthetic polynucleotide"
gaggtgcagttgcaacagtcaggagctgaactggtcaagccaggagccagcgtgaagatgagctgcaaggcctccggttacaccttcacctcctacaacatgcactgggtgaaacagaccccgggacaagggctcgaatggattggcgccatctaccccgggaatggcgatacttcgtacaaccagaagttcaagggaaaggccaccctgaccgccgacaagagctcctccaccgcgtatatgcagttgagctccctgacctccgaggactccgccgactactactgcgcacggtccaactactatggaagctcgtactggttcttcgatgtctggggggccggcaccactgtgaccgtcagctccgggggcggaggatccggtggaggcggaagcgggggtggaggatccgacattgtgctgactcagtccccggcaatcctgtcggcctcaccgggcgaaaaggtcacgatgacttgtagagcgtcgtccagcgtgaactacatggattggtaccaaaagaagcctggatcgtcacccaagccttggatctacgctacatctaacctggcctccggcgtgccagcgcggttcagcgggtccggctcgggcacctcatactcgctgaccatctcccgcgtggaggctgaggacgccgcgacctactactgccagcagtggtccttcaacccgccgacttttggaggcggtactaagctggagatcaaa

SEQ ID NO: 114 - protein, 243 aa, Artificial Sequence
  source: /note="Description of Artificial Sequence: Synthetic polypeptide"
EVQLQQSGAELVKPGASVKMSCKASGYTFTSYNMHWVKQTPGQGLEWIGAIYPGNGDTSYNQKFKGKATLTADKSSSTAYMQLSSLTSEDSADYYCARSNYYGSSYWFFDVWGAGTTVTVSSGGGGSGGGGSGGGGSDIVLTQSPAILSASPGEKVTMTCRASSSVNYMDWYQKKPGSSPKPWIYATSNLASGVPARFSGSGSGTSYSLTISRVEAEDAATYYCQQWSFNPPTFGGGTKLEIK

SEQ ID NO: 115 - DNA, 1491 bp, Artificial Sequence
  source: /note="Description of Artificial Sequence: Synthetic polynucleotide"
atgctgctgctggtgaccagcctgctgctgtgcgaactgccgcatccggcgtttctgctgattccgcaagtgcaactcgtccaatccggtgccgaagtcaagaagcctggttcctccgtgaaagtgtcgtgcaaagccagcggcgggacttttagctcctacgcgatcagctgggtcagacaggcccctggacaaggcctcgagtggatgggcggcatcattccgattttcggtaccgccaactacgcccagaagttccagggacgcgtgaccattactaccgacgagagcacctcaaccgcatacatggaactgtccagcctgcgctccgaggacacggctgtgtactattgcgccagacggggatggggaggattctcctccggctccgcattcgacatctggggacagggcactatggtcactgtgtcatccgggggaggaggatcaggcggtggaggatccggtggtggcggatccaacttcatgctgacccagccccactcagtgtcggaatcgcccggcaacaccgtgactatcagctgcaccggatccagcgggaccatcggctctaatttcgtgcagtggtaccagcagtccccagggagagctccgaccctgttgatctacgaggacacaaagcggccaagcggagtgccgcctagattcgccggctccgtggattcctcgtccaactcggcgtcgctgaccatcagcggactcaagactgaagatgaagccgactactactgtcagtcctacgactcgagcaactgggtgtttgggggcgggactaagctgaccgtgcttggagcggccgcaactaccacccctgcccctcggccgccgactccggccccaaccatcgcaagccaacccctctccttgcgccccgaagcttgccgcccggccgcgggtggagccgtgcatacccgggggctggactttgcctgcgatatctacatttgggccccgctggccggcacttgcggcgtgctcctgctgtcgctggtcatcaccctttactgcaagaggggccggaagaagctgctttacatcttcaagcagccgttcatgcggcccgtgcagacgactcaggaagaggacggatgctcgtgcagattccctgaggaggaagaggggggatgcgaactgcgcgtcaagttctcacggtccgccgacgcccccgcatatcaacagggccagaatcagctctacaacgagctgaacctgggaaggagagaggagtacgacgtgctggacaagcgacgcggacgcgacccggagatgggggggaaaccacggcggaaaaaccctcaggaaggactgtacaacgaactccagaaagacaagatggcggaagcctactcagaaatcgggatgaagggagagcggaggaggggaaagggtcacgacgggctgtaccagggactgagcaccgccactaaggatacctacgatgccttgcatatgcaagcactcccaccccgg

SEQ ID NO: 116 - protein, 497 aa, Artificial Sequence
  source: /note="Description of Artificial Sequence: Synthetic polypeptide"
MLLLVTSLLLCELPHPAFLLIPQVQLVQSGAEVKKPGSSVKVSCKASGGTFSSYAISWVRQAPGQGLEWMGGIIPIFGTANYAQKFQGRVTITTDESTSTAYMELSSLRSEDTAVYYCARRGWGGFSSGSAFDIWGQGTMVTVSSGGGGSGGGGSGGGGSNFMLTQPHSVSESPGNTVTISCTGSSGTIGSNFVQWYQQSPGRAPTLLIYEDTKRPSGVPPRFAGSVDSSSNSASLTISGLKTEDEADYYCQSYDSSNWVFGGGTKLTVLGAAATTTPAPRPPTPAPTIASQPLSLRPEACRPAAGGAVHTRGLDFACDIYIWAPLAGTCGVLLLSLVITLYCKRGRKKLLYIFKQPFMRPVQTTQEEDGCSCRFPEEEEGGCELRVKFSRSADAPAYQQGQNQLYNELNLGRREEYDVLDKRRGRDPEMGGKPRRKNPQEGLYNELQKDKMAEAYSEIGMKGERRRGKGHDGLYQGLSTATKDTYDALHMQALPPR

SEQ ID NO: 117 - DNA, 1479 bp, Artificial Sequence
  source: /note="Description of Artificial Sequence: Synthetic polynucleotide"
atgctgctgctggtgaccagcctgctgctgtgcgaactgccgcatccggcgtttctgctgattccggaagtccaattggtgcagagcggatccgaacttaagaaacctggcgcgagcgtgaaagtgtcctgcaaggcctccggagggactttctcgtcgtacgccattagctgggtccgccaagctcctggccaaggcctggagtggatgggcgggattatccccatcttcgggactgcgaactacgcccagaagtttcagggccgggtcactatcaccgccgacgaatcaacctcgaccgcctacatggaactgtcctcgcttcggtccgaggatactgccgtgtactattgtgcctcaacggccagacgcggatgggacaccgctggtccgctcgattactggggccagggaaccctcgtgaccgtcagctccggaggaggaggctccggtggtggaggatccgggggtggtggatccgacatccaaatgacccagtccccctcgtccctgagcgcctctgtgggcgacagagtgacaattgcatgcagggcctcacagactatctcccgctacctgaactggtaccagcagaagccaggaaaggcccctaagctgctcatctacgctgcgtcctcgctccaatccggggtgtcctcacggttttccggatcgggttccggcaccgagttcaccctgaccatcagcagcctgcagcccgaggacttcgcaacctacttctgccagcaaacctactccccgccgattacgttcggacaggggactcggctggaaatcaaggcggccgcaactaccacccctgcccctcggccgccgactccggccccaaccatcgcaagccaacccctctccttgcgccccgaagcttgccgcccggccgcgggtggagccgtgcatacccgggggctggactttgcctgcgatatctacatttgggccccgctggccggcacttgcggcgtgctcctgctgtcgctggtcatcaccctttactgcaagaggggccggaagaagctgctttacatcttcaagcagccgttcatgcggcccgtgcagacgactcaggaagaggacggatgctcgtgcagattccctgaggaggaagaggggggatgcgaactgcgcgtcaagttctcacggtccgccgacgcccccgcatatcaacagggccagaatcagctctacaacgagctgaacctgggaaggagagaggagtacgacgtgctggacaagcgacgcggacgcgacccggagatgggggggaaaccacggcggaaaaaccctcaggaaggactgtacaacgaactccagaaagacaagatggcggaagcctactcagaaatcgggatgaagggagagcggaggaggggaaagggtcacgacgggctgtaccagggactgagcaccgccactaaggatacctacgatgccttgcatatgcaagcactcccaccccgg

SEQ ID NO: 118 - protein, 493 aa, Artificial Sequence
  source: /note="Description of Artificial Sequence: Synthetic polypeptide"
MLLLVTSLLLCELPHPAFLLIPEVQLVQSGSELKKPGASVKVSCKASGGTFSSYAISWVRQAPGQGLEWMGGIIPIFGTANYAQKFQGRVTITADESTSTAYMELSSLRSEDTAVYYCASTARRGWDTAGPLDYWGQGTLVTVSSGGGGSGGGGSGGGGSDIQMTQSPSSLSASVGDRVTIACRASQTISRYLNWYQQKPGKAPKLLIYAASSLQSGVSSRFSGSGSGTEFTLTISSLQPEDFATYFCQQTYSPPITFGQGTRLEIKAAATTTPAPRPPTPAPTIASQPLSLRPEACRPAAGGAVHTRGLDFACDIYIWAPLAGTCGVLLLSLVITLYCKRGRKKLLYIFKQPFMRPVQTTQEEDGCSCRFPEEEEGGCELRVKFSRSADAPAYQQGQNQLYNELNLGRREEYDVLDKRRGRDPEMGGKPRRKNPQEGLYNELQKDKMAEAYSEIGMKGERRRGKGHDGLYQGLSTATKDTYDALHMQALPPR

SEQ ID NO: 119 - DNA, 1473 bp, Artificial Sequence
  source: /note="Description of Artificial Sequence: Synthetic polynucleotide"
atgctgctgctggtgaccagcctgctgctgtgcgaactgccgcatccggcgtttctgctgattccggaagtgcaactcgtcgaaacaggggcagaagtgaaaaacccaggctcaagcgtgaaagtgtcgtgcaaggcttcgggcggaactctgtccaactacgccatctcctgggtccgccaagctccgggaaagggcctcgagtggatgggcggaatcattcccattttcgggaccgccaactacgcgcaaaagttccagggccgggtcactatcaccgcggacgaaagcaccagcaccgcctacatggaactgtcctccctgcgctccgaggacactgccgtgtactattgcgcccggaggtcatcgtggtaccccgagggctgcttccagcactggggacagggcactctcgtgaccgtgtcgtcgggtggtggtggatcaggagggggaggatccggaggaggcggaagcgatattcagctgacccagtcaccgagctccctgtccgcctccaccggagacagagtgaccatcacgtgtcgggcctcccaagggatctcctcctacctggcctggtaccagcagaagcctggaaaggcaccgaagttgctgatctacgccgcgagcacccttcagtccggagtgcctagccgcttctcgggttccggctctggcactgacttcactctgaccattagctgcctgcagtccgaggattttgccacctactactgccagcagtactatagctaccccctgaccttcgggggcggaaccaagctcgacatcaaggcggccgcaactaccacccctgcccctcggccgccgactccggccccaaccatcgcaagccaacccctctccttgcgccccgaagcttgccgcccggccgcgggtggagccgtgcatacccgggggctggactttgcctgcgatatctacatttgggccccgctggccggcacttgcggcgtgctcctgctgtcgctggtcatcaccctttactgcaagaggggccggaagaagctgctttacatcttcaagcagccgttcatgcggcccgtgcagacgactcaggaagaggacggatgctcgtgcagattccctgaggaggaagaggggggatgcgaactgcgcgtcaagttctcacggtccgccgacgcccccgcatatcaacagggccagaatcagctctacaacgagctgaacctgggaaggagagaggagtacgacgtgctggacaagcgacgcggacgcgacccggagatgggggggaaaccacggcggaaaaaccctcaggaaggactgtacaacgaactccagaaagacaagatggcggaagcctactcagaaatcgggatgaagggagagcggaggaggggaaagggtcacgacgggctgtaccagggactgagcaccgccactaaggatacctacgatgccttgcatatgcaagcactcccaccccgg

SEQ ID NO: 120 - protein, 491 aa, Artificial Sequence
  source: /note="Description of Artificial Sequence: Synthetic polypeptide"
MLLLVTSLLLCELPHPAFLLIPEVQLVETGAEVKNPGSSVKVSCKASGGTLSNYAISWVRQAPGKGLEWMGGIIPIFGTANYAQKFQGRVTITADESTSTAYMELSSLRSEDTAVYYCARRSSWYPEGCFQHWGQGTLVTVSSGGGGSGGGGSGGGGSDIQLTQSPSSLSASTGDRVTITCRASQGISSYLAWYQQKPGKAPKLLIYAASTLQSGVPSRFSGSGSGTDFTLTISCLQSEDFATYYCQQYYSYPLTFGGGTKLDIKAAATTTPAPRPPTPAPTIASQPLSLRPEACRPAAGGAVHTRGLDFACDIYIWAPLAGTCGVLLLSLVITLYCKRGRKKLLYIFKQPFMRPVQTTQEEDGCSCRFPEEEEGGCELRVKFSRSADAPAYQQGQNQLYNELNLGRREEYDVLDKRRGRDPEMGGKPRRKNPQEGLYNELQKDKMAEAYSEIGMKGERRRGKGHDGLYQGLSTATKDTYDALHMQALPPR

SEQ ID NO: 121 - DNA, 1476 bp, Artificial Sequence
  source: /note="Description of Artificial Sequence: Synthetic polynucleotide"
atgctgctgctggtgaccagcctgctgctgtgcgaactgccgcatccggcgtttctgctgattccggaagtgcaactcgtccaatctggtgccgaagtcaagaagcctggctcaagcgtgaaagtgtcctgcaaagcgtcgggagggaccttcagctcctacgccatttcctgggtccgccaagcaccaggacagggcctggagtggatgggcggcatcatcccgatcttcgggactgccaactacgcccagaagttccaggggagagtgaccattaccgccgacgagtcgaccagcacggcctacatggaactgtccagcctgcgctccgaggacactgccgtgtactactgcgcgagggccagactcggtggagcgttcgacatctggggacagggcaccatggtcaccgtgtcatccggtggcggaggatccggtggtggcggatcaggagggggaggatcccagtccgtgctgactcagcctccctccgtgagcgctgcaccgggacagaaggtcaccatctcatgctcggggggaagctccaacatcgggaaccactacgtgtcctggtaccaacagttgcctggtgccgctccaaagctgctgatctatgacgataacaagcggccgtccggaatccccgaccggttctcggggtctagatccggaaccagcgcaactctcggcattaccggactgcagagcggcgatgaggccgactactactgtggcacatgggactcgtcgctggctgcccacgtgtttggcactggcaccaaggtcaccgtgcttggagcggccgcaactaccacccctgcccctcggccgccgactccggccccaaccatcgcaagccaacccctctccttgcgccccgaagcttgccgcccggccgcgggtggagccgtgcatacccgggggctggactttgcctgcgatatctacatttgggccccgctggccggcacttgcggcgtgctcctgctgtcgctggtcatcaccctttactgcaagaggggccggaagaagctgctttacatcttcaagcagccgttcatgcggcccgtgcagacgactcaggaagaggacggatgctcgtgcagattccctgaggaggaagaggggggatgcgaactgcgcgtcaagttctcacggtccgccgacgcccccgcatatcaacagggccagaatcagctctacaacgagctgaacctgggaaggagagaggagtacgacgtgctggacaagcgacgcggacgcgacccggagatgggggggaaaccacggcggaaaaaccctcaggaaggactgtacaacgaactccagaaagacaagatggcggaagcctactcagaaatcgggatgaagggagagcggaggaggggaaagggtcacgacgggctgtaccagggactgagcaccgccactaaggatacctacgatgccttgcatatgcaagcactcccaccccgg

SEQ ID NO: 122 - protein, 492 aa, Artificial Sequence
  source: /note="Description of Artificial Sequence: Synthetic polypeptide"
MLLLVTSLLLCELPHPAFLLIPEVQLVQSGAEVKKPGSSVKVSCKASGGTFSSYAISWVRQAPGQGLEWMGGIIPIFGTANYAQKFQGRVTITADESTSTAYMELSSLRSEDTAVYYCARARLGGAFDIWGQGTMVTVSSGGGGSGGGGSGGGGSQSVLTQPPSVSAAPGQKVTISCSGGSSNIGNHYVSWYQQLPGAAPKLLIYDDNKRPSGIPDRFSGSRSGTSATLGITGLQSGDEADYYCGTWDSSLAAHVFGTGTKVTVLGAAATTTPAPRPPTPAPTIASQPLSLRPEACRPAAGGAVHTRGLDFACDIYIWAPLAGTCGVLLLSLVITLYCKRGRKKLLYIFKQPFMRPVQTTQEEDGCSCRFPEEEEGGCELRVKFSRSADAPAYQQGQNQLYNELNLGRREEYDVLDKRRGRDPEMGGKPRRKNPQEGLYNELQKDKMAEAYSEIGMKGERRRGKGHDGLYQGLSTATKDTYDALHMQALPPR

SEQ ID NO: 123 - DNA, 1491 bp, Artificial Sequence
  source: /note="Description of Artificial Sequence: Synthetic polynucleotide"
atgctgctgctggtgaccagcctgctgctgtgcgaactgccgcatccggcgtttctgctgattccggaagtgcaacttgtccagagcggagccgaagtgaagaaacctggatcctccgtcaaagtgtcgtgcaaggcttcgggcggaaccttctcctcgtacgcgatctcatgggtcagacaggcacccggacagggactggagtggatgggcggcatcattcccatcttcggcaccgctaattacgcccagaagtttcaggggagagtgaccatcaccgccgacgagtccacctccactgcctacatggaactgtcctcactgaggtccgaggatactgccgtgtactactgcgcgtcgcaaaaggggggtggatggtccattgacgccttcgatatttggggacaggggacgatggtcacagtgtcatccggcggtggtggatccggtggtggcggatccggaggaggaggcagccagtccgtgctgacccagccgcctagcgtgtcggccgcatctgggcagcgcgtgaccatttcctgttccgggtcctcgtccaacatcggcaacaactacgcctcctggtaccaacagctcccgggaatggcccctaagctgctgatctacgaggacaacaagcggccatccgggatctcagaccggttcagcggatcccagtccggcacttccgcgagcctcgccatcaccggactgcaggctgaggacgaagccgactactactgccaatcatatgacagctcgctcagcggcgatgtggtgttcggcggtggcactaagctgaccgtgttgggagcggccgcaactaccacccctgcccctcggccgccgactccggccccaaccatcgcaagccaacccctctccttgcgccccgaagcttgccgcccggccgcgggtggagccgtgcatacccgggggctggactttgcctgcgatatctacatttgggccccgctggccggcacttgcggcgtgctcctgctgtcgctggtcatcaccctttactgcaagaggggccggaagaagctgctttacatcttcaagcagccgttcatgcggcccgtgcagacgactcaggaagaggacggatgctcgtgcagattccctgaggaggaagaggggggatgcgaactgcgcgtcaagttctcacggtccgccgacgcccccgcatatcaacagggccagaatcagctctacaacgagctgaacctgggaaggagagaggagtacgacgtgctggacaagcgacgcggacgcgacccggagatgggggggaaaccacggcggaaaaaccctcaggaaggactgtacaacgaactccagaaagacaagatggcggaagcctactcagaaatcgggatgaagggagagcggaggaggggaaagggtcacgacgggctgtaccagggactgagcaccgccactaaggatacctacgatgccttgcatatgcaagcactcccaccccgg

SEQ ID NO: 124 - protein, 497 aa, Artificial Sequence
  source: /note="Description of Artificial Sequence: Synthetic polypeptide"
MLLLVTSLLLCELPHPAFLLIPEVQLVQSGAEVKKPGSSVKVSCKASGGTFSSYAISWVRQAPGQGLEWMGGIIPIFGTANYAQKFQGRVTITADESTSTAYMELSSLRSEDTAVYYCASQKGGGWSIDAFDIWGQGTMVTVSSGGGGSGGGGSGGGGSQSVLTQPPSVSAASGQRVTISCSGSSSNIGNNYASWYQQLPGMAPKLLIYEDNKRPSGISDRFSGSQSGTSASLAITGLQAEDEADYYCQSYDSSLSGDVVFGGGTKLTVLGAAATTTPAPRPPTPAPTIASQPLSLRPEACRPAAGGAVHTRGLDFACDIYIWAPLAGTCGVLLLSLVITLYCKRGRKKLLYIFKQPFMRPVQTTQEEDGCSCRFPEEEEGGCELRVKFSRSADAPAYQQGQNQLYNELNLGRREEYDVLDKRRGRDPEMGGKPRRKNPQEGLYNELQKDKMAEAYSEIGMKGERRRGKGHDGLYQGLSTATKDTYDALHMQALPPR

SEQ ID NO: 125 - DNA, 1479 bp, Artificial Sequence
  source: /note="Description of Artificial Sequence: Synthetic polynucleotide"
atgctgctgctggtgaccagcctgctgctgtgcgaactgccgcatccggcgtttctgctgattccgcaagtccagttgcaacaatggggagcaggccttctgaaaccgtccgagacactgagcctgacgtgcgccgtctatggcggatcgttctccggatactactggtcgtggatcagacagcctccgggaaagggtctggaatggatcggcgaaatcaaccacagcggcagcaccaattacaacccgtcactgaagtcaagggtcaccattagcgtggacacttccaagaaccagttctccctgaaactgtcgagcgtgaccgctgccgatactgccgtgtactactgtgcccgcggccaagtcaagtatagctcaagcctcggctactggggccagggaaccctcgtgaccgtgtcctcgggtggaggaggctccggtggtggaggatccggtggcggaggatcgcagtccgtgctgacccagcctccctccgtgtctgctgcccctgggcaaaaggtcaccatttcgtgctccggctcatcgtccaacatcgggaacaactttgtgtcctggtaccagcagctgcccggtactgccccaaagctgctgatctacgaggacaacaagcgcccatccgggattccggatcggttcagcggatcacggtccggaactagcgcgaccctggggatcaccgggctccagactggcgacgaagcggactactactgcggaacttgggactcctccttgggggcctgggtgttcggcggagggaccaagctcaccgtgcttggagcggccgcaactaccacccctgcccctcggccgccgactccggccccaaccatcgcaagccaacccctctccttgcgccccgaagcttgccgcccggccgcgggtggagccgtgcatacccgggggctggactttgcctgcgatatctacatttgggccccgctggccggcacttgcggcgtgctcctgctgtcgctggtcatcaccctttactgcaagaggggccggaagaagctgctttacatcttcaagcagccgttcatgcggcccgtgcagacgactcaggaagaggacggatgctcgtgcagattccctgaggaggaagaggggggatgcgaactgcgcgtcaagttctcacggtccgccgacgcccccgcatatcaacagggccagaatcagctctacaacgagctgaacctgggaaggagagaggagtacgacgtgctggacaagcgacgcggacgcgacccggagatgggggggaaaccacggcggaaaaaccctcaggaaggactgtacaacgaactccagaaagacaagatggcggaagcctactcagaaatcgggatgaagggagagcggaggaggggaaagggtcacgacgggctgtaccagggactgagcaccgccactaaggatacctacgatgccttgcatatgcaagcactcccaccccgg

SEQ ID NO: 126 - protein, 493 aa, Artificial Sequence
  source: /note="Description of Artificial Sequence: Synthetic polypeptide"
MLLLVTSLLLCELPHPAFLLIPQVQLQQWGAGLLKPSETLSLTCAVYGGSFSGYYWSWIRQPPGKGLEWIGEINHSGSTNYNPSLKSRVTISVDTSKNQFSLKLSSVTAADTAVYYCARGQVKYSSSLGYWGQGTLVTVSSGGGGSGGGGSGGGGSQSVLTQPPSVSAAPGQKVTISCSGSSSNIGNNFVSWYQQLPGTAPKLLIYEDNKRPSGIPDRFSGSRSGTSATLGITGLQTGDEADYYCGTWDSSLGAWVFGGGTKLTVLGAAATTTPAPRPPTPAPTIASQPLSLRPEACRPAAGGAVHTRGLDFACDIYIWAPLAGTCGVLLLSLVITLYCKRGRKKLLYIFKQPFMRPVQTTQEEDGCSCRFPEEEEGGCELRVKFSRSADAPAYQQGQNQLYNELNLGRREEYDVLDKRRGRDPEMGGKPRRKNPQEGLYNELQKDKMAEAYSEIGMKGERRRGKGHDGLYQGLSTATKDTYDALHMQALPPR

SEQ ID NO: 127 - DNA, 1467 bp, Artificial Sequence
  source: /note="Description of Artificial Sequence: Synthetic polynucleotide"
atgctgctgctggtgaccagcctgctgctgtgcgaactgccgcatccggcgtttctgctgattccgcaagtccaactcgtcgaaactggtggtggcctcgtgaagcctggaggatccctgcgcctttcctgtgccgcttccggctttactttctcgtcgtactccatgaactgggtcagacaggctcccggaaagggcctggaatgggtgtcctccatctcgtcctcatcctcctacatctattacgcggactccgtgaagggcagattcaccatttcccgggacaacgccaagaacagcttgtacctccaaatgaactccctgcgggcagaggacaccgccgtgtactactgcgcgagggatggggatttctggagcggagccatcgactactggggccagggaactctcgtgaccgtcagctccggtggtggtggaagcggaggcggaggttctggggggggaggatcagacattcagctgacccagtcgccatcctccctgagcgcctcagtgggggaccgcgtgactattacatgccaggcctcccaagatatctcgaactacctgaactggtatcagcagaagcctggaaaggccccgaagctgttgatctacgatgccagcaacctggagactggggtgccttcccggttctcgggatcaggctcgggcaccgatttcaccttcacgatcagcagcctgcagcccgaggacattgcaacctactactgccagcagtacgacaatctgccgctttttgggggaggcaccaagctggaaatcaaagcggccgcaactaccacccctgcccctcggccgccgactccggccccaaccatcgcaagccaacccctctccttgcgccccgaagcttgccgcccggccgcgggtggagccgtgcatacccgggggctggactttgcctgcgatatctacatttgggccccgctggccggcacttgcggcgtgctcctgctgtcgctggtcatcaccctttactgcaagaggggccggaagaagctgctttacatcttcaagcagccgttcatgcggcccgtgcagacgactcaggaagaggacggatgctcgtgcagattccctgaggaggaagaggggggatgcgaactgcgcgtcaagttctcacggtccgccgacgcccccgcatatcaacagggccagaatcagctctacaacgagctgaacctgggaaggagagaggagtacgacgtgctggacaagcgacgcggacgcgacccggagatgggggggaaaccacggcggaaaaaccctcaggaaggactgtacaacgaactccagaaagacaagatggcggaagcctactcagaaatcgggatgaagggagagcggaggaggggaaagggtcacgacgggctgtaccagggactgagcaccgccactaaggatacctacgatgccttgcatatgcaagcactcccaccccgg

SEQ ID NO: 128 - protein, 489 aa, Artificial Sequence
  source: /note="Description of Artificial Sequence: Synthetic polypeptide"
MLLLVTSLLLCELPHPAFLLIPQVQLVETGGGLVKPGGSLRLSCAASGFTFSSYSMNWVRQAPGKGLEWVSSISSSSSYIYYADSVKGRFTISRDNAKNSLYLQMNSLRAEDTAVYYCARDGDFWSGAIDYWGQGTLVTVSSGGGGSGGGGSGGGGSDIQLTQSPSSLSASVGDRVTITCQASQDISNYLNWYQQKPGKAPKLLIYDASNLETGVPSRFSGSGSGTDFTFTISSLQPEDIATYYCQQYDNLPLFGGGTKLEIKAAATTTPAPRPPTPAPTIASQPLSLRPEACRPAAGGAVHTRGLDFACDIYIWAPLAGTCGVLLLSLVITLYCKRGRKKLLYIFKQPFMRPVQTTQEEDGCSCRFPEEEEGGCELRVKFSRSADAPAYQQGQNQLYNELNLGRREEYDVLDKRRGRDPEMGGKPRRKNPQEGLYNELQKDKMAEAYSEIGMKGERRRGKGHDGLYQGLSTATKDTYDALHMQALPPR

SEQ ID NO: 129 - DNA, 1467 bp, Artificial Sequence
  source: /note="Description of Artificial Sequence: Synthetic polynucleotide"
atgctgctgctggtgaccagcctgctgctgtgcgaactgccgcatccggcgtttctgctgattccggaggtgcaattggtgcagtcaggtggtggagtggtgcagccaggaagatcccttagactctcgtgtgcggcgtcaggctttaccttctcctcgtactccatgaactgggtcagacaggcaccgggaaagggactggaatgggtgtcctccatctcgtcctcctcctcctacatctactacgccgatagcgtgaagggccggttcaccatttcgcgcgacaacgccaagaacaccctgtacctccaaatgaattcgctgcgggccgaagataccgctgtctattactgcgcccgcgacaactggggctcgctggactattggggccagggaaccctcgtcaccgtgtcaagcggagggggtggatccggaggcggaggatccggtggagggggaagcgacattcagatgactcagagcccgtcctccctgtctgcctccgtgggggatcgcgtgaccatcacatgccaggcctcacaagacatcagcaattacctgaactggtaccagcagaagcctggaaaggcccccaagctgctgatctacgatgccagcaacctggagactggggtgccttcaaggttctccggttccggaagcggcactgacttcaccttcactatctcgagcctgcaacccgaggacattgccacctactactgccagcagtacgacaaccttccgcacatgtacacgttcggccagggcaccaagctcgaaatcaaagcggccgcaactaccacccctgcccctcggccgccgactccggccccaaccatcgcaagccaacccctctccttgcgccccgaagcttgccgcccggccgcgggtggagccgtgcatacccgggggctggactttgcctgcgatatctacatttgggccccgctggccggcacttgcggcgtgctcctgctgtcgctggtcatcaccctttactgcaagaggggccggaagaagctgctttacatcttcaagcagccgttcatgcggcccgtgcagacgactcaggaagaggacggatgctcgtgcagattccctgaggaggaagaggggggatgcgaactgcgcgtcaagttctcacggtccgccgacgcccccgcatatcaacagggccagaatcagctctacaacgagctgaacctgggaaggagagaggagtacgacgtgctggacaagcgacgcggacgcgacccggagatgggggggaaaccacggcggaaaaaccctcaggaaggactgtacaacgaactccagaaagacaagatggcggaagcctactcagaaatcgggatgaagggagagcggaggaggggaaagggtcacgacgggctgtaccagggactgagcaccgccactaaggatacctacgatgccttgcatatgcaagcactcccaccccgg

SEQ ID NO: 130 - protein, 489 aa, Artificial Sequence
  source: /note="Description of Artificial Sequence: Synthetic polypeptide"
MLLLVTSLLLCELPHPAFLLIPEVQLVQSGGGVVQPGRSLRLSCAASGFTFSSYSMNWVRQAPGKGLEWVSSISSSSSYIYYADSVKGRFTISRDNAKNTLYLQMNSLRAEDTAVYYCARDNWGSLDYWGQGTLVTVSSGGGGSGGGGSGGGGSDIQMTQSPSSLSASVGDRVTITCQASQDISNYLNWYQQKPGKAPKLLIYDASNLETGVPSRFSGSGSGTDFTFTISSLQPEDIATYYCQQYDNLPHMYTFGQGTKLEIKAAATTTPAPRPPTPAPTIASQPLSLRPEACRPAAGGAVHTRGLDFACDIYIWAPLAGTCGVLLLSLVITLYCKRGRKKLLYIFKQPFMRPVQTTQEEDGCSCRFPEEEEGGCELRVKFSRSADAPAYQQGQNQLYNELNLGRREEYDVLDKRRGRDPEMGGKPRRKNPQEGLYNELQKDKMAEAYSEIGMKGERRRGKGHDGLYQGLSTATKDTYDALHMQALPPR

SEQ ID NO: 131 - DNA, 2293 bp, Artificial Sequence
  source: /note="Description of Artificial Sequence: Synthetic polynucleotide"
atgctcttgctcgtgacttctttgcttttgtgcgaacttccgcacccagccttccttttgatacctcaggtacagcttcaacaaagcggaccgggacttgttaagcattcccaaaccctttctctcacgtgtgcaattagcggcgatagtgtatcctctaattctgcggcctggaactggatacgacaatcaccaagccggggactcgagtggttgggccgaacctactatcggtccaaatggtataatgactacgcagtatccgtgaaatctcgcattacgatcaatccagacacctccaaaaatcaattttctctgcagttgaatagcgtgactcccgaggacacggccgtttactattgcgcccaggaagttgaaccccacgatgcatttgatatttggggccagggaaccatggtgacagtgagtagtgggggtggaggatctggaggaggcggtagcggcgggggcggcagtgatatccagatgacgcagtcaccttccagcgtgtatgcgagtgtgggggacaaggtcaccataacctgtcgcgctagccaagatgtcagcgggtggctggcttggtaccagcagaaaccaggtttggctcctcagcttttgatctcaggagcgagcacgcttcagggtgaggtcccaagtcgctttagtggctctggctccgggacagacttcacgttgacgatcagcagtttgcagcctgaggatttcgcgacctactactgccagcaagcgaaatattttccgtacactttcggtcaggggaccaaattggagatcaaaggtgggggtggttcaggcggcggaggctcaggcggcggcggtagcggaggaggcggaagcgggggtggcggatcagaagtgcaactcgttcagagtggcgcggaggttaagaaacccggtgcatctgtaaaggttagctgtaaggcatcaggatacacttttaccagctattacatgcattgggtgagacaggctcccggtcaggggctcgaatggatggggttgatcaacccgagtggtggttcaacatcttacgcccagaagtttcagggccgagtaacaatgactcgggacacgtctacctcaactgtgtatatggagctttccagcctgcgctcagaggatacagcagtctattactgcgcacggtcagacagaggtataacggccactgatgcgttcgatatctggggacaagggactatggtaactgtgtcttccggaggaggaggtagtggagggggaggaagcggtggggggggctcacagtccgttttgactcagccaccaagcgtctcagtcgcaccggggcgaatggcgaaaattacttgcggcgggagcgacataggcaacaagaatgtgcattggtaccaacagaaaccaggtcaagcacctgttctcgtggtgtatgatgactacgatcgcccaagcgggatcccggagcggttctctggatcaaattctggtgatgcagccactctgacaatatcaacggtggaagtcggtgacgaggctgattacttctgccaagtatgggatggcagcggagatccctactggatgtttggaggaggtactcaactgacagttctgggcgcggccgcaacgaccactcctgcaccccgccctccgactccggccccaaccattgccagccagcccctgtccctgcggccggaagcctgcagaccggctgccggcggagccgtccatacccggggactggatttcgcctgcgatatctatatctgggcaccactcgccggaacctgtggagtgctgctgctgtcccttgtgatcaccctgtactgcaagcgcggacggaagaaactcttgtacatcttcaagcagccgttcatgcgccctgtgcaaaccacccaagaagaggacgggtgctcctgccggttcccggaagaggaagagggcggctgcgaactgcgcgtgaagttttcccggtccgccgacgctccggcgtaccagcaggggcaaaaccagctgtacaacgaacttaacctcggtcgccgggaagaatatgacgtgctggacaagcggcggggaagagatcccgagatgggtggaaagccgcggcggaagaaccctcaggagggcttgtacaacgagctgcaaaaggacaaaatggccgaagcctactccgagattggcatgaagggagagcgcagacgcgggaagggacacgatggactgtaccagggactgtcaaccgcgactaaggacacttacgacgccctgcacatgcaggccctgcccccgcgct

SEQ ID NO: 132 - protein, 764 aa, Artificial Sequence
  source: /note="Description of Artificial Sequence: Synthetic polypeptide"
MLLLVTSLLLCELPHPAFLLIPQVQLQQSGPGLVKHSQTLSLTCAISGDSVSSNSAAWNWIRQSPSRGLEWLGRTYYRSKWYNDYAVSVKSRITINPDTSKNQFSLQLNSVTPEDTAVYYCAQEVEPHDAFDIWGQGTMVTVSSGGGGSGGGGSGGGGSDIQMTQSPSSVYASVGDKVTITCRASQDVSGWLAWYQQKPGLAPQLLISGASTLQGEVPSRFSGSGSGTDFTLTISSLQPEDFATYYCQQAKYFPYTFGQGTKLEIKGGGGSGGGGSGGGGSGGGGSGGGGSEVQLVQSGAEVKKPGASVKVSCKASGYTFTSYYMHWVRQAPGQGLEWMGLINPSGGSTSYAQKFQGRVTMTRDTSTSTVYMELSSLRSEDTAVYYCARSDRGITATDAFDIWGQGTMVTVSSGGGGSGGGGSGGGGSQSVLTQPPSVSVAPGRMAKITCGGSDIGNKNVHWYQQKPGQAPVLVVYDDYDRPSGIPERFSGSNSGDAATLTISTVEVGDEADYFCQVWDGSGDPYWMFGGGTQLTVLGAAATTTPAPRPPTPAPTIASQPLSLRPEACRPAAGGAVHTRGLDFACDIYIWAPLAGTCGVLLLSLVITLYCKRGRKKLLYIFKQPFMRPVQTTQEEDGCSCRFPEEEEGGCELRVKFSRSADAPAYQQGQNQLYNELNLGRREEYDVLDKRRGRDPEMGGKPRRKNPQEGLYNELQKDKMAEAYSEIGMKGERRRGKGHDGLYQGLSTATKDTYDALHMQALPPR

SEQ ID NO: 133 - DNA, 1476 bp, Artificial Sequence
  source: /note="Description of Artificial Sequence: Synthetic polynucleotide"
atgcttcttttggtgacttcccttttgctgtgcgagttgccacaccccgccttcctgcttattccccaggtacagcttcaacagagtgggccgggactggtgaaacactcccaaacactttctctgacgtgcgctatatcaggtgactctgtttcatctaattctgctgcgtggaactggattcgacaatctcccagtcgcgggttggaatggctgggacgaacatattatcggtctaagtggtataacgattatgctgtatctgttaaatctcgaattacgattaatcctgacacctccaagaaccagttctccctccagttgaactcagtcacaccggaagacactgcggtctactattgcgctcaagaagtcgagccacatgatgcattcgacatctggggccagggaacgatggtcaccgtcagcagtggcggcggcggatctgggggtggcggttctggcggtggaggatcagacatacaaatgacgcagagtccctcaagtgtgtacgcgagtgtgggggataaggtaactattacgtgcagagcgtcacaggatgttagtggatggcttgcctggtatcagcagaagccaggccttgctccacagctccttatcagtggtgcttctacacttcagggcgaggttccgagtagattctctggttctggatctggtactgacttcactcttacaatttcttctttgcaaccagaagactttgcgacttattactgccaacaggccaaatacttcccttatacatttggccaaggtaccaagttggagataaaggcggccgcaactaccacccctgcccctcggccgccgactccggccccaaccatcgcaagccaacccctctccttgcgccccgaagcttgccgcccggccgcgggtggagccgtgcatacccgggggctggactttgcctgcgatatctacatttgggccccgctggccggcacttgcggcgtgctcctgctgtcgctggtcatcaccctttactgcaagaggggccggaagaagctgctttacatcttcaagcagccgttcatgcggcccgtgcagacgactcaggaagaggacggatgctcgtgcagattccctgaggaggaagaggggggatgcgaactgcgcgtcaagttctcacggtccgccgacgcccccgcatatcaacagggccagaatcagctctacaacgagctgaacctgggaaggagagaggagtacgacgtgctggacaagcgacgcggacgcgacccggagatgggggggaaaccacggcggaaaaaccctcaggaaggactgtacaacgaactccagaaagacaagatggcggaagcctactcagaaatcgggatgaagggagagcggaggaggggaaagggtcacgacgggctgtaccagggactgagcaccgccactaaggatacctacgatgccttgcatatgcaagcactcccaccccgg

SEQ ID NO: 134 - protein, 492 aa, Artificial Sequence
  source: /note="Description of Artificial Sequence: Synthetic polypeptide"
MLLLVTSLLLCELPHPAFLLIPQVQLQQSGPGLVKHSQTLSLTCAISGDSVSSNSAAWNWIRQSPSRGLEWLGRTYYRSKWYNDYAVSVKSRITINPDTSKNQFSLQLNSVTPEDTAVYYCAQEVEPHDAFDIWGQGTMVTVSSGGGGSGGGGSGGGGSDIQMTQSPSSVYASVGDKVTITCRASQDVSGWLAWYQQKPGLAPQLLISGASTLQGEVPSRFSGSGSGTDFTLTISSLQPEDFATYYCQQAKYFPYTFGQGTKLEIKAAATTTPAPRPPTPAPTIASQPLSLRPEACRPAAGGAVHTRGLDFACDIYIWAPLAGTCGVLLLSLVITLYCKRGRKKLLYIFKQPFMRPVQTTQEEDGCSCRFPEEEEGGCELRVKFSRSADAPAYQQGQNQLYNELNLGRREEYDVLDKRRGRDPEMGGKPRRKNPQEGLYNELQKDKMAEAYSEIGMKGERRRGKGHDGLYQGLSTATKDTYDALHMQALPPR

SEQ ID NO: 135 - DNA, 1476 bp, Artificial Sequence
  source: /note="Description of Artificial Sequence: Synthetic polynucleotide"
atgttgctgctcgtgacctcgctccttctgtgcgagctgccccatccggcttttctgctcatccctcaagtgcagctgcagcagtccggtcctggactggtcaagccgtcccagactctgagcctgacttgcgccattagcgggaactcagtctcgtccaattcggcggcctggaactggatccggcagtcaccatcaaggggcctggaatggctcgggcgcacttactaccggtccaaatggtataacgactacgccgtgtccgtgaagtcccggatcaccattaaccccgacacctcgaagaaccagttctcactccaactgaacagcgtgacccccgaggataccgcggtgtactactgcgcacaagaagtggaaccgcaggacgccttcgacatttggggacagggaacgatggtcacagtgtcgtccggtggaggaggttccggaggcggtggatctggaggcggaggttcggatatccagatgacccagagcccctcctcggtgtccgcatccgtgggcgataaggtcaccattacctgtagagcgtcccaggacgtgtccggatggctggcctggtaccagcagaagccaggcttggctcctcaactgctgatctttggcgccagcactcttcagggggaggtgccatcacgcttctccggaggtggttccggcaccgacttcaccctgaccatcagcagcctccagcctgaggacttcgccacttactactgccaacaggccaagtacttcccctataccttcggacaaggcactaagctggaaatcaaggcggccgcaactaccacccctgcccctcggccgccgactccggccccaaccatcgcaagccaacccctctccttgcgccccgaagcttgccgcccggccgcgggtggagccgtgcatacccgggggctggactttgcctgcgatatctacatttgggccccgctggccggcacttgcggcgtgctcctgctgtcgctggtcatcaccctttactgcaagaggggccggaagaagctgctttacatcttcaagcagccgttcatgcggcccgtgcagacgactcaggaagaggacggatgctcgtgcagattccctgaggaggaagaggggggatgcgaactgcgcgtcaagttctcacggtccgccgacgcccccgcatatcaacagggccagaatcagctctacaacgagctgaacctgggaaggagagaggagtacgacgtgctggacaagcgacgcggacgcgacccggagatgggggggaaaccacggcggaaaaaccctcaggaaggactgtacaacgaactccagaaagacaagatggcggaagcctactcagaaatcgggatgaagggagagcggaggaggggaaagggtcacgacgggctgtaccagggactgagcaccgccactaaggatacctacgatgccttgcatatgcaagcactcccaccccgg

SEQ ID NO: 136 - protein, 492 aa, Artificial Sequence
  source: /note="Description of Artificial Sequence: Synthetic polypeptide"
MLLLVTSLLLCELPHPAFLLIPQVQLQQSGPGLVKPSQTLSLTCAISGNSVSSNSAAWNWIRQSPSRGLEWLGRTYYRSKWYNDYAVSVKSRITINPDTSKNQFSLQLNSVTPEDTAVYYCAQEVEPQDAFDIWGQGTMVTVSSGGGGSGGGGSGGGGSDIQMTQSPSSVSASVGDKVTITCRASQDVSGWLAWYQQKPGLAPQLLIFGASTLQGEVPSRFSGGGSGTDFTLTISSLQPEDFATYYCQQAKYFPYTFGQGTKLEIKAAATTTPAPRPPTPAPTIASQPLSLRPEACRPAAGGAVHTRGLDFACDIYIWAPLAGTCGVLLLSLVITLYCKRGRKKLLYIFKQPFMRPVQTTQEEDGCSCRFPEEEEGGCELRVKFSRSADAPAYQQGQNQLYNELNLGRREEYDVLDKRRGRDPEMGGKPRRKNPQEGLYNELQKDKMAEAYSEIGMKGERRRGKGHDGLYQGLSTATKDTYDALHMQALPPR

SEQ ID NO: 137 - DNA, 190 bp, Artificial Sequence
  source: /note="Description of Artificial Sequence: Synthetic polynucleotide"
ggtacctgagctcagttctgagaaaagtagttctgagaaaagtagttctgagaaaagtagttctgagaaaagtagttctgagaaaagtctcgaggatatcaagatctggcctcggcggccaagcttagacactagagggtatataatggaagctcgacttccagcttggcaatccggtactgttggtaaa

SEQ ID NO: 138 - DNA, 214 bp, Artificial Sequence
  source: /note="Description of Artificial Sequence: Synthetic polynucleotide"
tgagctctgagtcagtgactcagtgagtcagtgactcagtgagtcagtgactcagctcgaggatctcgctagcgggaatttccggggactttccgggaatttccggggactttccgggaatttccagatctggcctcggcggccaagcttagacactagagggtatataatggaagctcgacttccagcttggcaatccggtactgttggtaaa

SEQ ID NO: 139 - DNA, 1670 bp, Artificial Sequence
  source: /note="Description of Artificial Sequence: Synthetic polynucleotide"
ggtacctgagctcagttctgagaaaagtagttctgagaaaagtagttctgagaaaagtagttctgagaaaagtagttctgagaaaagtctcgaggatatcaagatctggcctcggcggccaagcttagacactagagggtatataatggaagctcgacttccagcttggcaatccggtactgttggtaaaggcgcgccccaccatgctgctgctggtcaccagcctgctgctgtgcgagctccctcaccccgcctttctgcttatcccggacattcagatgacacagaccacctcgagcttgtccgcgtcgctgggcgatcgcgtgaccatctcctgccgggcctcccaagacatttcaaagtatctcaactggtaccagcagaagccggacggaaccgtgaaactgctgatctaccataccagccgcctgcactccggcgtgccgtcccgcttctccggatcgggttccggaactgactactcactgactatctccaacttggaacaagaggacatcgccacttacttctgtcaacaaggaaatacccttccctacaccttcggggggggtaccaagctggagatcactgggggcggaggctccggtggaggcggatccggcggtggagggagcgaagtcaagctgcaggaatcaggaccaggactcgtggcgccatcccagtccctgtcggtgacctgtactgtctccggagtcagcctccccgattacggagtgtcatggattaggcaacccccaagaaaagggctggaatggctcggagtgatctggggctccgaaaccacctactacaactcggcgctgaagtcccggctgaccatcatcaaggacaactccaagagccaagtgttcttgaagatgaacagcttgcagaccgacgataccgcaatctactactgtgccaagcactattactacggggggtcttacgccatggactactggggacagggcacctccgtgactgtgtcgtccgcggccgcgcccgcccctcggcccccgactcctgccccgacgatcgcttcccaacctctctcgctgcgcccggaagcatgccggcccgccgccggtggcgctgtccacactcgcggactggactttgataccgcactggcggccgtgatctgtagcgccctggccaccgtgctgctggcgctgctcatcctttgcgtgatctactgcaagcggcagcctaggcgaaagaagctcctctacattttcaagcaacccttcatgcgccccgtgcaaaccacccaggaggaggatggatgctcatgccggttccctgaggaagaagagggcggttgcgagctcagagtgaaattcagccggtcggctgacgccccggcgtaccagcagggccagaaccagctgtacaatgagctcaacctggggcgccgcgaagagtacgacgtgctggacaagaggagaggcagagatccggaaatgggcggaaagccaaggcggaagaacccgcaggaaggtctttacaacgaactgcagaaggacaagatggccgaggcctactccgagattgggatgaagggagaaagacggaggggaaagggacatgacggactttaccagggcctgagcactgccacgaaggacacctatgatgccctgcacatgcaggcgctgccgcctcgg

SEQ ID NO: 140 - DNA, 1694 bp, Artificial Sequence
  source: /note="Description of Artificial Sequence: Synthetic polynucleotide"
tgagctctgagtcagtgactcagtgagtcagtgactcagtgagtcagtgactcagctcgaggatctcgctagcgggaatttccggggactttccgggaatttccggggactttccgggaatttccagatctggcctcggcggccaagcttagacactagagggtatataatggaagctcgacttccagcttggcaatccggtactgttggtaaaggcgcgccccaccatgctgctgctggtcaccagcctgctgctgtgcgagctccctcaccccgcctttctgcttatcccggacattcagatgacacagaccacctcgagcttgtccgcgtcgctgggcgatcgcgtgaccatctcctgccgggcctcccaagacatttcaaagtatctcaactggtaccagcagaagccggacggaaccgtgaaactgctgatctaccataccagccgcctgcactccggcgtgccgtcccgcttctccggatcgggttccggaactgactactcactgactatctccaacttggaacaagaggacatcgccacttacttctgtcaacaaggaaatacccttccctacaccttcggggggggtaccaagctggagatcactgggggcggaggctccggtggaggcggatccggcggtggagggagcgaagtcaagctgcaggaatcaggaccaggactcgtggcgccatcccagtccctgtcggtgacctgtactgtctccggagtcagcctccccgattacggagtgtcatggattaggcaacccccaagaaaagggctggaatggctcggagtgatctggggctccgaaaccacctactacaactcggcgctgaagtcccggctgaccatcatcaaggacaactccaagagccaagtgttcttgaagatgaacagcttgcagaccgacgataccgcaatctactactgtgccaagcactattactacggggggtcttacgccatggactactggggacagggcacctccgtgactgtgtcgtccgcggccgcgcccgcccctcggcccccgactcctgccccgacgatcgcttcccaacctctctcgctgcgcccggaagcatgccggcccgccgccggtggcgctgtccacactcgcggactggactttgataccgcactggcggccgtgatctgtagcgccctggccaccgtgctgctggcgctgctcatcctttgcgtgatctactgcaagcggcagcctaggcgaaagaagctcctctacattttcaagcaacccttcatgcgccccgtgcaaaccacccaggaggaggatggatgctcatgccggttccctgaggaagaagagggcggttgcgagctcagagtgaaattcagccggtcggctgacgccccggcgtaccagcagggccagaaccagctgtacaatgagctcaacctggggcgccgcgaagagtacgacgtgctggacaagaggagaggcagagatccggaaatgggcggaaagccaaggcggaagaacccgcaggaaggtctttacaacgaactgcagaaggacaagatggccgaggcctactccgagattgggatgaagggagaaagacggaggggaaagggacatgacggactttaccagggcctgagcactgccacgaaggacacctatgatgccctgcacatgcaggcgctgccgcctcgg

SEQ ID NO: 141 - DNA, 735 bp, Artificial Sequence
  source: /note="Description of Artificial Sequence: Synthetic polynucleotide"
gacattcagatgactcagaccacctcctccctgtccgcctccctgggcgaccgcgtgaccatctcatgccgcgccagccaggacatctcgaagtacctcaactggtaccagcagaagcccgacggaaccgtgaagctcctgatctaccacacctcccggctgcacagcggagtgccgtctagattctcgggttcggggtcgggaactgactactcccttactatttccaacctggagcaggaggatattgccacctacttctgccaacaaggaaacaccctgccgtacacttttggcgggggaaccaagctggaaatcactggcagcacatccggttccgggaagcccggctccggagagggcagcaccaagggggaagtcaagctgcaggaatcaggacctggcctggtggccccgagccagtcactgtccgtgacttgtactgtgtccggagtgtcgctcccggattacggagtgtcctggatcaggcagccacctcggaaaggattggaatggctcggagtcatctggggttccgaaaccacctattacaactcggcactgaaatccaggctcaccattatcaaggataactccaagtcacaagtgttcctgaagatgaatagcctgcagactgacgacacggcgatctactattgcgccaagcactactactacggcggatcctacgctatggactactggggccaggggaccagcgtgaccgtgtcatcc

SEQ ID NO: 142 - DNA, 1473 bp, Artificial Sequence
  source: /note="Description of Artificial Sequence: Synthetic polynucleotide"
atgctccttctcgtgacctccctgcttctctgcgaactgccccatcctgccttcctgctgattcccgaggtgcagttgcaacagtcaggagctgaactggtcaagccaggagccagcgtgaagatgagctgcaaggcctccggttacaccttcacctcctacaacatgcactgggtgaaacagaccccgggacaagggctcgaatggattggcgccatctaccccgggaatggcgatacttcgtacaaccagaagttcaagggaaaggccaccctgaccgccgacaagagctcctccaccgcgtatatgcagttgagctccctgacctccgaggactccgccgactactactgcgcacggtccaactactatggaagctcgtactggttcttcgatgtctggggggccggcaccactgtgaccgtcagctccgggggcggaggatccggtggaggcggaagcgggggtggaggatccgacattgtgctgactcagtccccggcaatcctgtcggcctcaccgggcgaaaaggtcacgatgacttgtagagcgtcgtccagcgtgaactacatggattggtaccaaaagaagcctggatcgtcacccaagccttggatctacgctacatctaacctggcctccggcgtgccagcgcggttcagcgggtccggctcgggcacctcatactcgctgaccatctcccgcgtggaggctgaggacgccgcgacctactactgccagcagtggtccttcaacccgccgacttttggaggcggtactaagctggagatcaaagcggccgcaactaccacccctgcccctcggccgccgactccggccccaaccatcgcaagccaacccctctccttgcgccccgaagcttgccgcccggccgcgggtggagccgtgcatacccgggggctggactttgcctgcgatatctacatttgggccccgctggccggcacttgcggcgtgctcctgctgtcgctggtcatcaccctttactgcaagaggggccggaagaagctgctttacatcttcaagcagccgttcatgcggcccgtgcagacgactcaggaagaggacggatgctcgtgcagattccctgaggaggaagaggggggatgcgaactgcgcgtcaagttctcacggtccgccgacgcccccgcatatcaacagggccagaatcagctctacaacgagctgaacctgggaaggagagaggagtacgacgtgctggacaagcgacgcggacgcgacccggagatgggggggaaaccacggcggaaaaaccctcaggaaggactgtacaacgaactccagaaagacaagatggcggaagcctactcagaaatcgggatgaagggagagcggaggaggggaaagggtcacgacgggctgtaccagggactgagcaccgccactaaggatacctacgatgccttgcatatgcaagcactcccaccccgg

SEQ ID NO: 143 - protein, 491 aa, Artificial Sequence
  source: /note="Description of Artificial Sequence: Synthetic polypeptide"
MLLLVTSLLLCELPHPAFLLIPEVQLQQSGAELVKPGASVKMSCKASGYTFTSYNMHWVKQTPGQGLEWIGAIYPGNGDTSYNQKFKGKATLTADKSSSTAYMQLSSLTSEDSADYYCARSNYYGSSYWFFDVWGAGTTVTVSSGGGGSGGGGSGGGGSDIVLTQSPAILSASPGEKVTMTCRASSSVNYMDWYQKKPGSSPKPWIYATSNLASGVPARFSGSGSGTSYSLTISRVEAEDAATYYCQQWSFNPPTFGGGTKLEIKAAATTTPAPRPPTPAPTIASQPLSLRPEACRPAAGGAVHTRGLDFACDIYIWAPLAGTCGVLLLSLVITLYCKRGRKKLLYIFKQPFMRPVQTTQEEDGCSCRFPEEEEGGCELRVKFSRSADAPAYQQGQNQLYNELNLGRREEYDVLDKRRGRDPEMGGKPRRKNPQEGLYNELQKDKMAEAYSEIGMKGERRRGKGHDGLYQGLSTATKDTYDALHMQALPPR

SEQ ID NO: 144 - DNA, 750 bp, Artificial Sequence
  source: /note="Description of Artificial Sequence: Synthetic polynucleotide"
gaagtgcaattggtgcagagcggtggaggacttgtgaaacctggtggatccctgagactttcctgtgccgcttcgggcttcaccttctcggactactacatgtcctggattcgccaggcccctggaaagggactggaatgggtgtcatacatcagctcctccggttccaccatctactatgccgattccgtgaagggcagattcaccatctcgcgcgacaacgccaagaacactctctatctgcaaatgaactcactgcgggctgaggacaccgcggtctactactgcgcccgggacctcagcggaaagtccagcggatggtcccattacttcgattactggggacagggaaccctggtcaccgtgtccagcggcggggggggctcgggtggcggcggctccggcggcggcgggagcaacttcatgctgactcagccccactccgtgtccgagagcccgggaaagaccgtgactatttcgtgcacacggtcctccgggagcattgcgaacaactacgtgcagtggtaccagcagcggcccgatagggccccaaccactgtgatctacgaagatgaccagcggccgtctggagtcccggaccgcttctcggggtccatcgactcatcatccaattccgcatcgctgacgatcagcggactgaagatcgaggacgaagccgattactactgccagtcctacgacggcaccaactgggtctttgggggtggaaccaagctgactgtgctcgga

SEQ ID NO: 145 - protein, 250 aa, Artificial Sequence
  source: /note="Description of Artificial Sequence: Synthetic polypeptide"
EVQLVQSGGGLVKPGGSLRLSCAASGFTFSDYYMSWIRQAPGKGLEWVSYISSSGSTIYYADSVKGRFTISRDNAKNTLYLQMNSLRAEDTAVYYCARDLSGKSSGWSHYFDYWGQGTLVTVSSGGGGSGGGGSGGGGSNFMLTQPHSVSESPGKTVTISCTRSSGSIANNYVQWYQQRPDRAPTTVIYEDDQRPSGVPDRFSGSIDSSSNSASLTISGLKIEDEADYYCQSYDGTNWVFGGGTKLTVLG

SEQ ID NO: 146 - DNA, 729 bp, Artificial Sequence
  source: /note="Description of Artificial Sequence: Synthetic polynucleotide"
gaagtgcaacttgtcgaaagcggtggaggtcttgtccaacctggtcgctccctgaggctctcgtgtgccgcgagcggattcaccttctcatcgtacgctatgtcctgggtcagacaggctcctggaaagggcctggaatgggtggccgtgatctcctacgacggcagcaacaagtattacgccgactcagtgaagggccggttcaccatttcccgggacaacagcaagaacaccctgtacttgcaaatgaactccctgcgggccgaggataccgcggtgtactactgcgcccacctccgctttggatacggaatggatgtctggggacagggaactaccgtgaccgtgtcgtccgggggggggggaagcggcggcgggggatcgggtggcggcggatcccagactgtggtcacccaagagccttcactgaccgtgtccccgggtggcaccgtgacgctgacttgcgcgtcatctaccggggccgtgacctcggaccactacccctgctggttccagcagaaacccggacatccaccgagagccctggtgtactccactgacaccatccactcctggactccggcccggttctccggaagcctcctgggcgggaaggccgcactgacagtgtccggagtgcagcccgaggatgaagccgactactactgtctgctctactatgggggagcacgcgtgttcggtggcggcactcagctgaccgtgctggga

SEQ ID NO: 147 - protein, 243 aa, Artificial Sequence
  source: /note="Description of Artificial Sequence: Synthetic polypeptide"
EVQLVESGGGLVQPGRSLRLSCAASGFTFSSYAMSWVRQAPGKGLEWVAVISYDGSNKYYADSVKGRFTISRDNSKNTLYLQMNSLRAEDTAVYYCAHLRFGYGMDVWGQGTTVTVSSGGGGSGGGGSGGGGSQTVVTQEPSLTVSPGGTVTLTCASSTGAVTSDHYPCWFQQKPGHPPRALVYSTDTIHSWTPARFSGSLLGGKAALTVSGVQPEDEADYYCLLYYGGARVFGGGTQLTVLG

SEQ ID NO: 148 - DNA, 723 bp, Artificial Sequence
  source: /note="Description of Artificial Sequence: Synthetic polynucleotide"
caagtccaactcgtccagtccggtgccgaagtcaagaagcctggctcatccgtgaaagtgtcctgcaaagcatcgggcggaaccttctcctcctatgccatttcctgggtccgccaggcaccgggccagggtctggagtggatgggcgggattatccctatcttcggaactgccaaccacgcccaaaagttccagggacgcgtgaccattaccgccgatgaatcaacctcaaccgcctacatggaactgtccagcttgaggtccgaggacaccgccgtgtactactgcgcgttcatgatggtgccggagtactactttgactactggggccagggaacccttgtgaccgtgtcgtccggtggtggcggatccgggggggggggatctgggggcggcggaagcgatatccagatgacccagtcgccatcgagcctgtccgcttccgtgggcgacagagtgacgatcacttgccgggcttcacaaggcatcagaaatgacctgggctggtatcagcagaagcccggagaagcgcccaagcggctgatctacgcggccagcaccctgcaaaacggagtgccttcgcggttctccgggagcggctccggaactgacttcactctgactattaacagcctccagcccgaggatttcgccacatactactgtcagcagtacaacagctacccgtacaccttcggacagggaactaagctcgaaatcaag

SEQ ID NO: 149 - protein, 241 aa, Artificial Sequence
  source: /note="Description of Artificial Sequence: Synthetic polypeptide"
QVQLVQSGAEVKKPGSSVKVSCKASGGTFSSYAISWVRQAPGQGLEWMGGIIPIFGTANHAQKFQGRVTITADESTSTAYMELSSLRSEDTAVYYCAFMMVPEYYFDYWGQGTLVTVSSGGGGSGGGGSGGGGSDIQMTQSPSSLSASVGDRVTITCRASQGIRNDLGWYQQKPGEAPKRLIYAASTLQNGVPSRFSGSGSGTDFTLTINSLQPEDFATYYCQQYNSYPYTFGQGTKLEIK

SEQ ID NO: 150 - DNA, 756 bp, Artificial Sequence
  source: /note="Description of Artificial Sequence: Synthetic polynucleotide"
caactccaactccaagaatctggaccaggcctcgtgaagccctcccaaactctgtccctgacctgtaccgtgtcgggtggaagcatttcgagcggtggatactactggtcctggatcaggcagcatcctggaaagggactggagtggattgggtacatctactactccggctcaacctactacaacccgtccttgaaatcgcgcgtgacgatctccgtggacacttcaaagaaccagttcagcctgaagctttcctccgtgaccgcggccgatacagcggtgtactactgcgctcgggatcagagcgtggccgaccctggtggcggctactactactacggaatggatgtctggggacagggaaccaccgtgactgtgtccagcgggggcggcggatccgggggggggggatcgggcggcggcggttcgcagtccgtgctgacccagccacctagcgtgtcagtggcaccgggacagaccgcctccatttcctgcgggggaaatgacttcggtagccgctccgtgtcatggtatcaccagaagccgggacaggccccggtgctggtcatctatgacgacaacgacagaccctcgggcatccccgaacggttttcgggaagcacctccggagacactgccaccctgaccatctcccgggtcgaggtcggcgatgaagccgattactactgccaagtctgggacgacgactccgaccactgggtgttcggcggcggaactaagctgactgtgctgggg

SEQ ID NO: 151 - protein, 252 aa, Artificial Sequence
  source: /note="Description of Artificial Sequence: Synthetic polypeptide"
QLQLQESGPGLVKPSQTLSLTCTVSGGSISSGGYYWSWIRQHPGKGLEWIGYIYYSGSTYYNPSLKSRVTISVDTSKNQFSLKLSSVTAADTAVYYCARDQSVADPGGGYYYYGMDVWGQGTTVTVSSGGGGSGGGGSGGGGSQSVLTQPPSVSVAPGQTASISCGGNDFGSRSVSWYHQKPGQAPVLVIYDDNDRPSGIPERFSGSTSGDTATLTISRVEVGDEADYYCQVWDDDSDHWVFGGGTKLTVLG

SEQ ID NO: 152 - DNA, 723 bp, Artificial Sequence
  source: /note="Description of Artificial Sequence: Synthetic polynucleotide"
caggtgcagctgcaggagtccggcccaggactggtgaagccttcggagaccctgtccctcacctgcactgtctctggtggctccatcagcagtagtagttactactggggctggatccgccagcccccagggaaggggctggagtggattgggagtatctattatagtgggagcacctactacaacccgtccctcaagagtcgagtcaccatacccgtagacacgtccaagaaccagttctccctgaagctgagctctgtgaccgccgcagacacggctgtgtattactgtgcgagacacctggggggtgatgcttttgatatctggggccaagggaccacggtcaccgtctcctcaggaggtggcgggtctggtggtggcggtagcggtggaggcggatccctgcctgtgctgactcagcccccctcggtgtcagtggccccaggacagacggccaggattacctgtggggggaacaacattggaagtaaaagtgtgcactggtaccagcagaagccaggccaggcccctgtgctggtcgtctatgatgatagcgaccggccctcagggatccctgagcgattctctggctccaactctgggaacacagccactctgaccatcagcgggacccaggctatggatgaggctgactacttctgtcagtcttatgatagcagcaatcccgtggtattcggcggagggacccagctcaccgtttta

SEQ ID NO: 153 - protein, 241 aa, Artificial Sequence
  source: /note="Description of Artificial Sequence: Synthetic polypeptide"
QVQLQESGPGLVKPSETLSLTCTVSGGSISSSSYYWGWIRQPPGKGLEWIGSIYYSGSTYYNPSLKSRVTIPVDTSKNQFSLKLSSVTAADTAVYYCARHLGGDAFDIWGQGTTVTVSSGGGGSGGGGSGGGGSLPVLTQPPSVSVAPGQTARITCGGNNIGSKSVHWYQQKPGQAPVLVVYDDSDRPSGIPERFSGSNSGNTATLTISGTQAMDEADYFCQSYDSSNPVVFGGGTQLTVL

SEQ ID NO: 154 - DNA, 732 bp, Artificial Sequence
  source: /note="Description of Artificial Sequence: Synthetic polynucleotide"
caggcggcccaggtacagctgcagcagtcaggggctgaggtgaagaagcctgggtcctcggtgaaggtctcctgcaaggcttctggaggcaccttcagcagctatgctatcagctgggtgcgacaggcccctggacaagggcttgagtggatgggatggatcaaccctaacagtggtggcacaaactatgcacagaggtttcagggcagggtcaccatgaccagggacacgtccatcagcacagcctacatggagctgagcaggctgagatctgacgacacggccgtgtattactgtgcgagttataatgatgcttttgatatctggggccaaggcaccctggtcaccgtctcctcaggaggtggcgggtctggtggtggcggtagcggtggtggcggatccaattttatgctgactcagccccactctgtgtcggagtctccggggaagacggtaaccatctcctgcacccgcagcagtggcagcattgccagcaactatgtgcagtggtaccagcagcgcccgggcagtgcccccaccattgtgatctatgaggatgatcaaagaccctctggggtccctgatcggttctctggctccatcgacacctcctccaactctgcctccctcaccatctctggactgcagagtgaggacgaggctgactactactgtcagtcttatgagcccggcaatggggtattcggcggagggaccaaggtcaccgtccta

SEQ ID NO: 155 - protein, 244 aa, Artificial Sequence
  source: /note="Description of Artificial Sequence: Synthetic polypeptide"
QAAQVQLQQSGAEVKKPGSSVKVSCKASGGTFSSYAISWVRQAPGQGLEWMGWINPNSGGTNYAQRFQGRVTMTRDTSISTAYMELSRLRSDDTAVYYCASYNDAFDIWGQGTLVTVSSGGGGSGGGGSGGGGSNFMLTQPHSVSESPGKTVTISCTRSSGSIASNYVQWYQQRPGSAPTIVIYEDDQRPSGVPDRFSGSIDTSSNSASLTISGLQSEDEADYYCQSYEPGNGVFGGGTKVTVL

SEQ ID NO: 156 - DNA, 744 bp, Artificial Sequence
  source: /note="Description of Artificial Sequence: Synthetic polynucleotide"
caagaacagcttgtagagtccggcggtagattggtgacaccgggggggagccttaccctgtcttgtaaggcatctgggttcgatttcagtgcgtattatatgagctgggttcggcaggcgcccgggaaggggctggaatggatagccactatatacccgtcatccggcaagacttactacgcgacttgggtaaacgggaggtttacgataagctcagataacgcccaaaacacggttgatctccaaatgaatagcttgaccgccgctgatagggcgacctatttctgtgcgcgggactcttacgctgatgacggggccctcttcaatatatggggaccgggaacgctcgtaaccatatcatctggaggaggtgggagcggaggcggagggtcaggtgggggcgggagcgaactcgtacttacacaatctccaagcgtaagcgcagcgttggggagtccagcaaagatcacctgcactttgtcaagcgcccacaaaacggatacgatagattggtatcagcaactccaaggtgaagcgccacgatatctcatgcaggtacagagcgacgggagttatactaagaggcccggggtcccagacagattcagtggcagcagttcaggtgccgacagatacctgataataccctcagttcaagccgatgatgaagccgattactactgtggggctgactacataggtgggtatgttttcgggggcggcactcaattgacagttacaggg

SEQ ID NO: 157 - protein, 248 aa, Artificial Sequence
  source: /note="Description of Artificial Sequence: Synthetic polypeptide"
QEQLVESGGRLVTPGGSLTLSCKASGFDFSAYYMSWVRQAPGKGLEWIATIYPSSGKTYYATWVNGRFTISSDNAQNTVDLQMNSLTAADRATYFCARDSYADDGALFNIWGPGTLVTISSGGGGSGGGGSGGGGSELVLTQSPSVSAALGSPAKITCTLSSAHKTDTIDWYQQLQGEAPRYLMQVQSDGSYTKRPGVPDRFSGSSSGADRYLIIPSVQADDEADYYCGADYIGGYVFGGGTQLTVTG

SEQ ID NO: 158 - DNA, 720 bp, Artificial Sequence
  source: /note="Description of Artificial Sequence: Synthetic polynucleotide"
gaagtgcaactcgtcgaaactggagccgaagtgaaaaagcctggagcgtccgtcaaagtgtcgtgcaaggcctccggctacaccttcacgacctactacgtgcactgggtcagacaggctccgggtcaagggctggagtggatgggcatcattaacccctccggtggaagcacctcctatgcgcaaaagttccagggtcgcgtcaccatgactcgcgatacctccacttccactgtgtacatggaactgagctccctgaggtccgaggacaccgccgtgtactactgcgcacgggatggaggcttgggcggctacgaggcttggggacagggcaccctcgtgactgtgtcaagcggagggggtggatccggagggggaggatcaggcggtggtggaagcgatatccagcttacccagtcgccttccgcgctgtctgcatcggccggcgacagagtgacaattacctgtcaagccagccaggacatctccaactatctgaactggtaccagcagaagcccggaaaggctccgaagctgctgatctacgacgccagcaacctggaacggggcgtgccatcacggttctcgggatcagggtcgggcactgagttcaccttcaccatctcctccctccaacccgaggacattgccacctactactgccagcagtacgacaacctcccgatcacctttggacaggggactcgcctggaaatcaag

SEQ ID NO: 159 - protein, 240 aa, Artificial Sequence
  source: /note="Description of Artificial Sequence: Synthetic polypeptide"
EVQLVETGAEVKKPGASVKVSCKASGYTFTTYYVHWVRQAPGQGLEWMGIINPSGGSTSYAQKFQGRVTMTRDTSTSTVYMELSSLRSEDTAVYYCARDGGLGGYEAWGQGTLVTVSSGGGGSGGGGSGGGGSDIQLTQSPSALSASAGDRVTITCQASQDISNYLNWYQQKPGKAPKLLIYDASNLERGVPSRFSGSGSGTEFTFTISSLQPEDIATYYCQQYDNLPITFGQGTRLEIK

SEQ ID NO: 160 - DNA, 759 bp, Artificial Sequence
  source: /note="Description of Artificial Sequence: Synthetic polynucleotide"
gaagtgcaattggtccagagcggaggaggacttgtgaagccaggcggatccctgagattgtcatgcgccgcatcggggttcaccttttcctcctactccatgaactgggtcagacaggcgcccggaaagggacttgaatgggtgtcgtccatttcctcctcctcgtcctacatctactacgccgactccgtgaagggccgcttcaccatctcccgggacaacgccaagaacagcctgtatctccaaatgaactccctgcgggccgaagatactgctgtgtattactgcgctcgggacttcccgtacgactcatcgggctattactcggacgcgttcgatatctggggccagggaactatggtcaccgtcagctctggtggcggtggttccggagggggtggatccggtggcggaggatcagagattgtgctgacccagtccccgctgtcactgcccgtgactccgggagagcctgcctcgatctcgtgtcggtccagccagtccctgctgcactcgaatgggtacaactacctcgattggtacctccaaaagcctgggcagtcaccccaactgctgatctacctcgggagcaacagagccagcggagtgcctgaccgctttagcggttccggatccggcaccgacttcaccctgaaaatcagccgggtggaagccgaggatgtcggcgtgtactactgcatgcaggcactgcagactctggggtacaccttcggccagggcacgaagctcgagatcaag

SEQ ID NO: 161 - protein, 253 aa, Artificial Sequence
  source: /note="Description of Artificial Sequence: Synthetic polypeptide"
EVQLVQSGGGLVKPGGSLRLSCAASGFTFSSYSMNWVRQAPGKGLEWVSSISSSSSYIYYADSVKGRFTISRDNAKNSLYLQMNSLRAEDTAVYYCARDFPYDSSGYYSDAFDIWGQGTMVTVSSGGGGSGGGGSGGGGSEIVLTQSPLSLPVTPGEPASISCRSSQSLLHSNGYNYLDWYLQKPGQSPQLLIYLGSNRASGVPDRFSGSGSGTDFTLKISRVEAEDVGVYYCMQALQTLGYTFGQGTKLEIK

SEQ ID NO: 162 - DNA, 747 bp, Artificial Sequence
  source: /note="Description of Artificial Sequence: Synthetic polynucleotide"
caagtgcaactcgtccaatccggtgccgaagtcaagaagcctggttcctccgtgaaagtgtcgtgcaaagccagcggcgggacttttagctcctacgcgatcagctgggtcagacaggcccctggacaaggcctcgagtggatgggcggcatcattccgattttcggtaccgccaactacgcccagaagttccagggacgcgtgaccattactaccgacgagagcacctcaaccgcatacatggaactgtccagcctgcgctccgaggacacggctgtgtactattgcgccagacggggatggggaggattctcctccggctccgcattcgacatctggggacagggcactatggtcactgtgtcatccgggggaggaggatcaggcggtggaggatccggtggtggcggatccaacttcatgctgacccagccccactcagtgtcggaatcgcccggcaacaccgtgactatcagctgcaccggatccagcgggaccatcggctctaatttcgtgcagtggtaccagcagtccccagggagagctccgaccctgttgatctacgaggacacaaagcggccaagcggagtgccgcctagattcgccggctccgtggattcctcgtccaactcggcgtcgctgaccatcagcggactcaagactgaagatgaagccgactactactgtcagtcctacgactcgagcaactgggtgtttgggggcgggactaagctgaccgtgcttgga

SEQ ID NO: 163 - protein, 249 aa, Artificial Sequence
  source: /note="Description of Artificial Sequence: Synthetic polypeptide"
QVQLVQSGAEVKKPGSSVKVSCKASGGTFSSYAISWVRQAPGQGLEWMGGIIPIFGTANYAQKFQGRVTITTDESTSTAYMELSSLRSEDTAVYYCARRGWGGFSSGSAFDIWGQGTMVTVSSGGGGSGGGGSGGGGSNFMLTQPHSVSESPGNTVTISCTGSSGTIGSNFVQWYQQSPGRAPTLLIYEDTKRPSGVPPRFAGSVDSSSNSASLTISGLKTEDEADYYCQSYDSSNWVFGGGTKLTVLG

SEQ ID NO: 164 - DNA, 735 bp, Artificial Sequence
  source: /note="Description of Artificial Sequence: Synthetic polynucleotide"
gaagtccaattggtgcagagcggatccgaacttaagaaacctggcgcgagcgtgaaagtgtcctgcaaggcctccggagggactttctcgtcgtacgccattagctgggtccgccaagctcctggccaaggcctggagtggatgggcgggattatccccatcttcgggactgcgaactacgcccagaagtttcagggccgggtcactatcaccgccgacgaatcaacctcgaccgcctacatggaactgtcctcgcttcggtccgaggatactgccgtgtactattgtgcctcaacggccagacgcggatgggacaccgctggtccgctcgattactggggccagggaaccctcgtgaccgtcagctccggaggaggaggctccggtggtggaggatccgggggtggtggatccgacatccaaatgacccagtccccctcgtccctgagcgcctctgtgggcgacagagtgacaattgcatgcagggcctcacagactatctcccgctacctgaactggtaccagcagaagccaggaaaggcccctaagctgctcatctacgctgcgtcctcgctccaatccggggtgtcctcacggttttccggatcgggttccggcaccgagttcaccctgaccatcagcagcctgcagcccgaggacttcgcaacctacttctgccagcaaacctactccccgccgattacgttcggacaggggactcggctggaaatcaag

SEQ ID NO: 165 - protein, 245 aa, Artificial Sequence
  source: /note="Description of Artificial Sequence: Synthetic polypeptide"
EVQLVQSGSELKKPGASVKVSCKASGGTFSSYAISWVRQAPGQGLEWMGGIIPIFGTANYAQKFQGRVTITADESTSTAYMELSSLRSEDTAVYYCASTARRGWDTAGPLDYWGQGTLVTVSSGGGGSGGGGSGGGGSDIQMTQSPSSLSASVGDRVTIACRASQTISRYLNWYQQKPGKAPKLLIYAASSLQSGVSSRFSGSGSGTEFTLTISSLQPEDFATYFCQQTYSPPITFGQGTRLEIK

SEQ ID NO: 166 - DNA, 729 bp, Artificial Sequence
  source: /note="Description of Artificial Sequence: Synthetic polynucleotide"
gaagtgcaactcgtcgaaacaggggcagaagtgaaaaacccaggctcaagcgtgaaagtgtcgtgcaaggcttcgggcggaactctgtccaactacgccatctcctgggtccgccaagctccgggaaagggcctcgagtggatgggcggaatcattcccattttcgggaccgccaactacgcgcaaaagttccagggccgggtcactatcaccgcggacgaaagcaccagcaccgcctacatggaactgtcctccctgcgctccgaggacactgccgtgtactattgcgcccggaggtcatcgtggtaccccgagggctgcttccagcactggggacagggcactctcgtgaccgtgtcgtcgggtggtggtggatcaggagggggaggatccggaggaggcggaagcgatattcagctgacccagtcaccgagctccctgtccgcctccaccggagacagagtgaccatcacgtgtcgggcctcccaagggatctcctcctacctggcctggtaccagcagaagcctggaaaggcaccgaagttgctgatctacgccgcgagcacccttcagtccggagtgcctagccgcttctcgggttccggctctggcactgacttcactctgaccattagctgcctgcagtccgaggattttgccacctactactgccagcagtactatagctaccccctgaccttcgggggcggaaccaagctcgacatcaag

SEQ ID NO: 167 - protein, 243 aa, Artificial Sequence
  source: /note="Description of Artificial Sequence: Synthetic polypeptide"
EVQLVETGAEVKNPGSSVKVSCKASGGTLSNYAISWVRQAPGKGLEWMGGIIPIFGTANYAQKFQGRVTITADESTSTAYMELSSLRSEDTAVYYCARRSSWYPEGCFQHWGQGTLVTVSSGGGGSGGGGSGGGGSDIQLTQSPSSLSASTGDRVTITCRASQGISSYLAWYQQKPGKAPKLLIYAASTLQSGVPSRFSGSGSGTDFTLTISCLQSEDFATYYCQQYYSYPLTFGGGTKLDIK

SEQ ID NO: 168 - DNA, 732 bp, Artificial Sequence
  source: /note="Description of Artificial Sequence: Synthetic polynucleotide"
gaagtgcaactcgtccaatctggtgccgaagtcaagaagcctggctcaagcgtgaaagtgtcctgcaaagcgtcgggagggaccttcagctcctacgccatttcctgggtccgccaagcaccaggacagggcctggagtggatgggcggcatcatcccgatcttcgggactgccaactacgcccagaagttccaggggagagtgaccattaccgccgacgagtcgaccagcacggcctacatggaactgtccagcctgcgctccgaggacactgccgtgtactactgcgcgagggccagactcggtggagcgttcgacatctggggacagggcaccatggtcaccgtgtcatccggtggcggaggatccggtggtggcggatcaggagggggaggatcccagtccgtgctgactcagcctccctccgtgagcgctgcaccgggacagaaggtcaccatctcatgctcggggggaagctccaacatcgggaaccactacgtgtcctggtaccaacagttgcctggtgccgctccaaagctgctgatctatgacgataacaagcggccgtccggaatccccgaccggttctcggggtctagatccggaaccagcgcaactctcggcattaccggactgcagagcggcgatgaggccgactactactgtggcacatgggactcgtcgctggctgcccacgtgtttggcactggcaccaaggtcaccgtgcttgga

SEQ ID NO: 169 - protein, 244 aa, Artificial Sequence
  source: /note="Description of Artificial Sequence: Synthetic polypeptide"
EVQLVQSGAEVKKPGSSVKVSCKASGGTFSSYAISWVRQAPGQGLEWMGGIIPIFGTANYAQKFQGRVTITADESTSTAYMELSSLRSEDTAVYYCARARLGGAFDIWGQGTMVTVSSGGGGSGGGGSGGGGSQSVLTQPPSVSAAPGQKVTISCSGGSSNIGNHYVSWYQQLPGAAPKLLIYDDNKRPSGIPDRFSGSRSGTSATLGITGLQSGDEADYYCGTWDSSLAAHVFGTGTKVTVLG

SEQ ID NO: 170 - DNA, 747 bp, Artificial Sequence
  source: /note="Description of Artificial Sequence: Synthetic polynucleotide"
gaagtgcaacttgtccagagcggagccgaagtgaagaaacctggatcctccgtcaaagtgtcgtgcaaggcttcgggcggaaccttctcctcgtacgcgatctcatgggtcagacaggcacccggacagggactggagtggatgggcggcatcattcccatcttcggcaccgctaattacgcccagaagtttcaggggagagtgaccatcaccgccgacgagtccacctccactgcctacatggaactgtcctcactgaggtccgaggatactgccgtgtactactgcgcgtcgcaaaaggggggtggatggtccattgacgccttcgatatttggggacaggggacgatggtcacagtgtcatccggcggtggtggatccggtggtggcggatccggaggaggaggcagccagtccgtgctgacccagccgcctagcgtgtcggccgcatctgggcagcgcgtgaccatttcctgttccgggtcctcgtccaacatcggcaacaactacgcctcctggtaccaacagctcccgggaatggcccctaagctgctgatctacgaggacaacaagcggccatccgggatctcagaccggttcagcggatcccagtccggcacttccgcgagcctcgccatcaccggactgcaggctgaggacgaagccgactactactgccaatcatatgacagctcgctcagcggcgatgtggtgttcggcggtggcactaagctgaccgtgttggga

SEQ ID NO: 171 - protein, 249 aa, Artificial Sequence
  source: /note="Description of Artificial Sequence: Synthetic polypeptide"
EVQLVQSGAEVKKPGSSVKVSCKASGGTFSSYAISWVRQAPGQGLEWMGGIIPIFGTANYAQKFQGRVTITADESTSTAYMELSSLRSEDTAVYYCASQKGGGWSIDAFDIWGQGTMVTVSSGGGGSGGGGSGGGGSQSVLTQPPSVSAASGQRVTISCSGSSSNIGNNYASWYQQLPGMAPKLLIYEDNKRPSGISDRFSGSQSGTSASLAITGLQAEDEADYYCQSYDSSLSGDVVFGGGTKLTVLG

SEQ ID NO: 172 - DNA, 735 bp, Artificial Sequence
  source: /note="Description of Artificial Sequence: Synthetic polynucleotide"
caagtccagttgcaacaatggggagcaggccttctgaaaccgtccgagacactgagcctgacgtgcgccgtctatggcggatcgttctccggatactactggtcgtggatcagacagcctccgggaaagggtctggaatggatcggcgaaatcaaccacagcggcagcaccaattacaacccgtcactgaagtcaagggtcaccattagcgtggacacttccaagaaccagttctccctgaaactgtcgagcgtgaccgctgccgatactgccgtgtactactgtgcccgcggccaagtcaagtatagctcaagcctcggctactggggccagggaaccctcgtgaccgtgtcctcgggtggaggaggctccggtggtggaggatccggtggcggaggatcgcagtccgtgctgacccagcctccctccgtgtctgctgcccctgggcaaaaggtcaccatttcgtgctccggctcatcgtccaacatcgggaacaactttgtgtcctggtaccagcagctgcccggtactgccccaaagctgctgatctacgaggacaacaagcgcccatccgggattccggatcggttcagcggatcacggtccggaactagcgcgaccctggggatcaccgggctccagactggcgacgaagcggactactactgcggaacttgggactcctccttgggggcctgggtgttcggcggagggaccaagctcaccgtgcttgga

SEQ ID NO: 173 - protein, 245 aa, Artificial Sequence
  source: /note="Description of Artificial Sequence: Synthetic polypeptide"
QVQLQQWGAGLLKPSETLSLTCAVYGGSFSGYYWSWIRQPPGKGLEWIGEINHSGSTNYNPSLKSRVTISVDTSKNQFSLKLSSVTAADTAVYYCARGQVKYSSSLGYWGQGTLVTVSSGGGGSGGGGSGGGGSQSVLTQPPSVSAAPGQKVTISCSGSSSNIGNNFVSWYQQLPGTAPKLLIYEDNKRPSGIPDRFSGSRSGTSATLGITGLQTGDEADYYCGTWDSSLGAWVFGGGTKLTVLG

SEQ ID NO: 174 - DNA, 723 bp, Artificial Sequence
  source: /note="Description of Artificial Sequence: Synthetic polynucleotide"
caagtccaactcgtcgaaactggtggtggcctcgtgaagcctggaggatccctgcgcctttcctgtgccgcttccggctttactttctcgtcgtactccatgaactgggtcagacaggctcccggaaagggcctggaatgggtgtcctccatctcgtcctcatcctcctacatctattacgcggactccgtgaagggcagattcaccatttcccgggacaacgccaagaacagcttgtacctccaaatgaactccctgcgggcagaggacaccgccgtgtactactgcgcgagggatggggatttctggagcggagccatcgactactggggccagggaactctcgtgaccgtcagctccggtggtggtggaagcggaggcggaggttctggggggggaggatcagacattcagctgacccagtcgccatcctccctgagcgcctcagtgggggaccgcgtgactattacatgccaggcctcccaagatatctcgaactacctgaactggtatcagcagaagcctggaaaggccccgaagctgttgatctacgatgccagcaacctggagactggggtgccttcccggttctcgggatcaggctcgggcaccgatttcaccttcacgatcagcagcctgcagcccgaggacattgcaacctactactgccagcagtacgacaatctgccgctttttgggggaggcaccaagctggaaatcaaa

SEQ ID NO: 175 - protein, 241 aa, Artificial Sequence
  source: /note="Description of Artificial Sequence: Synthetic polypeptide"
QVQLVETGGGLVKPGGSLRLSCAASGFTFSSYSMNWVRQAPGKGLEWVSSISSSSSYIYYADSVKGRFTISRDNAKNSLYLQMNSLRAEDTAVYYCARDGDFWSGAIDYWGQGTLVTVSSGGGGSGGGGSGGGGSDIQLTQSPSSLSASVGDRVTITCQASQDISNYLNWYQQKPGKAPKLLIYDASNLETGVPSRFSGSGSGTDFTFTISSLQPEDIATYYCQQYDNLPLFGGGTKLEIK

SEQ ID NO: 176 - DNA, 723 bp, Artificial Sequence
  source: /note="Description of Artificial Sequence: Synthetic polynucleotide"
gaggtgcaattggtgcagtcaggtggtggagtggtgcagccaggaagatcccttagactctcgtgtgcggcgtcaggctttaccttctcctcgtactccatgaactgggtcagacaggcaccgggaaagggactggaatgggtgtcctccatctcgtcctcctcctcctacatctactacgccgatagcgtgaagggccggttcaccatttcgcgcgacaacgccaagaacaccctgtacctccaaatgaattcgctgcgggccgaagataccgctgtctattactgcgcccgcgacaactggggctcgctggactattggggccagggaaccctcgtcaccgtgtcaagcggagggggtggatccggaggcggaggatccggtggagggggaagcgacattcagatgactcagagcccgtcctccctgtctgcctccgtgggggatcgcgtgaccatcacatgccaggcctcacaagacatcagcaattacctgaactggtaccagcagaagcctggaaaggcccccaagctgctgatctacgatgccagcaacctggagactggggtgccttcaaggttctccggttccggaagcggcactgacttcaccttcactatctcgagcctgcaacccgaggacattgccacctactactgccagcagtacgacaaccttccgcacatgtacacgttcggccagggcaccaagctcgaaatcaaa

SEQ ID NO: 177 - protein, 241 aa, Artificial Sequence
  source: /note="Description of Artificial Sequence: Synthetic polypeptide"
EVQLVQSGGGVVQPGRSLRLSCAASGFTFSSYSMNWVRQAPGKGLEWVSSISSSSSYIYYADSVKGRFTISRDNAKNTLYLQMNSLRAEDTAVYYCARDNWGSLDYWGQGTLVTVSSGGGGSGGGGSGGGGSDIQMTQSPSSLSASVGDRVTITCQASQDISNYLNWYQQKPGKAPKLLIYDASNLETGVPSRFSGSGSGTDFTFTISSLQPEDIATYYCQQYDNLPHMYTFGQGTKLEIK

SEQ ID NO: 178 - DNA, 1548 bp, Artificial Sequence
  source: /note="Description of Artificial Sequence: Synthetic polynucleotide"
caggtacagcttcaacaaagcggaccgggacttgttaagcattcccaaaccctttctctcacgtgtgcaattagcggcgatagtgtatcctctaattctgcggcctggaactggatacgacaatcaccaagccggggactcgagtggttgggccgaacctactatcggtccaaatggtataatgactacgcagtatccgtgaaatctcgcattacgatcaatccagacacctccaaaaatcaattttctctgcagttgaatagcgtgactcccgaggacacggccgtttactattgcgcccaggaagttgaaccccacgatgcatttgatatttggggccagggaaccatggtgacagtgagtagtgggggtggaggatctggaggaggcggtagcggcgggggcggcagtgatatccagatgacgcagtcaccttccagcgtgtatgcgagtgtgggggacaaggtcaccataacctgtcgcgctagccaagatgtcagcgggtggctggcttggtaccagcagaaaccaggtttggctcctcagcttttgatctcaggagcgagcacgcttcagggtgaggtcccaagtcgctttagtggctctggctccgggacagacttcacgttgacgatcagcagtttgcagcctgaggatttcgcgacctactactgccagcaagcgaaatattttccgtacactttcggtcaggggaccaaattggagatcaaaggtgggggtggttcaggcggcggaggctcaggcggcggcggtagcggaggaggcggaagcgggggtggcggatcagaagtgcaactcgttcagagtggcgcggaggttaagaaacccggtgcatctgtaaaggttagctgtaaggcatcaggatacacttttaccagctattacatgcattgggtgagacaggctcccggtcaggggctcgaatggatggggttgatcaacccgagtggtggttcaacatcttacgcccagaagtttcagggccgagtaacaatgactcgggacacgtctacctcaactgtgtatatggagctttccagcctgcgctcagaggatacagcagtctattactgcgcacggtcagacagaggtataacggccactgatgcgttcgatatctggggacaagggactatggtaactgtgtcttccggaggaggaggtagtggagggggaggaagcggtggggggggctcacagtccgttttgactcagccaccaagcgtctcagtcgcaccggggcgaatggcgaaaattacttgcggcgggagcgacataggcaacaagaatgtgcattggtaccaacagaaaccaggtcaagcacctgttctcgtggtgtatgatgactacgatcgcccaagcgggatcccggagcggttctctggatcaaattctggtgatgcagccactctgacaatatcaacggtggaagtcggtgacgaggctgattacttctgccaagtatgggatggcagcggagatccctactggatgtttggaggaggtactcaactgacagttctgggc

SEQ ID NO: 179 - protein, 516 aa, Artificial Sequence
  source: /note="Description of Artificial Sequence: Synthetic polypeptide"
QVQLQQSGPGLVKHSQTLSLTCAISGDSVSSNSAAWNWIRQSPSRGLEWLGRTYYRSKWYNDYAVSVKSRITINPDTSKNQFSLQLNSVTPEDTAVYYCAQEVEPHDAFDIWGQGTMVTVSSGGGGSGGGGSGGGGSDIQMTQSPSSVYASVGDKVTITCRASQDVSGWLAWYQQKPGLAPQLLISGASTLQGEVPSRFSGSGSGTDFTLTISSLQPEDFATYYCQQAKYFPYTFGQGTKLEIKGGGGSGGGGSGGGGSGGGGSGGGGSEVQLVQSGAEVKKPGASVKVSCKASGYTFTSYYMHWVRQAPGQGLEWMGLINPSGGSTSYAQKFQGRVTMTRDTSTSTVYMELSSLRSEDTAVYYCARSDRGITATDAFDIWGQGTMVTVSSGGGGSGGGGSGGGGSQSVLTQPPSVSVAPGRMAKITCGGSDIGNKNVHWYQQKPGQAPVLVVYDDYDRPSGIPERFSGSNSGDAATLTISTVEVGDEADYFCQVWDGSGDPYWMFGGGTQLTVLG

SEQ ID NO: 180 - DNA, 732 bp, Artificial Sequence
  source: /note="Description of Artificial Sequence: Synthetic polynucleotide"
caggtacagctgcagcagtcaggtccaggactggtgaagcactcgcagaccctctcactcacctgtgccatctccggggacagtgtctctagcaacagtgctgcttggaactggatcaggcagtccccatcgagaggccttgagtggctgggaaggacatactacaggtccaagtggtataatgattatgcagtatctgtgaaaagtcgaataaccatcaacccagacacatccaagaaccagttctccctgcagttgaactctgtgactcccgaggacacggctgtgtattactgtgcccaagaggtagaacctcatgatgcttttgatatctggggccaagggacaatggtcaccgtctcttcaggaggtggcgggtctggcggtggaggtagcggtggtggcggatccgacatccagatgacccagtctccatcttccgtgtatgcatctgtaggagacaaagtcaccatcacttgtcgggcgagtcaggatgttagcggctggttagcctggtatcagcagaaaccagggctagcccctcagctcctgatctctggtgcatccactttgcaaggtgaagtcccatcaaggttcagcggcagtggatctgggacagattttactctcaccatcagcagcctgcagcctgaagattttgccacttattattgtcaacaggctaaatatttcccttacacttttggccaggggaccaagctggaaatcaaa

SEQ ID NO: 181 - protein, 244 aa, Artificial Sequence
  source: /note="Description of Artificial Sequence: Synthetic polypeptide"
QVQLQQSGPGLVKHSQTLSLTCAISGDSVSSNSAAWNWIRQSPSRGLEWLGRTYYRSKWYNDYAVSVKSRITINPDTSKNQFSLQLNSVTPEDTAVYYCAQEVEPHDAFDIWGQGTMVTVSSGGGGSGGGGSGGGGSDIQMTQSPSSVYASVGDKVTITCRASQDVSGWLAWYQQKPGLAPQLLISGASTLQGEVPSRFSGSGSGTDFTLTISSLQPEDFATYYCQQAKYFPYTFGQGTKLEIK

SEQ ID NO: 182 - DNA, 732 bp, Artificial Sequence
  source: /note="Description of Artificial Sequence: Synthetic polynucleotide"
caggtacagctgcagcagtcaggtccaggactggtgaagccctcgcagaccctctcactcacctgtgccatctcagggaacagtgtctctagcaacagtgctgcttggaactggatcaggcagtccccatcgagaggccttgagtggctgggaaggacatactacaggtccaagtggtataatgattatgcagtatctgtgaaaagtcgaataaccatcaacccagacacatccaagaaccagttctccctgcagctgaactctgtgactcccgaggacacggctgtgtattactgtgcccaagaggtagaacctcaagatgcttttgatatctggggccaagggacaatggtcaccgtctcttcaggaggtggcgggtctggcggtggaggtagcggtggtggcggatccgacatccagatgacccagtctccatcttccgtgtctgcatctgtaggagacaaagtcaccatcacttgtcgggcgagtcaggatgttagcggctggttagcctggtatcagcagaaaccagggctagcccctcagctcctgatctttggtgcatccactttgcaaggtgaagtcccatcaagattcagcggcggtggatctgggacagattttactctcaccatcagcagcctgcagcctgaagattttgccacttattattgtcaacaggctaaatatttcccttacacttttggccaggggaccaagctggaaatcaaa

SEQ ID NO: 183 - protein, 244 aa, Artificial Sequence
  source: /note="Description of Artificial Sequence: Synthetic polypeptide"
QVQLQQSGPGLVKPSQTLSLTCAISGNSVSSNSAAWNWIRQSPSRGLEWLGRTYYRSKWYNDYAVSVKSRITINPDTSKNQFSLQLNSVTPEDTAVYYCAQEVEPQDAFDIWGQGTMVTVSSGGGGSGGGGSGGGGSDIQMTQSPSSVSASVGDKVTITCRASQDVSGWLAWYQQKPGLAPQLLIFGASTLQGEVPSRFSGGGSGTDFTLTISSLQPEDFATYYCQQAKYFPYTFGQGTKLEIK

SEQ ID NO: 184 - protein, 18 aa, Artificial Sequence
  source: /note="Description of Artificial Sequence: Synthetic peptide"
GSTSGSGKPGSGEGSTKG

SEQ ID NO: 185 - protein, 5 aa, Artificial Sequence
  source: /note="Description of Artificial Sequence: Synthetic peptide"
GGGGS

SEQ ID NO: 186 - protein, 4 aa, Artificial Sequence
  source: /note="Description of Artificial Sequence: Synthetic peptide"
GFLG

SEQ ID NO: 187 - protein, 15 aa, Artificial Sequence
  source: /note="Description of Artificial Sequence: Synthetic peptide"
GGGGSGGGGSGGGGS

SEQ ID NO: 188 - protein, 4 aa, Artificial Sequence
  source: /note="Description of Artificial Sequence: Synthetic peptide"
RAKR

SEQ ID NO: 189 - protein, 25 aa, Artificial Sequence
  source: /note="Description of Artificial Sequence: Synthetic peptide"
GGGGSGGGGSGGGGSGGGGSGGGGS